European Patent Specification EP 3 458 107 B1, published March 13, 2024. Title: POLYNUCLEOTIDES ENCODING JAGGED1 FOR THE TREATMENT OF ALAGILLE SYNDROME. Applicant: ModernaTX, Inc. Application Not Yet Assigned. The sequence listing filed with the application follows.

SEQUENCE LISTING (133 sequences)

SEQ ID NO: 1 - protein, 1218 aa, Homo sapiens
MRSPRTRGRSGRPLSLLLALLCALRAKVCGASGQFELEILSMQNVNGELQNGNCCGGARNPGDRKCTRDECDTYFKVCLKEYQSRVTAGGPCSFGSGSTPVIGGNTFNLKASRGNDRNRIVLPFSFAWPRSYTLLVEAWDSSNDTVQPDSIIEKASHSGMINPSRQWQTLKQNTGVAHFEYQIRVTCDDYYYGFGCNKFCRPRDDFFGHYACDQNGNKTCMEGWMGPECNRAICRQGCSPKHGSCKLPGDCRCQYGWQGLYCDKCIPHPGCVHGICNEPWQCLCETNWGGQLCDKDLNYCGTHQPCLNGGTCSNTGPDKYQCSCPEGYSGPNCEIAEHACLSDPCHNRGSCKETSLGFECECSPGWTGPTCSTNIDDCSPNNCSHGGTCQDLVNGFKCVCPPQWTGKTCQLDANECEAKPCVNAKSCKNLIASYYCDCLPGWMGQNCDININDCLGQCQNDASCRDLVNGYRCICPPGYAGDHCERDIDECASNPCLNGGHCQNEINRFQCLCPTGFSGNLCQLDIDYCEPNPCQNGAQCYNRASDYFCKCPEDYEGKNCSHLKDHCRTTPCEVIDSCTVAMASNDTPEGVRYISSNVCGPHGKCKSQSGGKFTCDCNKGFTGTYCHENINDCESNPCRNGGTCIDGVNSYKCICSDGWEGAYCETNINDCSQNPCHNGGTCRDLVNDFYCDCKNGWKGKTCHSRDSQCDEATCNNGGTCYDEGDAFKCMCPGGWEGTTCNIARNSSCLPNPCHNGGTCVVNGESFTCVCKEGWEGPICAQNTNDCSPHPCYNSGTCVDGDNWYRCECAPGFAGPDCRININECQSSPCAFGATCVDEINGYRCVCPPGHSGAKCQEVSGRPCITMGSVIPDGAKWDDDCNTCQCLNGRIACSKVWCGPRPCLLHKGHSECPSGQSCIPILDDQCFVHPCTGVGECRSSSLQPVKTKCTSDSYYQDNCANITFTFNKEMMSPGLTTEHICSELRNLNILKNVSAEYSIYIACEPSPSANNEIHVAISAEDIRDDGNPIKEITDKIIDLVSKRDGNSSLIAAVAEVRVQRRPLKNRTDFLVPLLSSVLTVAWICCLVTAFYWCLRKRRKPGSHTHSASEDNTTNNVREQLNQIKNPIEKHGANTVPIKDYENKNSKMSKIRTHNSEVEEDDMDKHQQKARFAKQPAYTLVDREEKPPNGTPTKHPNWTNKQDNRDLESAQSLNRMEYIV

SEQ ID NO: 2 - DNA, 3654 bp, Homo sapiens
atgcgttccccacggacgcgcggccggtccgggcgccccctaagcctcctgctcgccctgctctgtgccctgcgagccaaggtgtgtggggcctcgggtcagttcgagttggagatcctgtccatgcagaacgtgaacggggagctgcagaacgggaactgctgcggcggcgcccggaacccgggagaccgcaagtgcacccgcgacgagtgtgacacatacttcaaagtgtgcctcaaggagtatcagtcccgcgtcacggccggggggccctgcagcttcggctcagggtccacgcctgtcatcgggggcaacaccttcaacctcaaggccagccgcggcaacgaccgcaaccgcatcgtgctgcctttcagtttcgcctggccgaggtcctatacgttgcttgtggaggcgtgggattccagtaatgacaccgttcaacctgacagtattattgaaaaggcttctcactcgggcatgatcaaccccagccggcagtggcagacgctgaagcagaacacgggcgttgcccactttgagtatcagatccgcgtgacctgtgatgactactactatggctttggctgcaataagttctgccgccccagagatgacttctttggacactatgcctgtgaccagaatggcaacaaaacttgcatggaaggctggatgggccccgaatgtaacagagctatttgccgacaaggctgcagtcctaagcatgggtcttgcaaactcccaggtgactgcaggtgccagtacggctggcaaggcctgtactgtgataagtgcatcccacacccgggatgcgtccacggcatctgtaatgagccctggcagtgcctctgtgagaccaactggggcggccagctctgtgacaaagatctcaattactgtgggactcatcagccgtgtctcaacgggggaacttgtagcaacacaggccctgacaaatatcagtgttcctgccctgaggggtattcaggacccaactgtgaaattgctgagcacgcctgcctctctgatccctgtcacaacagaggcagctgtaaggagacctccctgggctttgagtgtgagtgttccccaggctggaccggccccacatgctctacaaacattgatgactgttctcctaataactgttcccacgggggcacctgccaggacctggttaacggatttaagtgtgtgtgccccccacagtggactgggaaaacgtgccagttagatgcaaatgaatgtgaggccaaaccttgtgtaaacgccaaatcctgtaagaatctcattgccagctactactgcgactgtcttcccggctggatgggtcagaattgtgacataaatattaatgactgccttggccagtgtcagaatgacgcctcctgtcgggatttggttaatggttatcgctgtatctgtccacctggctatgcaggcgatcactgtgagagagacatcgatgaatgtgccagcaacccctgtttgaatgggggtcactgtcagaatgaaatcaacagattccagtgtctgtgtcccactggtttctctggaaacctctgtcagctggacatcgattattgtgagcctaatccctgccagaacggtgcccagtgctacaaccgtgccagtgactatttctgcaagtgccccgaggactatgagggcaagaactgctcacacctgaaagaccactgccgcacgaccccctgtgaagtgattgacagctgcacagtggccatggcttccaacgacacacctgaaggggtgcggtatatttcctccaacgtctgtggtcctcacgggaagtgcaagagtcagtcgggaggcaaattcacctgtgactgtaacaaaggcttcacgggaacatactgccatgaaaatattaatgactgtgagagcaacccttgtagaaacggtggcacttgcatcgatggtgtcaactcctacaagtgcatctgtagtgacggctgggagggggcctactgtgaaaccaatattaatgactgcagccagaacccctgccacaatgggggcacgtgtcgcgacctggtcaatgacttctactgtgactgtaaaaatgggtggaaaggaaagacctgccactcacgtgacagtcagtgtgatgaggccacgtgcaacaacggtggcacctgctatgatgagggggatgcttttaagtgcatgtgtcctggcggctgggaaggaacaacctgtaacatagcccgaaacagtagctgcctgcccaacccctgccataatgggggcacatgtgtggtcaacggcgagtcctttacgtgcgtctgcaaggaaggctgggaggggcccatctgtgctcagaataccaatgactgcagccctcatccctgttacaacagcggcacctgtgtggatggagacaactggtaccggtgcgaatgtgccccgggttttgctgggcccgactgcagaataaacatcaatgaatgccagtcttcaccttgtgcctttggagcgacctgtgtggatgagatcaatggctaccggtgtgtctgccctccagggcacagtggtgccaagtgccaggaagtttcagggagaccttgcatcaccatggggagtgtgataccagatggggccaaatgggatgatgactgtaatacctgccagtgcctgaatggacggatcgcctgctcaaaggtctggtgtggccctcgaccttgcctgctccacaaagggcacagcgagtgccccagcgggcagagctgcatccccatcctggacgaccagtgcttcgtccacccctgcactggtgtgggcgagtgtcggtcttccagtctccagccggtgaagacaaagtgcacctctgactcctattaccaggataactgtgcgaacatcacatttacctttaacaaggagatgatgtcaccaggtcttactacggagcacatttgcagtgaattgaggaatttgaatattttgaagaatgtttccgctgaatattcaatctacatcgcttgcgagccttccccttcagcgaacaatgaaatacatgtggccatttctgctgaagatatacgggatgatgggaacccgatcaaggaaatcactgacaaaataatcgatcttgttagtaaacgtgatggaaacagctcgctgattgctgccgttgcagaagtaagagttcagaggcggcctctgaagaacagaacagatttccttgttcccttgctgagctctgtcttaactgtggcttggatctgttgcttggtgacggccttctactggtgcctgcggaagcggcggaagccgggcagccacacacactcagcctctgaggacaacaccaccaacaacgtgcgggagcagctgaaccagatcaaaaaccccattgagaaacatggggccaacacggtccccatcaaggattatgagaacaagaactccaaaatgtctaaaataaggacacacaattctgaagtagaagaggacgacatggacaaacaccagcagaaagcccggtttgccaagcagccggcgtacacgctggtagacagagaagagaagccccccaacggcacgccgacaaaacacccaaactggacaaacaaacaggacaacagagacttggaaagtgcccagagcttaaaccgaatggagtacatcgta

SEQ ID NO: 3 - protein, 1054 aa, Artificial Sequence
  Synthetic polypeptide
MRSPRTRGRSGRPLSLLLALLCALRAKVCGASGQFELEILSMQNVNGELQNGNCCGGARNPGDRKCTRDECDTYFKVCLKEYQSRVTAGGPCSFGSGSTPVIGGNTFNLKASRGNDRNRIVLPFSFAWPRSYTLLVEAWDSSNDTVQPDSIIEKASHSGMINPSRQWQTLKQNTGVAHFEYQIRVTCDDYYYGFGCNKFCRPRDDFFGHYACDQNGNKTCMEGWMGPECNRAICRQGCSPKHGSCKLPGDCRCQYGWQGLYCDKCIPHPGCVHGICNEPWQCLCETNWGGQLCDKDLNYCGTHQPCLNGGTCSNTGPDKYQCSCPEGYSGPNCEIAEHACLSDPCHNRGSCKETSLGFECECSPGWTGPTCSTNIDDCSPNNCSHGGTCQDLVNGFKCVCPPQWTGKTCQLDANECEAKPCVNAKSCKNLIASYYCDCLPGWMGQNCDININDCLGQCQNDASCRDLVNGYRCICPPGYAGDHCERDIDECASNPCLNGGHCQNEINRFQCLCPTGFSGNLCQLDIDYCEPNPCQNGAQCYNRASDYFCKCPEDYEGKNCSHLKDHCRTTPCEVIDSCTVAMASNDTPEGVRYISSNVCGPHGKCKSQSGGKFTCDCNKGFTGTYCHENINDCESNPCRNGGTCIDGVNSYKCICSDGWEGAYCETNINDCSQNPCHNGGTCRDLVNDFYCDCKNGWKGKTCHSRDSQCDEATCNNGGTCYDEGDAFKCMCPGGWEGTTCNIARNSSCLPNPCHNGGTCVVNGESFTCVCKEGWEGPICAQNTNDCSPHPCYNSGTCVDGDNWYRCECAPGFAGPDCRININECQSSPCAFGATCVDEINGYRCVCPPGHSGAKCQEVSGRPCITMGSVIPDGAKWDDDCNTCQCLNGRIACSKVWCGPRPCLLHKGHSECPSGQSCIPILDDQCFVHPCTGVGECRSSSLQPVKTKCTSDSYYQDNCANITFTFNKEMMSPGLTTEHICSELRNLNILKNVSAEYSIYIACEPSPSANNEIHVAISAEDIRDDGNPIKEITDKIIDLVSKRDGNSSLIAAVAE

SEQ ID NO: 4 - DNA, 3162 bp, Artificial Sequence
  Synthetic polynucleotide
atgagaagtccacggacgcgcggccgctcagggcgtccattgtccctcctgctcgccctgctctgcgccctccgagccaaggtctgtggtgccagtggtcagttcgagttggagatcctgtccatgcagaatgtgaacggggaactgcagaatgggaactgctgcggcggcgcccggaatccgggagaccgaaaatgcacacgcgacgaatgcgacacgtacttcaaagtctgtctcaaggaataccaatcacgcgttacggccggggggccctgtagcttcggatcagggtccacccctgttatcgggggtaacaccttcaaccttaaggccagcaggggcaacgaccgcaaccgcatcgtgctgcctttctcgtttgcctggccgaggtcctatacgttgcttgtggaggcgtgggattcttctaatgataccgttcagcctgacagcattattgaaaaggcttctcacagcggcatgatcaatcccagccggcaatggcaaacgctgaagcaaaacacgggggtggcccactttgagtatcaaatccgcgtgacatgcgatgactactactacggcttcggatgtaataagttctgccgccctagagacgatttctttggccactatgcctgtgatcagaatggcaacaaaacttgtatggagggctggatggggcccgaatgtaacagagcaatttgtcgacagggctgtagtcctaagcacgggtcttgcaaactcccaggtgattgtaggtgtcagtacggttggcaaggcctgtattgtgataagtgtattccacatcccggatgcgtccacggtatctgcaacgagccctggcaatgtctctgtgagacaaattgggggggccagctttgcgacaaagatctcaattattgcggtacgcatcaaccgtgccttaatgggggaacttgcagcaatacaggacctgataagtaccagtgctcctgccctgaggggtattcaggacccaactgtgagattgccgagcacgcttgcttgtcagatccctgccacaatcgaggctcatgtaaggagacaagcctgggctttgaatgtgagtgttctccaggctggaccggacccacatgctcaacaaacattgatgattgttctcctaacaactgttctcatggcgggacctgccaagacctggttaacggttttaagtgtgtatgcccaccccagtggactgggaagacgtgccaactagatgcgaacgaatgcgaagccaaaccctgtgtgaacgccaaatcctgtaagaatttaattgctagctactactgcgattgccttcctggctggatgggtcagaattgtgacataaatattaatgactgcttgggccagtgtcagaatgacgcctcttgccgggatttggtgaatggttatcgctgtatctgtccaccgggctatgcaggcgatcactgcgagagagatattgatgagtgtgccagcaatccctgtttgaatgggggtcactgccagaacgaaattaacagattccagtgcctgtgtcccacgggtttttctggaaacctctgtcagctggatatcgactattgtgagcctaacccctgccagaatggtgcgcaatgctacaatagggcgagtgactacttctgtaagtgtcccgaagattatgagggaaagaactgctcacacctgaaggaccactgcagaacaaccccctgtgaagtgatagatagctgcacagttgcgatggcttccaatgatacaccagagggggtgcggtatatttcttccaacgtctgcggtccacacggcaagtgcaagagtcaatcgggaggaaaattcacctgcgactgtaacaagggcttcaccggaacctactgccatgagaatatcaatgattgcgagagcaacccatgcaggaacggtgggacctgcatcgacggggtcaactcctacaaatgcatctgcagtgacggctgggaaggggcctactgtgaaaccaacattaatgactgcagccagaacccttgtcataatgggggcacgtgtcgcgacctagtcaacgacttctattgtgactgtaaaaatgggtggaaaggaaagacatgccacagccgtgatagccagtgtgatgaggcaacgtgcaacaacggtggcacttgctatgatgagggggatgcttttaagtgcatgtgtcctggcggctgggaaggaactacatgcaatatcgcccgaaacagtagctgcctgcctaatccctgccataacgggggaacatgtgtggttaacggcgagtccttcacgtgcgtttgtaaagaaggctgggagggccctatatgtgctcagaataccaatgactgcagcccgcatccctgttacaatagcggcacctgtgttgacggtgacaattggtatcggtgcgaatgtgcgccgggtttcgcaggtccagactgcagaataaatatcaatgaatgccaaagctcaccgtgcgcctttggagcgacctgtgtggatgaaatcaacggctatcggtgtgtctgccctcccgggcatagtggtgccaaatgccaggaagtgtccggcagaccttgcatcaccatggggagtgtgataccggatggcgctaaatgggatgatgattgtaatacctgtcagtgcctgaacggacggatcgcttgttcaaaggtctggtgtggccctcgaccatgcttgttacataagggacactccgagtgccccagcggtcagtcgtgtatccctattctggacgaccagtgcttcgtccatccctgtactggtgtgggcgagtgtaggtctagcagtctccagccggttaagacaaaatgcaccagtgactcctattaccaagataactgtgcgaacatcacatttacctttaataaagagatgatgtcaccaggtcttaccacggagcacatttgcagtgaattgaggaatttgaatattttgaagaatgtttccgctgaatattcaatctacatcgcttgcgagccttccccttcagcgaacaatgaaatacatgtggccatttctgctgaagatatacgggatgatgggaacccgatcaaggaaatcactgacaaaataatcgatcttgttagtaaacgtgatgggaacagctcgctgattgctgcagttgcagaa

SEQ ID NO: 5 - protein, 1046 aa, Artificial Sequence
  Synthetic polypeptide
MRSPRTRGRSGRPLSLLLALLCALRAKVCGASGQFELEILSMQNVNGELQNGNCCGGARNPGDRKCTRDECDTYFKVCLKEYQSRVTAGGPCSFGSGSTPVIGGNTFNLKASRGNDRNRIVLPFSFAWPRSYTLLVEAWDSSNDTVQPDSIIEKASHSGMINPSRQWQTLKQNTGVAHFEYQIRVTCDDYYYGFGCNKFCRPRDDFFGHYACDQNGNKTCMEGWMGPECNRAICRQGCSPKHGSCKLPGDCRCQYGWQGLYCDKCIPHPGCVHGICNEPWQCLCETNWGGQLCDKDLNYCGTHQPCLNGGTCSNTGPDKYQCSCPEGYSGPNCEIAEHACLSDPCHNRGSCKETSLGFECECSPGWTGPTCSTNIDDCSPNNCSHGGTCQDLVNGFKCVCPPQWTGKTCQLDANECEAKPCVNAKSCKNLIASYYCDCLPGWMGQNCDININDCLGQCQNDASCRDLVNGYRCICPPGYAGDHCERDIDECASNPCLNGGHCQNEINRFQCLCPTGFSGNLCQLDIDYCEPNPCQNGAQCYNRASDYFCKCPEDYEGKNCSHLKDHCRTTPCEVIDSCTVAMASNDTPEGVRYISSNVCGPHGKCKSQSGGKFTCDCNKGFTGTYCHENINDCESNPCRNGGTCIDGVNSYKCICSDGWEGAYCETNINDCSQNPCHNGGTCRDLVNDFYCDCKNGWKGKTCHSRDSQCDEATCNNGGTCYDEGDAFKCMCPGGWEGTTCNIARNSSCLPNPCHNGGTCVVNGESFTCVCKEGWEGPICAQNTNDCSPHPCYNSGTCVDGDNWYRCECAPGFAGPDCRININECQSSPCAFGATCVDEINGYRCVCPPGHSGAKCQEVSGRPCITMGSVIPDGAKWDDDCNTCQCLNGRIACSKVWCGPRPCLLHKGHSECPSGQSCIPILDDQCFVHPCTGVGECRSSSLQPVKTKCTSDSYYQDNCANITFTFNKEMMSPGLTTEHICSELRNLNILKNVSAEYSIYIACEPSPSANNEIHVAISAEDIRDDGNPIKEITDKIIDLVSKRDGNS

SEQ ID NO: 6 - DNA, 3138 bp, Artificial Sequence
  Synthetic polynucleotide
atgaggtcacctcggacgagaggtcggagcgggcgacctttatctctcctcctagctctgctgtgcgcgctaagggcgaaagtgtgcggtgcgagcggtcaattcgaacttgaaattcttagtatgcaaaacgtaaatggcgaactgcaaaatgggaattgctgtggcggggcgcggaatcccggcgacagaaaatgcacgcgggatgagtgcgacacgtactttaaagtctgccttaaggagtaccaaagtagggtgacagcaggcgggccttgtagtttcggctcgggtagcacccctgtaattggcggtaataccttcaacttgaaggcctcacgcggcaatgacagaaatcgtatagttctgccctttagttttgcatggccgaggtcgtataccttgttggtagaggcgtgggactcatcgaacgacactgtccagcccgactcgatcattgaaaaggcctcgcacagtgggatgataaatcctagccggcagtggcaaacactcaagcagaacacgggcgtcgcgcactttgagtaccagataagagtaacatgtgatgattactattacggtttcggttgtaacaaattctgtcgtcctcgagacgacttctttggacattacgcatgtgaccaaaacggtaataagacatgtatggaaggctggatgggccccgagtgcaacagggcgatctgtagacagggttgttccccgaaacatggttcttgcaaactaccgggtgactgcaggtgtcaatatggttggcagggcctgtactgtgataaatgcataccgcatcctgggtgcgtccatggtatctgtaatgagccatggcagtgcctctgtgagacaaattggggtggccaactttgtgacaaggacctaaactattgtgggactcatcaaccgtgtctgaatgggggaacatgttcaaatactggtcctgacaagtatcagtgtagttgtccagaaggttactcggggccaaattgtgagatagcggaacatgcctgcctctcagacccgtgtcataatcggggctcttgcaaggaaacatccctagggtttgagtgcgagtgttctcctggttggacgggtccgacgtgctccacaaacatcgacgattgtagcccgaataactgttcccacgggggaacatgccaggatctagttaacggttttaagtgtgtttgtccgccccaatggaccggaaaaacctgtcagttggatgccaatgaatgtgaggccaaaccgtgcgtgaacgcgaaatcgtgtaagaatttgatcgcttcgtactactgtgattgtttgccgggatggatgggacaaaactgcgatataaatattaatgactgtttgggccaatgccaaaatgatgcatcctgtagggatcttgtaaacggatacaggtgcatatgtcctccaggctacgctggtgatcactgcgagagagatatagacgaatgtgcctcgaacccttgcctaaatggtggtcattgtcaaaatgagataaatcgattccagtgtctatgcccgaccggcttctcggggaatctttgtcagttagacatagattattgtgagcccaatccatgtcaaaacggcgcccagtgctacaatcgggctagcgattacttctgtaagtgcccggaggattacgaagggaagaattgctcacatttaaaagaccactgccgtacgacgccttgcgaagttattgactcctgcaccgtggccatggcctccaacgatacgcctgagggggtcaggtacatatctagtaacgtttgtggcccccatggaaagtgcaaatcccagtccggcgggaaattcacatgcgattgcaacaagggttttacgggtacttattgccacgagaacattaatgattgtgaaagcaacccatgtagaaatgggggtacctgtattgatggtgtcaacagttacaaatgtatttgtagcgatggctgggaaggcgcctactgcgagacaaatataaacgactgctcccagaacccctgccacaatgggggcacctgccgcgacttggtaaatgatttttattgcgattgcaagaacggttggaagggcaaaacatgccactcgcgagactcgcagtgtgacgaagccacgtgcaataatggtggcacgtgctatgacgagggagacgccttcaagtgtatgtgccctggcgggtgggagggtacaacatgtaacatcgccaggaactcgagttgtctccctaatccctgtcataacggtgggacctgtgtagtcaacggggaatcctttacatgtgtttgcaaggaaggctgggaaggcccaatctgtgcccagaatacgaacgattgctcaccgcatccgtgttataactcgggcacgtgtgtagatggcgataattggtatcgctgtgaatgcgctccaggattcgccggtccggattgtcgaataaatattaacgagtgtcagtcatcgccttgtgcctttggcgcgacatgtgttgacgaaattaacggatatcgttgcgtttgtccgcccggccattccggcgcaaaatgccaagaagttagtggaagaccttgcatcactatgggctccgttatccctgacggcgcgaagtgggacgacgattgcaacacctgccagtgtttaaatggcaggatcgcgtgttcgaaagtttggtgcgggccacgtccctgcctcctgcacaaaggacattctgagtgccctagtggtcaaagttgtataccgatattggatgatcaatgttttgtacacccgtgcacaggagttggagaatgtcgctcaagctcactccaaccagttaaaacgaagtgtacgagtgacagttattaccaggataactgtgcgaatataacattcacatttaacaaagagatgatgtctcctgggctgacgactgaacatatctgtagtgagctaaggaaccttaacatcttgaaaaacgtatctgctgaatactcaatatacatagcctgtgagccatccccttccgcgaacaatgaaatacatgtagccatttcagcagaagacatccgtgatgacggaaacccgatcaaggaaataacagacaaaataatcgacctggtctcaaaacgggatggaaattcc

SEQ ID NO: 7 - protein, 261 aa, Artificial Sequence
  Synthetic polypeptide
MGVKVLFALICIAVAEACDDYYYGFGCNKFCRPRDKTHTCPPCPAPEAAGGPSVFLFPPKPKDTLYITREPEVTCVVVDVSHEDPEVKFNWYVDGVEVHNAKTKPREEQYNSTYRVVSVLTVLHQDWLNGKEYKCKVSNKALPAPIEKTISKAKGQPREPQVYTLPPSRDELTKNQVSLTCLVKGFYPSDIAVEWESNGQPENNYKTTPPVLDSDGSFFLYSKLTVDKSRWQQGNVFSCSVMHEALKFHYTQKSLSLSPGK

SEQ ID NO: 8 - DNA, 783 bp, Artificial Sequence
  Synthetic polynucleotide
atgggagtcaaagttctgtttgccctgatctgcatcgctgtggccgaggcctgtgatgactactactatggctttggctgcaataagttctgccgccccagagacaagacccacacctgccccccctgccccgcccccgaggccgccggcgggcccagcgtgttcctgttcccccccaagcccaaggacaccctgtacatcaccagggagcccgaggtgacctgcgtggtggtggacgtgagccacgaggaccccgaggtgaagttcaactggtacgtggacggcgtggaggtgcacaacgccaagaccaagcccagggaggagcagtacaacagcacctacagggtggtgagcgtgctgaccgtgctgcaccaggactggctgaacggcaaggagtacaagtgcaaggtgagcaacaaggccctgcccgcccccatcgagaagaccatcagcaaggccaagggccagcccagggagccccaggtgtacaccctgccccccagcagggacgagctgaccaagaaccaggtgagcctgacctgcctggtgaagggcttctaccccagcgacatcgccgtggagtgggagagcaacggccagcccgagaacaactacaagaccaccccccccgtgctggacagcgacggcagcttcttcctgtacagcaagctgaccgtggacaagagcaggtggcagcagggcaacgtgttcagctgcagcgtgatgcacgaggccctgaagttccactacacccagaagagcctgagcctgagccccggcaag

SEQ ID NO: 9 - protein, 276 aa, Artificial Sequence
  Synthetic polypeptide
MGVKVLFALICIAVAEADKTHTCPPCPAPEAAGGPSVFLFPPKPKDTLYITREPEVTCVVVDVSHEDPEVKFNWYVDGVEVHNAKTKPREEQYNSTYRVVSVLTVLHQDWLNGKEYKCKVSNKALPAPIEKTISKAKGQPREPQVYTLPPSRDELTKNQVSLTCLVKGFYPSDIAVEWESNGQPENNYKTTPPVLDSDGSFFLYSKLTVDKSRWQQGNVFSCSVMHEALKFHYTQKSLSLSPGKGGGGSGGGGSGGGGSCDDYYYGFGCNKFCRPR

SEQ ID NO: 10 - DNA, 828 bp, Artificial Sequence
  Synthetic polynucleotide
atgggagtcaaagttctgtttgccctgatctgcatcgctgtggccgaggccgacaagacccacacctgccccccctgccccgcccccgaggccgccggcggtcccagcgtgttcctgttcccccccaagcccaaggacaccctgtacatcaccagggagcccgaggtgacctgcgtggtggtggacgtgagccacgaggaccccgaggtgaagttcaactggtacgtggacggcgtggaggtgcacaacgccaagaccaagcccagggaggagcagtacaacagcacctacagggtggtgagcgtgctgaccgtgctgcaccaggactggctgaacggcaaggagtacaagtgcaaggtgagcaacaaggccctgcccgcccccatcgagaagaccatcagcaaggccaagggccagcccagggagccccaggtgtacaccctgccccccagcagggacgagctgaccaagaaccaggtgagcctgacctgcctggtgaagggcttctaccccagcgacatcgccgtggagtgggagagcaacggccagcccgagaacaactacaagaccaccccccccgtgctggacagcgacggcagcttcttcctgtacagcaagctgaccgtggacaagagcaggtggcagcagggcaacgtgttcagctgcagcgtgatgcacgaggccctgaagttccactacacccagaagagcctgagcctgagccccggcaagggtggcggtggctcgggcggtggtgggtcgggtggcggcggatcttgtgatgactactactatggctttggctgcaataagttctgccgccccaga

SEQ ID NO: 11 - DNA, 3654 bp, Artificial Sequence
  Synthetic polynucleotide
atgcgaagccccaggacccgcggccgtagcggtaggcccctgtccctgctgctggccctgctgtgcgccctcagggccaaggtgtgcggcgccagcggccagttcgagctcgagatcctgagcatgcagaacgtgaacggcgagctccagaatgggaattgttgcggcggcgccaggaaccccggtgacaggaaatgcacccgcgacgagtgcgacacctacttcaaagtgtgcctcaaggagtaccagagcagggtgaccgccggcgggccctgcagcttcgggagcggctccacgcccgtgatcggcgggaacaccttcaacctgaaggccagcaggggcaacgatcggaaccggatcgtgctgccgttctccttcgcctggccgcgaagctacaccctgctggtggaagcgtgggacagcagcaacgacaccgtgcagcccgacagcatcatcgagaaggcctcacactccggtatgatcaaccccagcaggcagtggcagaccctgaagcagaacaccggagtggcccacttcgaataccagatcagggtgacatgcgacgactactactacggcttcgggtgcaacaagttctgcaggccccgcgacgacttcttcggacactacgcctgtgaccagaacgggaacaagacgtgtatggaggggtggatggggcccgaatgcaacagggccatctgtcggcagggttgctcccccaagcacggctcctgcaaactgcccggcgattgccggtgccagtacgggtggcaaggtctgtactgcgacaagtgcatcccgcatcccggctgcgtgcacggcatctgcaacgagccctggcagtgcctgtgcgaaaccaactggggcggccagctctgtgacaaggaccttaactactgcggcacccaccagccctgcctgaacggcgggacctgcagcaacaccgggcccgacaagtaccagtgtagctgccccgaagggtactcgggtcccaactgcgagatcgccgagcacgcctgcctgtccgacccctgccataacaggggcagctgtaaggagacctccctgggcttcgagtgtgagtgctcccccggatggaccggccccacctgcagcaccaatattgacgactgcagcccaaataactgctcccacggcggcacctgccaggacctcgtgaacggctttaagtgcgtctgtcccccccagtggaccggcaagacctgccagctggacgccaatgagtgcgaggccaagccctgtgtaaacgccaagagctgcaagaacctgatcgccagctactactgtgactgcctgcccggctggatgggccagaactgcgacatcaacatcaacgactgcctcgggcagtgccagaacgacgccagctgcagggatctggtgaacggctacaggtgcatctgcccccccggatacgccggcgaccattgcgaaagggacatcgatgagtgcgcctccaatccctgtctgaacggcggccactgccagaacgagatcaacaggttccagtgcctgtgccccaccggcttcagcgggaacctgtgccagctggacatcgactattgcgagcccaatccctgccagaacggggcgcagtgctacaacagggccagcgactacttctgcaagtgccccgaggactacgagggcaagaattgcagccacctgaaagaccactgccgcaccaccccctgtgaggttatcgacagctgtacggtcgccatggcctcgaacgacacccccgaaggcgtgaggtatatctccagcaacgtgtgcgggccacacggcaaatgtaagtcccagagcggcgggaagttcacctgcgactgcaacaagggcttcacaggcacgtactgccatgagaacatcaacgattgtgagagcaacccctgcaggaacggcgggacctgcatagacggcgtgaacagctataagtgcatctgcagcgatggctgggagggagcctactgcgaaaccaacatcaatgactgcagccagaacccctgtcacaacgggggcacatgccgggacctggtgaatgatttctactgcgactgcaagaatggctggaagggcaagacctgccacagcagggactcccagtgtgacgaggccacctgcaataacgggggcacctgctacgacgagggcgacgcctttaagtgcatgtgccccggcggttgggagggtaccacctgcaacatcgcgcggaacagcagctgtctgcccaacccctgccacaacgggggcacgtgcgtggtgaacggcgagagcttcacctgcgtgtgtaaggaggggtgggagggccccatctgcgcccagaacaccaacgattgctcgccccacccctgttacaacagcgggacctgcgtggacggtgataactggtacaggtgcgagtgcgcaccaggcttcgccgggccggactgcaggatcaacatcaacgaatgtcagagctccccgtgcgccttcggcgccacgtgcgtagacgagatcaatggctacaggtgcgtgtgccccccaggccacagcggggccaaatgccaggaagtcagcggccgaccctgcatcaccatgggttccgttatcccagacggagccaagtgggatgacgattgtaacacctgtcagtgtctgaatggccggatcgcgtgcagcaaggtgtggtgcggccccaggccgtgcctgctgcacaagggccactccgaatgtccctccggtcagagctgcatccccatcctcgacgaccagtgctttgtacacccctgcaccggagtcggcgagtgcaggtcctcgtctctgcagcccgtgaaaaccaagtgcaccagcgactcctactaccaggacaactgcgccaacatcacgttcacctttaacaaggagatgatgagccccgggctgaccacggagcacatctgctcggagctgaggaacctgaacatactgaagaacgtgagcgccgagtacagcatctacattgcctgcgagcccagccccagcgccaacaacgagatccacgtggcgatctccgccgaagacatccgggacgacggcaaccccatcaaggagataaccgacaagatcatcgacctggtgagcaagcgggacggcaacagctccctgatcgccgccgtggccgaggtgcgggtacagaggcggcccctcaagaacaggacggacttcctcgtgccgctcctgtcgtccgtgctgaccgtggcctggatctgctgtctggtgaccgccttctactggtgcctgcggaagcggcgcaagccggggagccacacccactcggccagcgaagacaacacgaccaacaacgtgagggagcagctgaatcagatcaagaatcccatagagaaacacggcgccaacaccgtgcccatcaaggattacgagaacaagaacagcaagatgtccaaaatcagaacccacaatagcgaagtggaggaagacgacatggataagcaccagcagaaggccaggttcgccaagcagcccgcctacaccctggtagacagggaggagaagccccccaacggcacccccacgaaacacccgaactggaccaacaagcaggataatagggacctggagtccgcgcagagcctgaaccgcatggagtacatcgtg

SEQ ID NO: 12 - DNA, 3654 bp, Artificial Sequence
  Synthetic polynucleotide
atgaggagccccaggacccggggccgtagcgggaggccgctctcgctgctgctggccctgctctgcgccctgagggccaaggtgtgtggcgcctccgggcagttcgagctggaaatcctgagcatgcagaacgtcaacggcgagctgcagaacggcaactgctgcggcggagcgcggaaccccggggacaggaagtgcaccagggacgagtgtgacacgtacttcaaagtctgcctcaaggagtaccagagccgggtgaccgccgggggcccatgctccttcggcagcggcagcacccccgtcatcggaggcaacacctttaatctgaaggccagcagggggaacgacaggaataggatcgtcctgccctttagcttcgcctggcccaggtcctacaccctgctggtcgaggcctgggacagctccaacgacaccgtccagcccgacagtatcatcgagaaggcgtcccactccggcatgatcaatcccagcaggcagtggcagacgctgaagcagaacaccggcgtggcccacttcgagtatcagatccgggtgacgtgcgacgactactactacgggttcggctgcaacaagttctgtaggccccgggacgatttcttcggccactacgcatgcgaccagaacggcaacaagacctgcatggagggctggatgggccccgagtgcaacagggctatctgccgccagggctgctcccccaagcacggcagctgtaagctgcccggcgattgccggtgtcagtacgggtggcagggactgtattgcgacaagtgcataccccacccaggctgcgtgcacggcatctgtaacgagccctggcaatgcctctgcgagaccaactgggggggacaactgtgcgacaaggacctgaactactgcggtacccaccagccctgcctgaacggcggcacctgcagtaacaccggccccgacaagtatcagtgcagctgccccgaggggtattccggcccgaactgcgagatcgccgagcacgcctgcctcagcgacccatgccacaatagaggcagctgcaaggaaacctccctggggttcgagtgtgagtgctcccccgggtggaccgggcccacctgctccaccaacatcgacgactgcagccccaataactgcagccacgggggcacctgtcaggacctggtgaacggctttaagtgcgtctgccccccccagtggaccggtaagacgtgccagctggacgccaatgagtgcgaagccaagccctgcgtcaatgccaagagctgtaagaacctcatcgcgtcctactattgcgactgcctgcccgggtggatgggacagaactgcgacatcaacatcaacgactgcctcgggcagtgccagaacgacgccagctgccgggacctggtgaacggctatagatgcatctgcccccccggctacgccggggaccactgcgagagggacatcgacgagtgcgcctccaacccctgcctgaatggaggccactgccagaacgaaatcaacaggttccagtgtctgtgccccaccggattcagcggaaacctgtgccagctggacatcgactattgcgaacccaacccctgtcagaacggcgcccagtgctacaaccgggcaagcgactacttctgcaagtgccctgaggactacgagggcaagaactgcagccacctcaaggaccactgcaggacgaccccctgtgaggtgatcgacagctgtaccgtggccatggcctcgaacgacacccctgagggcgtgaggtatatctccagcaacgtctgcggcccccacggcaaatgtaagagccaatccgggggcaagttcacctgcgactgcaacaagggatttaccggcacctactgccacgagaacatcaacgactgcgagtccaatccctgccgtaacggcggcacctgcatcgacggtgtcaacagctacaagtgcatctgcagcgacggctgggagggagcgtactgcgaaaccaacataaacgattgttcccagaacccctgccacaacggcggcacctgccgggaccttgtgaacgacttttactgtgactgcaagaatgggtggaagggcaaaacgtgccacagcagagacagccagtgcgacgaagccacctgtaacaacggcggcacctgctacgacgagggcgacgcctttaagtgtatgtgcccgggcggctgggaaggcacgacctgcaacatcgcccggaacagcagctgcctcccgaacccttgccacaacggcgggacctgcgtggtgaatggcgaatccttcacctgcgtgtgcaaggagggctgggagggccccatctgcgcccaaaacaccaatgactgtagcccccacccctgctacaactccggcacatgtgtggatggcgacaactggtacaggtgtgagtgcgcccccggattcgccggccccgactgccggatcaacattaacgagtgtcagagcagcccctgcgccttcggcgccacctgcgtcgatgagataaacggatataggtgcgtgtgcccccccggacacagcggcgcgaagtgccaggaggtgagcggcaggccctgcatcacaatgggcagcgtgatcccggacggcgccaagtgggacgacgattgcaacacctgccagtgcctgaacggccggatagcctgctccaaagtgtggtgcggcccccgcccctgcctgctgcacaagggccacagcgagtgcccctccggccagagctgcatccccatactggacgaccaatgtttcgtgcatccctgcaccggcgtgggcgagtgtcggagcagcagcctgcagcccgtgaagactaagtgcacctccgactcctactatcaggacaactgtgccaacatcaccttcaccttcaacaaggagatgatgagccccggcctgacaacggagcacatctgcagcgagctgcgcaatctgaacatcctgaaaaatgtgagcgccgagtacagcatctacatcgcctgtgagccgagccccagcgctaataacgagatccacgtggccatctccgccgaggacatcagggatgacggcaaccccatcaaagagatcaccgacaagatcatcgacctggtgtccaagcgggacggcaactccagcctgatcgcagccgtggccgaagtgagggtccagcggcggcccctgaagaaccgaaccgacttcctggtccccctgctgagcagcgtgctgaccgtcgcatggatctgttgcctggtgacggccttctactggtgcctcaggaaaagacggaagcccgggagccacacccacagcgccagcgaggacaacaccaccaacaacgtgcgggagcagctgaaccaaatcaagaaccccatcgagaagcatggcgccaataccgtgcccatcaaagactacgagaacaagaacagcaagatgagcaagatccgcacccataactcggaggtggaagaagacgatatggataagcaccagcaaaaggcccggttcgcgaagcagcccgcctataccctcgtggaccgggaagaaaagccgcccaacggcacccccaccaagcaccccaactggaccaacaaacaggacaacagggacctcgagagcgcccagtccctcaaccgtatggagtacatcgtc

SEQ ID NO: 13 - DNA, 3654 bp, Artificial Sequence
  Synthetic polynucleotide
atgaggtccccgcgtacccgaggcaggtccgggaggcccctgtccctgctgctcgccttactttgcgccctgagggccaaagtctgcggcgcctccggccaattcgagctggagatcctcagcatgcagaacgtgaacggcgagctgcaaaacgggaactgctgcgggggagcccgcaaccccggcgaccggaagtgcaccagggacgagtgcgacacctacttcaaggtgtgcctcaaggagtatcagtcaagggtgaccgccggaggcccctgtagcttcggctccgggtcgacccccgtgataggcggaaacaccttcaacctgaaggccagcagggggaacgacaggaataggatcgtgctccccttctcgttcgcctggcccaggagctacaccctcctcgtggaggcctgggacagcagcaacgatacggtgcagcccgactccatcatcgagaaggccagccactccggcatgatcaaccccagccgccagtggcagaccctgaagcaaaacacgggcgtggcacacttcgagtaccagataagggtcacttgcgacgactactactacgggttcgggtgcaacaagttttgcaggccccgggacgacttcttcggacactatgcctgcgaccagaacggcaacaagacctgtatggagggttggatgggccccgaatgcaatcgcgccatttgccggcaggggtgcagccctaagcacggaagctgtaagctccccggcgactgccgctgccagtacggctggcagggactgtactgtgacaagtgtatcccccaccccggctgcgtgcacggcatctgcaatgagccttggcagtgcctgtgcgagaccaattggggcggccagctgtgcgacaaggacctgaactactgcggcacccaccagccctgcctgaacggtgggacctgcagcaacaccgggccagacaagtaccagtgcagctgccccgagggctatagcgggcccaattgcgagatcgccgagcacgcctgcctgtccgacccctgtcacaaccggggctcctgcaaggagacctccctggggtttgagtgcgagtgctcccccggttggaccggccccacctgctccaccaacatcgacgactgctcccccaacaattgcagccacggcggcacatgccaggatctggtgaacggcttcaagtgtgtgtgtcccccccagtggaccggcaagacctgccagctggacgcgaacgagtgcgaagcaaagccctgcgtgaacgccaagtcctgcaaaaacctgatcgccagctattactgcgactgcctgcccggctggatggggcagaactgtgacataaacataaacgactgcctcggccagtgccagaatgacgcgagctgccgggacctcgtgaacggctaccgatgcatctgccccccgggctacgccggcgaccattgcgaacgggatatcgacgagtgtgccagcaacccctgcctgaacggggggcactgccagaacgagataaacaggttccagtgcctgtgccccaccggcttcagcggcaacctgtgccaactcgacatcgactactgcgagcccaacccctgccaaaacggtgcccaatgctacaaccgggcctcggactacttttgcaagtgcccggaggactatgagggcaagaattgttcccacctcaaggaccactgccggaccaccccctgcgaggtgatcgactcctgcaccgtggccatggctagtaacgatacccccgagggcgttaggtacatctcctccaacgtgtgcggcccccacgggaagtgcaagtcgcagagcggcggcaagttcacctgcgactgcaataagggcttcaccggtacctactgccacgagaacatcaacgactgcgagagcaatccctgccggaacgggggtacctgcatcgacggcgtgaactcctacaagtgtatctgctcagatggctgggaaggcgcgtactgtgagaccaacataaacgactgtagccagaacccctgtcataacgggggcacctgcagggacctggtgaacgacttctactgcgactgcaagaacgggtggaaaggcaaaacttgccactccagggactcccagtgcgatgaggccacctgcaataacggcggcacgtgctacgacgagggggacgccttcaagtgcatgtgccccgggggctgggaggggaccacctgcaacatcgccaggaacagctcctgcctgcccaacccatgccacaatggaggcacctgcgtagtgaatggcgagtccttcacctgtgtgtgcaaggagggctgggaggggcccatctgcgcccagaacaccaacgactgcagcccacacccgtgctacaactccggcacctgcgtcgacggcgacaactggtacaggtgcgagtgcgcccccggcttcgcgggcccggactgccggattaatatcaacgagtgccagagcagcccctgcgccttcggggccacctgcgtcgacgaaatcaacgggtaccggtgcgtgtgcccccccggccacagcggggcaaagtgccaggaagtcagcggcaggccctgcatcaccatgggcagcgtcattcccgatggcgcaaagtgggacgacgactgcaacacttgccagtgcctgaatggcaggatcgcctgcagcaaggtgtggtgcggcccaaggccctgcctgctgcacaaaggccacagcgaatgcccaagcggtcagagctgcatccccatcctggatgaccagtgcttcgtgcacccctgcaccggggtcggtgagtgtaggagcagcagcctgcagcccgtgaagaccaagtgcacctccgattcctactaccaggacaattgcgccaacataacttttaccttcaacaaggagatgatgagccccggcctcaccacggagcacatctgcagcgagctgcgcaacctcaacatcctgaagaacgtgagcgccgagtacagcatttacatcgcctgcgagcccagcccctccgccaacaacgagatccacgtggccatcagcgccgaggacataagggatgacgggaatcccatcaaggagatcaccgacaagatcatcgacctggtgtccaagcgggacggcaatagcagcctgatcgccgccgtcgcggaggtgcgggtgcagaggcgcccgctgaagaaccggaccgacttcctcgtgcccctgctgagcagcgtgctgacggtggcctggatctgctgcctggtgacagccttctactggtgcctgcggaagaggaggaagcccgggagccacacccatagcgcgtccgaggacaacacgacaaacaacgtcagagagcagctgaaccaaatcaagaatcccatcgaaaaacacggcgccaacaccgtgcccatcaaagattacgagaacaagaacagcaagatgagcaaaatccggacccacaactcggaggtggaggaggacgacatggacaagcaccaacagaaggcccgctttgccaagcagcccgcctacaccctggtggaccgggaggaaaagccgccgaatggtacaccgaccaagcatcccaattggacaaacaagcaggataacagggacctggaaagcgcccagagcctgaaccggatggagtacatcgta

SEQ ID NO: 14 - DNA, 3654 bp, Artificial Sequence
  Synthetic polynucleotide
atgaggagccccaggaccagggggaggagcgggaggccgctgagcctgctcctggccctgctgtgtgccctgcgcgccaaggtgtgcggcgcgtccggacagtttgagctggagatcctgtccatgcagaacgtgaacggcgagctccagaacgggaactgctgcgggggcgcaaggaaccccggtgacaggaagtgcacccgcgacgagtgcgacacgtactttaaggtgtgcctgaaagagtaccagagcagggtgactgccggcggaccctgctcgtttggaagcggcagcactcctgtgatcggtggcaacaccttcaatctgaaggcctccagggggaacgataggaacaggatcgtgctgccattcagctttgcctggccccggtcatacaccctgctggtggaggcctgggactccagcaacgacaccgtgcagcccgactccatcatagagaaggcgagccacagcggcatgatcaacccctccaggcagtggcagaccctcaagcagaacaccggcgtcgcccacttcgaataccagatcagggtcacgtgcgacgactactactacggctttggctgcaataagttctgcaggccccgggacgacttcttcgggcactacgcctgcgaccagaacgggaacaaaacctgtatggaggggtggatgggccccgaatgcaaccgagccatctgccgccaggggtgctcccccaagcacggctcctgtaaactccccggcgattgcaggtgtcagtacggctggcagggtctctactgcgacaagtgcatcccgcaccccggctgcgtccacggcatctgtaatgagccctggcaatgcctgtgcgagaccaactggggcggccagctgtgcgacaaggacctcaattattgtggcacccaccagccatgcctgaatggtggcacctgcagcaacacaggcccagacaagtaccagtgcagctgtcccgagggctactcgggccccaactgcgaaatcgccgagcacgcttgcctgagcgacccctgtcacaacaggggcagctgcaaggaaaccagcctggggttcgagtgcgagtgcagccccgggtggaccggccccacctgcagcaccaacatcgacgactgcagccccaacaactgtagccatggcggcacctgccaggatctggtcaacggcttcaagtgcgtgtgtcccccccagtggaccggcaagacctgccagctcgacgccaacgagtgtgaagcaaagccctgcgtgaatgccaagtcctgcaagaacctgatagcctcctactactgcgactgcctgcccggctggatgggccagaactgtgacatcaacatcaacgactgcctggggcagtgtcagaatgacgccagctgccgcgacctggtgaatggctataggtgcatctgcccccccggatacgccggcgaccactgcgagagggatatcgatgagtgcgccagcaacccttgcctgaacggcgggcactgccagaacgagattaacaggttccagtgcctgtgccccaccggcttcagcggcaatctgtgccagctggatatcgactactgcgagcccaacccgtgccagaacggcgcccagtgctacaacagggcctccgactacttctgtaagtgtcccgaggactatgagggcaagaactgttcccacctgaaagaccactgcaggaccaccccctgcgaggtgatcgactcgtgcaccgtggccatggcgagcaatgacaccccggaaggcgtgcgctatatcagcagcaatgtgtgcgggccccacggcaagtgcaagagccagagcggcgggaagttcacctgcgactgcaacaagggcttcaccggcacgtactgccacgagaacatcaacgattgcgagtccaacccctgccggaacggcggcacctgcatagatggagtgaactcctataagtgcatctgctccgatgggtgggagggcgcctactgtgaaaccaacatcaacgactgcagccagaacccctgccataatggtggcacgtgccgggacctggttaatgacttctactgcgactgcaagaacggctggaagggcaagacctgccacagcagagatagccagtgcgacgaggccacgtgcaacaatggcgggacctgctacgacgagggggacgccttcaaatgcatgtgccccggcggatgggaggggaccacctgcaacatcgccaggaactccagctgcctgcccaacccgtgccataacggtggcacctgcgtggtgaacggcgaaagcttcacctgcgtgtgcaaggagggctgggagggccccatctgcgcccagaacaccaatgactgctccccccacccatgctacaactccgggacctgtgtggacggcgacaactggtataggtgcgagtgtgcccccggcttcgccggccccgactgcaggatcaacatcaacgaatgtcagagctccccctgcgcctttggcgccacatgtgtcgatgagattaacggctaccggtgcgtctgcccccccggccacagcggcgcgaagtgccaggaagtctccggcaggccctgtatcaccatgggcagcgtgatccccgacggcgccaagtgggacgacgactgcaacacctgtcaatgcctgaatggcaggatcgcctgcagcaaagtctggtgcgggccccggccctgcctgctgcacaagggccacagcgagtgcccttccggccagagctgcatcccgatcctggacgatcagtgttttgtccatccatgcaccggcgtgggcgagtgtaggtcgagcagcctgcagcccgtgaaaacaaagtgcaccagcgacagctactaccaggataactgtgccaacatcacctttaccttcaacaaggagatgatgagccccggactgaccaccgagcatatctgttcagagctgaggaacctgaacatcctcaagaacgtcagcgccgagtacagcatctacatcgcctgcgagcccagcccctccgccaacaacgaaatccacgtggccataagcgccgaggacatcagggacgacggcaatccgatcaaggagataaccgacaagatcatcgacctcgtgagtaagagggacgggaacagtagcctcatcgccgccgtcgccgaggtgagggtgcagcggaggcccctgaagaacaggaccgattttctggtccccctgctgagctccgtgctgaccgtggcctggatctgctgcctggtgacggcgttctactggtgcctccggaaacgacggaagcccgggagccatacccactccgccagcgaggacaacaccaccaataacgtgagggagcagctgaatcagatcaagaatccgatcgagaagcacggcgccaacaccgtgccgatcaaagactacgagaacaagaattccaagatgagcaagatcaggacccacaactccgaggtggaggaagatgacatggacaagcaccagcagaaagccaggtttgccaagcagcccgcctataccctggtggacagggaggagaaacccccgaatggcacccccaccaaacacccaaactggaccaacaagcaggacaacagggatctggagagcgcccagagcctcaaccgtatggagtacatcgtg

SEQ ID NO: 15 - DNA, 3654 bp, Artificial Sequence
  Synthetic polynucleotide
atgaggtcaccccggacccggggacgctccggcaggcccctgagcctgctgctggccctgctgtgcgccctcagggccaaggtctgcggcgcctccggtcagttcgaactcgagatcctgagcatgcagaacgtgaacggtgaactgcagaacggcaactgctgcggcggcgccaggaatcccggcgaccgaaagtgcaccagggacgagtgcgacacctactttaaggtgtgcctaaaggagtaccagagccgggtgacggccggcggcccctgttccttcggcagcggcagcacgcccgtgatcggcggcaacaccttcaacctcaaggcctcgcgcggcaacgatcggaacaggatcgtgctgccgttttcctttgcctggcccaggtcgtacaccctgctggtggaggcctgggacagctccaatgacaccgtgcagccagactccataatcgagaaggccagccacagcgggatgattaatccaagcaggcagtggcaaaccctgaagcagaacaccggagtggcccatttcgagtaccagatcagggtgacctgcgacgactactactacggcttcggatgcaacaagttctgcaggccccgggacgacttcttcggccattacgcctgcgaccagaacggcaacaagacctgcatggagggttggatgggccccgaatgcaatagggccatctgcaggcaaggctgttcccccaaacacgggagctgtaaactccccggcgactgccgatgccagtacgggtggcaaggcctctactgcgacaagtgcatcccccatcccggctgcgtgcatggcatttgcaacgaaccctggcaatgcctctgcgagaccaactgggggggccagctctgcgacaaggatctgaactactgcggcacacaccagccttgcctgaacggagggacctgcagtaataccggccccgacaagtaccagtgcagctgccccgagggctatagcggccccaactgcgaaattgccgagcacgcctgcctgagcgacccctgtcacaacaggggcagctgcaaggagaccagtctgggcttcgagtgcgagtgcagcccaggctggacgggccccacctgctccaccaacatcgacgactgctcccccaacaattgcagccacggcggcacctgccaagatctcgtgaacggcttcaagtgcgtgtgtccgccgcagtggaccgggaaaacctgccaactggacgccaacgagtgtgaggcaaagccctgcgtgaacgcgaagtcctgtaagaacctgatcgccagctactattgcgactgcctgccgggctggatggggcagaactgtgacatcaacatcaacgattgcctgggccagtgtcagaacgacgccagctgcagggacctggtcaacggctacaggtgcatctgtcccccggggtatgccggggaccactgcgaacgagatatcgacgagtgcgcctcgaacccttgcctcaatggcggccactgccagaacgagatcaacaggttccagtgcctgtgccccaccggcttcagcggcaatctgtgccagctggacatcgactattgtgaacccaacccgtgccagaacggcgcccagtgctacaaccgcgcctccgactacttctgcaagtgcccggaggactacgagggcaagaactgcagccatctgaaggaccactgtagaaccacgccctgcgaggtgatcgactcctgcaccgtcgccatggcctcaaacgacacccccgagggagtgcgctacatcagctcgaacgtgtgcggcccccatggaaaatgcaagagccagtccgggggcaagttcacctgcgactgcaacaagggcttcaccggcacgtattgccatgagaacatcaatgactgcgagagcaacccgtgccgtaacgggggcacctgtatcgatggcgtgaacagctacaagtgcatctgtagcgacggctgggagggcgcctattgcgaaaccaacatcaacgactgttcccagaacccatgccacaacgggggcacctgtagggacctggtcaacgacttttactgtgactgcaagaacggttggaaaggcaagacctgccactcgagggacagccagtgtgacgaggccacgtgcaacaatggcggcacctgttacgacgagggcgacgcctttaagtgcatgtgtcccgggggttgggagggtaccacctgtaacatcgccaggaactcaagctgcctgcccaatccctgccataacggtgggacctgcgtggtgaacggcgaaagcttcacctgcgtgtgcaaggagggctgggagggccccatctgtgcccagaacaccaatgactgcagcccccacccctgttacaacagcgggacctgcgtggatggtgacaactggtacaggtgtgagtgcgcccccgggtttgccggccccgactgcaggatcaacatcaacgagtgccagagcagcccctgtgccttcggcgccacctgcgtggacgagatcaacgggtaccggtgcgtgtgcccccccggccactccggcgccaagtgccaggaggtgtccggcaggccctgcatcaccatgggcagcgtcatccccgacggcgccaaatgggacgacgactgcaacacctgtcagtgcctgaacggcaggatcgcctgctccaaggtttggtgcgggcccaggccctgcctgctgcacaagggacatagcgaatgccccagcggccagagctgcatccccatcctggacgaccagtgcttcgtgcatccctgcaccggggtgggcgagtgccggagctcctcgctgcaacccgtcaagaccaagtgcacctcggacagctattaccaggacaactgcgccaacatcaccttcaccttcaacaaggaaatgatgagccccggcctgaccaccgagcatatctgcagcgagctgcggaacctgaacatactgaagaacgttagcgccgagtactccatctacatcgcctgcgagcccagcccgagcgcgaataatgagatccacgtcgccatcagcgccgaggacatccgggacgacggcaaccccatcaaggagatcaccgacaagatcatcgacctggtcagcaagcgtgacggcaactccagcctgatcgccgcggtggctgaggtgcgagtccagaggaggcccctgaagaacaggacggacttcctcgtccctctgctgagcagcgtgctgaccgtggcctggatctgttgcctggtgaccgccttttactggtgcctgcgaaagaggaggaagccgggcagccacacccacagcgcctcagaagacaacaccacaaacaacgtccgcgagcagctcaaccagatcaaaaaccccatcgaaaagcacggcgccaacaccgtgcccatcaaggactacgagaacaagaatagcaagatgagcaagatccgcactcacaacagcgaggtggaggaggacgacatggacaagcaccagcagaaggccaggtttgccaagcagcccgcctacaccctggtggaccgggaggagaagccgcccaatggcacccccacgaagcacccgaactggaccaacaaacaggacaacagggacctggagagcgcccagagcctgaaccgcatggagtacatcgtg

SEQ ID NO: 16 - DNA, 3654 bp, Artificial Sequence
  Synthetic polynucleotide
atgcggtcccccaggaccagggggcgcagcgggaggcccctgagcctgctgctggccttactgtgtgccctgagggccaaggtgtgcggcgccagcgggcagttcgagctggagatactgtccatgcaaaacgtgaacggcgaactgcagaatgggaattgctgcggtggcgccaggaaccctggggaccgcaagtgtacccgggacgagtgcgacacctacttcaaggtgtgtctcaaggaatatcagtcccgcgtgaccgccgggggcccctgcagcttcggctcaggcagcaccccagtcatcgggggcaacaccttcaacctgaaggccagccgtggcaacgacaggaacaggatagtgctgcccttctccttcgcgtggcccaggtcctacaccctgctggtggaggcgtgggatagctcgaatgataccgtccagcccgactccatcatcgagaaagcctcccactccggtatgatcaatccaagcaggcagtggcagaccctgaagcagaacacgggcgtggcccactttgagtaccagatcagggtcacctgcgacgactactactacggcttcggctgtaataaattttgccggcctcgggacgacttcttcggccactacgcctgcgaccagaacggcaataagacgtgtatggagggctggatgggcccggagtgtaatagggccatctgccgacaggggtgcagccccaagcacggcagctgcaagctgcccggcgactgcaggtgtcagtacggctggcaaggactgtattgtgacaagtgcattccccatccgggctgtgtgcacggaatctgcaatgagccctggcagtgcctgtgcgagaccaactggggcggccagctgtgtgacaaggatctgaactactgtggcacccaccagccctgcctgaacggcgggacctgctccaataccgggcccgacaagtaccagtgttcctgccccgagggctacagcggtccaaactgcgagatcgccgagcacgcctgcctgagcgacccctgccataacaggggctcctgcaaggagaccagcctgggcttcgaatgcgagtgctcccccgggtggaccggccccacctgcagtaccaacatcgatgactgcagccccaataactgttcccacggcggcacctgccaggacctggtgaacggcttcaaatgcgtctgtccgccccagtggaccggaaagacctgtcagctcgacgcaaacgagtgcgaggccaagccctgcgtgaacgccaagagctgcaagaatctgatcgcctcctactactgcgattgtctgcccggatggatgggccaaaactgcgacatcaacatcaacgattgtctggggcagtgccagaacgacgccagctgcagggacctggtcaacggctacaggtgcatctgcccccccggctatgccggagaccattgcgagcgagacatcgacgagtgtgcctcgaacccctgcctgaacggggggcactgccagaacgaaatcaacaggttccaatgcctctgccccaccgggttcagcggcaacctgtgccagctggacatcgactattgcgagcccaacccctgccagaacggggcgcagtgttataaccgggcctcggactacttctgtaagtgtcccgaggactacgagggcaaaaactgctcccacctgaaggaccactgccgtaccacaccctgcgaagtcatcgactcctgcaccgtggccatggccagcaacgacacccccgagggagtgcggtacatcagcagcaacgtgtgcgggccgcatggcaagtgtaagtcccagagcgggggcaagtttacatgtgactgtaacaagggcttcaccggcacatactgccacgagaacatcaacgattgcgagagcaacccctgccggaatgggggcacctgcatcgacggggtgaacagctataagtgtatctgctccgatggctgggagggcgcctactgcgagactaacatcaatgactgctcgcagaacccgtgccacaacgggggaacctgcagggatctcgtgaacgacttctactgcgactgcaagaacgggtggaaggggaagacctgccacagccgcgactcccagtgcgacgaggccacctgcaacaatgggggcacctgctacgacgagggcgacgccttcaagtgcatgtgccccggcgggtgggagggcaccacctgcaacatcgcccggaactccagctgcctgcccaatccgtgtcacaatgggggcacctgcgtggtgaacggcgagtcgttcacgtgcgtgtgcaaggaaggctgggagggaccgatctgcgcccaaaataccaacgactgtagcccccacccctgttataacagcggcacctgcgtcgacggggacaattggtaccggtgcgagtgcgcccccggcttcgccggccccgactgccgaatcaacatcaacgaatgtcaaagctcaccctgtgccttcggggcaacctgtgtggacgagatcaacggctaccggtgtgtgtgccccccgggacactccggggccaagtgccaggaggtgagcgggcgaccatgcatcaccatgggctccgtgatccccgacggcgccaagtgggacgacgactgcaacacctgccagtgcctgaacggcaggatcgcctgctccaaggtgtggtgtggcccccggccctgtctcctgcacaaaggtcacagcgagtgccccagcggccagagctgcatcccgatccttgacgaccagtgcttcgtgcacccgtgtacaggcgtaggggagtgcaggagctcctcgctccagcccgtgaaaaccaagtgtaccagcgactcatactatcaggacaactgtgccaatatcacctttaccttcaacaaggaaatgatgagccccgggctgaccaccgagcacatctgcagcgagctgcggaaccttaacattctgaaaaatgtgtccgccgagtacagcatatacatcgcctgcgagccgagccctagcgccaacaatgagatacacgtggccatcagcgctgaggacatcagggatgacggcaacccgatcaaggagatcaccgacaagataatagacctcgtcagcaaaagggacggcaacagcagcctgatcgccgccgtcgccgaggtgagggtgcagcgccggcccctgaagaacaggaccgacttcctggtgcccctcctgagctccgtgctgaccgtggcctggatctgctgcctggtgaccgccttctactggtgtctgaggaaaaggaggaagcctggcagccacacccatagcgcctccgaggacaataccaccaacaacgtcagggaacagctcaaccaaatcaagaaccccatcgagaagcacggcgccaataccgtgcccatcaaggattacgagaacaagaatagcaagatgtccaagatccgcacacataattccgaggtcgaggaagacgacatggataagcaccagcagaaggccagattcgccaagcagcccgcctacaccctggtggacagggaggagaagccccccaacggcacacccaccaagcatcccaactggaccaacaagcaggacaacagggacctggagagcgcccagtccctgaaccgtatggagtacatcgtc

SEQ ID NO: 17 - DNA, 3654 bp, Artificial Sequence
  Synthetic polynucleotide
atgaggagccccaggacaaggggccggagcggcaggcccctgagcctgctgctcgccctcctctgtgccctgcgcgccaaagtgtgcggggcctcaggccagttcgagctcgagatcctgtccatgcaaaacgtgaacggcgaactgcagaacggaaattgctgcggtggcgcccgtaaccccggcgaccgcaagtgcaccagggacgagtgcgacacctacttcaaggtgtgtctgaaggagtaccagagcagggtcaccgccggcggcccctgcagctttggctccggcagcacccccgtgatcggcggcaacaccttcaacctgaaggctagccgcggcaacgacaggaacaggatcgtgcttccatttagcttcgcctggcccaggagctacaccctgcttgtggaggcctgggacagctccaacgacaccgtgcagcccgacagcatcatcgagaaggccagccactccggcatgatcaaccccagccggcagtggcagaccctgaagcagaacaccggcgtcgcgcacttcgagtaccagatcagggtgacatgtgacgactattactatggctttggatgtaacaagttctgcaggcccagagacgacttcttcggccactacgcctgcgaccagaacggaaataagacctgtatggaaggctggatggggcccgagtgcaaccgagccatctgcaggcaaggctgcagccccaagcacggcagctgcaagctgcccggggactgccggtgccagtacggctggcagggcttgtattgcgacaagtgcatcccgcaccccggctgcgtgcacgggatctgcaacgagccctggcagtgcctgtgcgagacgaactggggcggccagctgtgcgacaaggacctgaactactgcgggacgcatcaaccctgtctcaacggcggtacctgcagcaataccggccccgacaagtaccagtgctcttgccccgagggctatagcgggcccaactgtgagatcgccgagcacgcttgcctgtccgacccctgccacaaccggggctcctgcaaggagacctccctgggcttcgagtgcgaatgcagccccgggtggaccggtcccacgtgcagcaccaacatcgatgactgtagccccaacaactgcagccacggcggcacgtgccaggacctcgtgaacggcttcaagtgcgtgtgccccccccagtggaccggcaagacctgccagctcgacgccaatgagtgcgaagccaagccctgcgtcaacgccaagtcctgcaagaacctgatcgccagttactactgcgactgtctgcccggatggatgggccagaattgcgacatcaacatcaatgactgcctgggccagtgccagaatgacgcgtcctgtagggatctggtgaacgggtacaggtgcatatgtccccccggctatgccggggatcactgcgagagggatatcgatgagtgcgccagcaacccctgtctgaacggtggccactgccagaacgagattaacaggttccagtgcctgtgccccaccggcttcagcggcaacctgtgccagctggatatcgactactgtgagcccaacccgtgccagaacggcgcccagtgctacaaccgagccagcgattatttttgcaaatgtcccgaggattacgaagggaagaattgcagccacctgaaggaccattgcaggaccaccccctgcgaagtgatcgacagctgcaccgtggccatggcctcgaatgacacgcccgagggagtgaggtacatcagtagcaatgtgtgcggcccccatgggaagtgcaagagccagtcgggcggaaagtttacctgcgactgtaacaagggcttcaccgggacctactgtcacgaaaacatcaacgactgcgagtccaacccgtgtaggaacggcgggacctgcatagacggggtgaatagctataagtgcatctgttcagacggatgggagggggcctactgcgagaccaacatcaacgattgctcgcagaacccctgccacaacggcggcacctgccgggacctggtgaacgacttctactgcgactgtaaaaacggctggaaggggaagacctgccactccagggacagccagtgcgacgaggcgacctgcaacaacggcggcacctgctacgacgagggcgatgccttcaagtgtatgtgccccggaggctgggagggcaccacctgcaacatcgcccgcaacagcagctgcctgcccaatccctgccacaatggtggaacatgcgtggtgaacggggagagctttacgtgcgtgtgcaaggagggatgggagggccccatctgtgcccagaacaccaacgactgctccccccatccctgttacaacagcggcacctgtgtggacggggacaactggtaccgctgcgagtgcgcccccggcttcgccggcccggactgccgtatcaacatcaacgagtgtcagagcagcccctgcgcattcggcgccacctgcgtggatgaaataaacggctacaggtgtgtgtgcccccccggccacagcggagccaaatgccaggaggtgagcgggcgcccatgcatcaccatggggagcgtgatcccagacggggcgaagtgggatgacgactgtaacacctgccagtgcctgaacggccgaatcgcctgcagcaaggtgtggtgcgggccccggccctgcctgctgcacaaaggccacagcgagtgccccagcggccagagctgcataccgatcctggacgaccagtgcttcgtacacccctgcaccggggtgggcgagtgccggtcctcctcgctccagcccgtcaagaccaagtgcaccagcgatagctactaccaggacaactgcgccaacatcacctttacctttaacaaggagatgatgagccccggcctgaccacggagcacatctgcagcgagctgcgcaacctcaacatcctgaaaaacgtgtcggccgagtactccatctacatcgcctgcgagccctccccctccgccaacaatgaaatccacgtggccatcagcgccgaggacatccgagacgatgggaaccccatcaaggaaatcaccgacaagataatcgacctggtgagtaaaagggacgggaacagcagcctgatcgctgccgtggcggaggtgagggtccagaggaggccgctgaaaaatcggaccgactttctggtgcccctgctgagctccgtgctgaccgtcgcctggatctgctgcctggtcaccgccttctactggtgcctgaggaagcgtaggaagcccggcagccacacgcacagcgccagcgaggacaacaccaccaacaacgtgcgggagcagctgaaccagatcaagaaccccatcgagaagcacggcgcgaacacagtgccgatcaaggattacgagaacaagaattccaagatgagcaagatcaggacccacaacagcgaggtggaggaggacgacatggataaacaccagcagaaggccaggttcgccaagcagcccgcctataccctggtcgacagggaggagaaaccccctaatggcacccccaccaagcaccccaactggacaaacaagcaggacaacagggacctggagagcgcccagagcctgaaccgtatggagtatatcgtg

SEQ ID NO: 18 - DNA, 3654 bp, Artificial Sequence
  Synthetic polynucleotide
atgcggagccccagaacccgtggccggagcggcaggcccctgtcactactgctggccctgctgtgcgcgcttagggccaaggtctgcggcgccagcggccagttcgagctggagatcctgagcatgcagaacgtgaacggcgagctgcagaacggcaactgctgcggcggggccaggaaccccggagaccgcaaatgcacccgggacgagtgcgacacctattttaaagtgtgcctgaaggagtaccagagcagggtgaccgccggcggcccctgcagcttcggcagcggcagcacccccgtgatcggcgggaataccttcaacctgaaggccagccgcggcaacgacaggaaccgaatcgtgctgccctttagcttcgcctggcctcggagctacaccctgctggtggaagcctgggactcctccaacgacaccgtgcaacccgactccattatcgagaaggcctcccacagcggcatgataaaccccagccggcagtggcagacactgaagcaaaacaccggggtcgcacatttcgagtaccagatcagggtgacgtgtgacgactactactacgggttcggatgcaacaagttctgcaggcccagggacgacttcttcggccactacgcctgtgaccagaacggcaataagacctgcatggaggggtggatgggcccggagtgcaacagggccatatgccggcagggctgctccccaaaacacgggtcctgcaagctgcctggcgactgcaggtgtcagtacggctggcaggggctgtactgcgataagtgcatcccccaccccggctgcgtccacggcatctgcaacgagccatggcagtgtctgtgcgagaccaactggggtgggcagctgtgcgacaaggatctgaactactgcggcacccaccagccctgcctcaacgggggaacgtgctcgaacaccgggcccgataagtaccagtgctcctgccccgaaggctactcgggacctaactgtgagatcgctgagcacgcatgcctgagcgacccatgccataacaggggtagttgcaaggagacctccctcggttttgaatgcgagtgcagccccggctggaccggccccacctgctcgaccaacatcgacgactgcagcccaaacaactgctcccacggcggcacgtgtcaggacctggtgaatggcttcaagtgtgtgtgccccccccagtggaccggaaaaacctgccagctggatgccaacgagtgtgaggccaagccctgcgtgaacgcgaagtcctgcaagaacctgatcgcctcctactactgtgactgcctgcccggttggatgggccaaaactgcgacatcaacatcaacgactgcctgggccagtgccagaacgacgccagctgcagggacctagtgaacgggtatcggtgcatctgcccccccggctacgccggcgatcactgcgaaagggacatcgacgagtgcgccagcaacccgtgcctgaacggggggcactgccagaacgagatcaacaggttccagtgcctctgccccaccgggttcagcgggaacctctgccagctcgacatcgactactgcgagcccaatccctgccagaacggcgcgcaatgctacaatagggcctcggactacttctgcaagtgccccgaggactacgagggcaaaaactgcagccacctgaaggaccactgtaggacaaccccctgcgaagtcatcgactcctgcaccgtggccatggcctccaacgacaccccagaaggcgtacgttacatcagctccaacgtctgcgggccccacgggaagtgcaagagccagagcggcggcaagttcacgtgtgactgcaacaaagggttcaccggcacctactgccatgagaacataaatgactgcgagtccaacccctgtcggaacggcggcacctgcatcgacggcgtaaactcttacaaatgtatctgcagcgacggctgggagggcgcctactgcgagaccaacatcaacgactgcagccaaaacccctgtcacaacggcgggacctgccgcgacctcgtcaacgacttctactgcgactgcaagaacggctggaagggcaagacctgccacagccgggactcgcagtgtgatgaggccacctgcaacaatggcggcacctgctatgatgagggggacgccttcaaatgtatgtgccccggcgggtgggagggcaccacttgcaacatcgccaggaactcctcctgcctccccaacccctgccacaacggagggacgtgcgtggtgaacggggagagcttcacctgcgtgtgcaaggagggctgggaaggccccatttgcgcgcagaacactaacgattgcagcccccacccctgctacaactccggcacctgcgtggacggggacaactggtaccggtgcgagtgcgcccccggcttcgccggcccggactgcaggatcaacatcaacgaatgtcagagcagcccctgcgccttcggagccacctgcgtggacgagataaacggctaccggtgcgtctgcccccccggtcactctggtgccaagtgccaagaggtcagcggcaggccgtgcatcaccatgggctccgtgatcccggatggcgccaaatgggacgatgactgcaacacctgccagtgccttaacggtcggatcgcgtgcagcaaggtgtggtgtggccccaggccctgcctcctgcacaaggggcacagcgagtgcccctccggacagtcctgtatccccatcctggacgaccagtgcttcgtccacccctgcaccggagtgggcgaatgcaggagcagctccctgcagccggtgaagaccaagtgcaccagcgactcctactaccaggacaattgcgccaacatcaccttcaccttcaacaaggagatgatgagccccggcctgaccaccgagcacatctgcagcgagctgcgcaacctgaacatcttgaagaacgtgagcgccgagtattccatctacatcgcctgcgagcccagcccgagcgccaataacgagatccacgtggccatcagcgccgaggacatccgggatgacggcaatcccatcaaggagatcaccgataagatcatcgacctggtcagcaagcgcgacggcaatagctcgctgatcgcggccgtggccgaggtgagggtgcagcggcggcccctgaagaacaggaccgactttctggtacccctcctgagctcggtgctgaccgttgcctggatctgttgtctggtgaccgccttctactggtgcctgcggaaaaggcggaagcccggctcccatacccatagcgcatccgaagacaacaccaccaacaacgtccgtgagcagctgaaccagatcaagaaccccatagagaaacacggcgccaacaccgtgcccatcaaggactacgaaaacaagaactccaagatgtccaaaatcaggacccacaacagcgaggtggaagaggacgacatggataaacaccagcagaaggcccgtttcgccaagcagcccgcctacaccttagtggacagggaggagaaaccccccaacgggacccccaccaagcacccaaactggacgaacaagcaggataaccgggacctggaatcagcgcagtccctgaacagaatggaatacatcgtc

SEQ ID NO: 19 - DNA, 3654 bp, Artificial Sequence
  Synthetic polynucleotide
atgaggtccccccgaaccaggggcaggtccggtcggcccctgagcctgctcctggccctcctgtgcgccctgagagccaaggtgtgtggagccagcgggcagttcgagctcgagatcctctccatgcagaacgtgaacggcgagctgcagaacggcaactgctgcggaggcgccaggaatcccggcgatcggaagtgcaccagggacgagtgcgacacctatttcaaggtgtgcctcaaggagtaccaaagcagggtgaccgccggcggcccctgctccttcggcagcggcagcacccccgtgatagggggcaacacgttcaacctcaaggccagcaggggcaacgacaggaaccgcatcgtgctgcccttcagctttgcgtggccccgttcctacaccctgctggtcgaggcctgggacagctccaacgataccgtgcagcccgactccatcattgagaaggccagccacagcggcatgatcaaccccagcaggcagtggcaaaccctgaagcagaacaccggagtggcccatttcgaataccagatcagggtgacctgcgatgactactattatggttttgggtgcaacaaattctgccggccccgagacgacttcttcggtcactatgcctgcgaccagaacggcaacaagacctgtatggaggggtggatgggccctgagtgcaaccgggccatctgtcgccaggggtgctcccccaagcacggcagctgcaagctgcctggcgattgccggtgtcagtacgggtggcagggtctctactgcgacaagtgcatcccccacccgggctgtgtgcacggcatctgcaacgagccctggcagtgcctgtgcgaaaccaattggggcggccaactgtgcgacaaggacctgaactactgtggcacccaccagccctgcctgaacgggggcacttgctccaacacgggccccgacaagtatcagtgcagctgtcctgagggctacagcggccccaactgtgagatcgccgagcatgcctgcctgagcgacccgtgccacaatcgtggcagctgtaaggagaccagcctgggcttcgagtgcgagtgcagcccgggttggaccggacccacctgcagcaccaacatcgacgattgcagccccaacaactgttcacacgggggcacgtgccaagacctggtgaacgggttcaagtgtgtctgccccccccagtggaccggcaaaacctgtcagctcgacgccaacgaatgtgaggccaagccctgcgtgaatgcgaagagctgcaagaacctgatcgcgtcgtactattgcgattgcctgcccggctggatgggccagaactgcgacatcaacatcaacgactgcctgggccagtgccaaaacgacgcctcttgccgcgatctggtcaacgggtaccgctgcatctgccctccggggtacgccggggatcactgtgagagggacatagatgagtgcgcgtccaacccctgcctgaacggggggcactgccagaacgagatcaacaggtttcagtgcctgtgccccaccggcttctccggcaacctgtgccagcttgacatcgactactgcgagcccaatccctgccagaatggcgcccagtgctacaacagggccagcgactatttctgcaagtgtcccgaggactacgaggggaagaattgctcccacctgaaagaccactgcaggacgaccccctgtgaggtgatcgacagctgcaccgtggccatggcctccaacgacacccccgagggcgtgaggtacatcagcagcaacgtctgcggcccccacggcaagtgcaagagccagagcggcggaaagttcacctgcgactgcaacaaggggttcacgggcacctactgccacgagaacatcaacgactgcgagtccaacccctgcaggaacggcggcacgtgcatagacggggttaacagctataagtgtatctgctcggacgggtgggaaggcgcctactgcgagaccaacatcaacgactgctcacagaatccgtgccacaacgggggcacctgcagggacctggtgaacgacttctattgcgactgcaagaacggctggaaaggtaagacatgccactcccgggactcccagtgcgacgaggccacctgcaacaacggaggaacctgctacgatgagggcgacgccttcaagtgcatgtgccccgggggatgggaaggcaccacctgcaacatcgccaggaactccagctgtctccccaacccgtgccacaacggcgggacgtgcgtggtgaatggcgagtccttcacgtgcgtgtgcaaggagggctgggagggccccatctgcgcgcagaacaccaacgattgcagcccccacccgtgctacaactcaggcacctgcgtcgacggtgacaactggtaccggtgcgagtgcgccccagggttcgcgggccccgactgcaggatcaacatcaacgagtgccagtccagcccctgcgcctttggcgccacctgcgtggacgagatcaacggctacaggtgcgtgtgcccccccggccatagcggcgccaagtgccaggaggtgagcggcaggccctgcatcaccatgggcagcgtgatccccgacggcgccaagtgggacgacgactgcaatacgtgccagtgcctgaacggacgcattgcctgctccaaggtgtggtgcggcccccggccgtgcctgctccacaaggggcacagcgagtgcccctccggccagagctgcatccccatcctcgacgaccagtgcttcgtccacccctgcaccggcgtgggcgagtgcaggtcctccagcctgcagccagtgaaaaccaagtgtaccagcgactcctactaccaggacaactgcgccaacatcacattcacattcaacaaggagatgatgagcccgggcctgaccaccgagcacatctgcagcgaactcagaaacctgaacatcctgaagaacgtgtcggccgagtacagcatctatatcgcgtgcgagcccagccccagcgcgaataacgagatccacgtggccataagcgcggaggacatccgggacgacggcaaccccatcaaggagatcaccgacaagattattgacctggtctccaagagggacggcaatagctccctgattgccgccgtcgccgaagtgcgggtgcaaagaaggcccctgaaaaaccggacggatttcctggtccccctcctgagcagcgtgctgaccgtcgcctggatctgctgtctggtgacggccttctactggtgcctcagaaagaggcgcaaacccggctcgcacacccatagcgcctcagaggacaacaccacgaataacgtgcgggaacagctgaaccaaataaaaaaccccatcgagaagcacggggctaacaccgtgccgatcaaggactacgagaacaagaacagcaagatgtccaagatccgaacccacaacagcgaggtcgaggaggacgacatggacaagcaccagcagaaggcgaggttcgccaagcagcccgcctacaccctggtagaccgggaggagaagccgcccaacggcacccccacgaaacaccccaactggaccaacaaacaagacaacagggacctggagagcgcccagtccctgaacaggatggaatatattgtc

SEQ ID NO: 20 - DNA, 3654 bp, Artificial Sequence
  Synthetic polynucleotide
atgaggagccccaggacacggggccggagcgggcgacctctgtccctgctcctggccctgctgtgcgccctgagagccaaagtgtgcggcgccagcgggcagttcgagctggagatactgagcatgcagaacgtgaacggcgagctgcagaacggcaactgttgtgggggcgcgcggaaccccggggacaggaagtgcacccgggacgagtgcgacacctacttcaaggtgtgcctcaaggaataccaaagccgtgtgacagctgggggcccctgcagcttcgggtccggatccacccccgtcatcggcggcaacaccttcaacctcaaggccagcaggggcaacgacaggaaccgaatcgtgctgcccttttcgtttgcctggccccgcagctacaccctcctagtggaggcctgggacagcagcaacgacaccgtgcagcccgactccatcatcgagaaggcatcccacagcgggatgatcaatccctcccgccagtggcagacgctgaagcagaacaccggcgtggcccacttcgaataccaaatcagggtgacgtgcgatgactactattacggcttcgggtgcaacaagttctgcaggccgagggatgacttcttcggccactatgcctgcgaccagaacggaaacaaaacctgcatggagggttggatgggacccgagtgcaacagggccatctgccgccagggctgctcaccaaagcacggcagctgtaagctacccggcgactgtcggtgccagtacggttggcagggcctgtactgtgacaagtgcatcccccaccccggctgcgtgcacggcatctgcaatgagccgtggcagtgcctgtgtgaaaccaactggggtgggcagctgtgcgacaaggacctgaattactgcggcacccaccagccctgtctgaacggcggcacctgctccaacaccggcccggacaagtatcagtgcagttgccccgagggctatagcggccccaactgcgagatcgccgagcacgcctgcctgtccgacccgtgccacaacagggggagctgcaaagagaccagcctggggttcgagtgcgagtgcagccccgggtggaccggacccacctgcagcaccaacatcgatgattgcagccctaacaactgctcccacggcggcacctgccaggacctggtgaacggctttaagtgcgtatgccccccccaatggacggggaagacctgtcagctcgacgccaatgaatgcgaggcaaaaccgtgtgtgaacgccaagagctgcaaaaacctcatcgcgtcctactactgcgactgcctgcccggctggatggggcagaactgtgacatcaacatcaacgattgcctgggccaatgccagaatgatgcctcctgcagggaccttgtgaacggctacaggtgcatatgcccccccggctacgccggcgatcactgcgagcgggatatagacgagtgtgccagcaacccctgcctcaacggggggcactgccagaatgagatcaacagatttcaatgcctgtgccccacaggatttagcggaaatctgtgccaactggacatcgactactgcgagcccaatccctgccagaacggggcccagtgctacaaccgggccagcgactacttttgcaagtgccccgaggactacgagggaaaaaactgcagccacctgaaggaccattgcaggaccaccccctgtgaggtgattgacagctgcaccgtggccatggcctcaaacgacacccccgagggtgtgaggtatatcagctcgaacgtgtgcggcccccacggcaagtgcaagtcacaaagcgggggaaagttcacctgcgactgcaacaagggcttcaccggtacctactgccacgagaacatcaacgactgtgagagcaacccctgtagaaacggggggacctgcatcgacggagtgaattcctataagtgcatctgtagcgacgggtgggagggcgcctactgcgagaccaatatcaacgattgcagccagaacccctgccacaacgggggcacctgccgagatctcgtgaacgacttctactgcgactgtaaaaacggttggaaaggcaaaacctgccactcccgcgattcccagtgcgatgaggcgacctgcaataatggaggcacctgctacgacgagggcgacgcctttaagtgcatgtgccccggcggctgggaaggcaccacctgcaatatcgcgagaaatagcagctgcctgcccaacccctgccataacggcgggacctgcgtggtgaatggcgagagcttcacctgcgtctgtaaggagggctgggaaggtcccatctgtgcccagaacaccaacgactgcagcccccatccctgctacaacagcggcacctgcgtggacggcgacaattggtacaggtgcgagtgcgcccccgggtttgccggccccgactgcaggatcaacatcaacgagtgccagagtagcccctgtgccttcggcgccacctgcgtggacgagatcaacggctaccggtgcgtgtgcccccccggccactccggcgccaagtgtcaagaggtgagcggacgaccctgtatcaccatgggctcggtgatccccgacggcgccaagtgggacgacgactgcaacacgtgccagtgcctcaacgggaggatcgcctgcagcaaggtgtggtgcggtcccaggccctgcctgctgcacaaaggccactccgagtgccccagcggccagagctgtatccccatcctggatgatcagtgcttcgtccatccctgtactggcgtgggcgagtgcaggagcagcagcctccagcccgtgaaaaccaagtgcacgagcgactcctattaccaagataactgtgccaacatcaccttcacctttaacaaggagatgatgtcgcccggactgaccaccgagcatatctgcagcgagctgaggaacctgaacatactgaagaatgtgtccgccgaatattccatctacatcgcctgtgagcctagcccgagcgccaacaacgagatccacgtggccatctccgccgaggatatcagggacgacgggaaccccatcaaagagatcaccgataagatcatcgacctggtgtctaagcgcgacggtaacagctccctaatcgccgccgtggccgaggtgcgcgtgcagcgcaggccgctgaagaaccgcaccgacttcctggtgcccctgctgagcagcgtgctcaccgtggcctggatatgctgcctggtgaccgccttctactggtgcctgcggaagcggcgtaaaccgggaagccatacccacagcgccagcgaggataataccaccaataacgtgcgggagcagctgaaccagatcaagaaccccatcgaaaagcacggggcgaacaccgtgcccatcaaggactacgagaataagaactccaagatgagcaagatccgcacacacaacagcgaggtggaggaggacgatatggacaagcaccagcagaaggccaggttcgccaagcagcccgcctacacccttgtggaccgcgaagagaagcccccgaacggcacccccaccaagcaccccaactggaccaacaaacaggataaccgtgacctggaaagcgcgcagtccctgaaccgcatggagtacatagtg

SEQ ID NO: 21 - DNA, 3654 bp, Artificial Sequence
  Synthetic polynucleotide
atgaggagcccccggaccagggggcggagcggcaggcccctgagcctcctgctggccctgctttgcgcactgagggccaaggtgtgtggggccagcgggcagttcgagctcgaaatcctgagcatgcagaacgtgaacggcgagctgcagaatggcaattgttgcggcggcgccaggaaccccggcgaccggaagtgcacccgggacgaatgcgacacctacttcaaggtgtgcctcaaggagtaccagagccgcgtgaccgccggcggaccctgcagcttcggcagcggcagcacccccgtgatcgggggcaacaccttcaacctgaaggcatcccgcgggaacgacaggaacaggatcgtgctgccgttcagcttcgcctggccgcgatcctacacgctgctggttgaggcctgggacagcagcaatgacacggtgcaacccgacagcattatcgagaaggccagccactccggcatgatcaacccctcccggcagtggcagaccctgaagcagaacactggagttgcacacttcgagtaccaaatcagggtcacgtgcgacgactactattacgggttcggctgtaacaagttctgcaggccccgtgatgacttctttggacactacgcctgcgaccagaacggaaacaagacctgcatggaagggtggatgggccccgagtgcaacagggccatctgtagacaaggctgcagccccaaacacggctcctgtaagctgcccggcgactgccggtgccagtacggctggcaggggctctactgcgacaagtgcattccccatcccggctgcgtgcacggcatatgtaacgaaccctggcaatgcctctgcgagaccaactggggcgggcagctgtgcgacaaagacctgaactactgtggcacccatcagccctgcctgaacggggggacttgctccaataccggtcccgacaagtatcagtgcagctgccccgagggctactccgggcccaactgcgagatcgccgaacacgcctgtctgtccgacccctgccacaacagaggcagctgcaaggagaccagcctgggctttgagtgcgagtgctcccccggctggaccgggcccacctgcagcaccaacatcgacgattgcagccccaacaattgctcccacggcggcacttgccaagacctggtgaacggcttcaagtgcgtgtgccccccccagtggaccggtaaaacatgccagctggacgccaacgagtgcgaggccaagccctgcgtgaacgccaagagctgcaaaaacctgatcgccagttactactgcgactgcctgcctggatggatgggccagaactgcgacatcaacatcaacgactgcctgggccagtgccagaacgacgcaagctgccgtgacctggtgaacggctacaggtgcatctgcccccccgggtacgccggtgaccactgcgaacgggacatagatgagtgcgccagcaacccctgcctgaacggcggacactgccagaatgagatcaataggttccaatgcctctgccccaccggctttagcggcaatctgtgccagctggacatcgattactgtgagcccaacccctgccagaatggagcccagtgctacaaccgggcctccgactatttctgtaagtgtcccgaagactacgagggtaagaactgctcccacctgaaggaccactgccggaccactccgtgcgaggtcatcgacagctgcaccgtcgccatggccagcaatgacacacccgagggcgtgaggtacatctcctccaacgtgtgtggcccccacggcaagtgcaagagccagagcggaggcaagttcacctgcgactgcaacaaggggttcaccggcacttactgccacgagaacatcaacgactgcgaatccaacccctgtcgaaacgggggcacctgcattgacggcgtgaacagctataagtgcatctgctccgacgggtgggagggggcctactgcgaaaccaatataaacgattgcagccagaacccctgtcacaacgggggcacatgcagggacctggtcaacgacttctactgtgactgcaagaacggctggaagggcaagacatgtcacagcagggacagccagtgcgacgaggccacctgtaacaatggcggcacctgctatgacgaaggcgacgccttcaaatgtatgtgccccggcggttgggaggggacgacgtgcaatattgcgaggaactccagctgtctgcccaacccctgccacaacggaggcacctgtgtggtgaacggcgagagctttacgtgcgtctgtaaagagggctgggaaggccccatctgcgcccaaaacacgaacgactgcagcccccacccctgttacaatagcggcacctgcgtcgacggtgacaactggtataggtgcgagtgtgccccgggctttgccgggcccgactgccggatcaatatcaacgagtgccagtccagcccatgtgcgttcggcgccacctgcgtggacgaaatcaacggctacaggtgcgtctgccccccggggcacagcggagccaaatgtcaggaagtctctgggaggccctgcatcaccatgggcagcgtaatccccgacggggctaagtgggacgacgactgcaatacctgtcagtgtctgaacggcaggattgcctgcagcaaagtgtggtgtggcccgcggccctgtctcctgcacaagggccactccgagtgtcccagcggccaatcctgcatccccatcctcgacgaccagtgctttgtgcacccctgcacaggcgtgggagagtgtaggtcgagctccctgcagcccgtgaagaccaagtgcaccagcgattcctactaccaggacaactgcgcgaatatcacctttacctttaacaaggagatgatgagccccgggctgaccaccgagcacatctgcagcgagctgcggaacctgaacatcctcaaaaacgtcagcgccgagtatagcatctacattgcctgcgagcccagccccagcgccaacaacgaaatacacgtggccatcagcgccgaggacatcagggacgacggcaacccgatcaaggagatcaccgataagataatcgacctggtgtccaagagggacggcaatagctccctgatcgccgccgtggccgaagtgagggtgcagaggaggcccctgaaaaacaggaccgatttcctggttcccctgctgagcagcgtgctgacagtggcttggatctgctgcctcgtaactgcattctactggtgcctgaggaagaggaggaagcccggcagtcacacccacagcgcctccgaggataacaccactaacaatgtgcgggagcagctgaaccagatcaagaatcccatagaaaaacatggcgccaacaccgtgcccattaaagattacgagaacaaaaatagcaagatgtccaagatccgcacccacaacagcgaggtggaggaggacgacatggacaagcaccagcagaaggccaggttcgccaagcagcccgcgtacaccctggtggaccgtgaggagaagccccccaacggcacccccaccaagcaccccaactggaccaacaagcaagataatcgggacctggaatccgcccagagcctgaacaggatggagtacatcgtg

SEQ ID NO: 22 - DNA, 3654 bp, Artificial Sequence
  Synthetic polynucleotide
atgaggagcccgagaacgagggggcggtccggcaggccgctgagcctcctgctggccctgctgtgcgccctgcgggcaaaggtgtgtggcgcctccgggcagttcgagctggagatcctgagcatgcaaaacgtgaacggcgaactccagaacggcaattgctgcggcggcgccagaaaccccggggatcgaaagtgcacccgggacgagtgcgacacctacttcaaagtgtgtctcaaagaataccagagcagggtgaccgccggcgggccctgcagcttcggcagcggcagcacccccgtgatcggcgggaacaccttcaacctgaaggccagccgcggcaacgacaggaatcggatcgtgttgccgttcagcttcgcctggccccgttcctacaccctgctggtggaggcctgggacagcagcaacgataccgtgcagccagacagcataatcgagaaggccagccactccggtatgatcaaccccagcaggcagtggcagaccctgaagcaaaacaccggcgtggcccatttcgagtaccagatcagggtcacgtgcgacgactattactacgggttcgggtgcaacaagttctgcaggccccgggatgacttctttggacactacgcctgtgaccagaacggaaacaaaacttgcatggagggctggatgggcccggagtgcaatagggccatttgcaggcaaggctgcagccccaagcacggctcctgcaagctccccggcgactgccgatgccaatatggctggcagggcctctactgtgacaagtgcatcccccacccgggctgcgtccacggaatctgcaatgagccctggcagtgtctgtgcgagacgaactggggtggccagctgtgcgacaaggacctgaactactgcgggacccaccagccctgcctgaacggcgggacctgttccaacaccggcccggacaagtatcagtgcagctgcccggaagggtactccggcccgaactgcgaaatcgccgaacacgcttgcctcagcgacccctgccacaaccgcgggagctgcaaggagaccagcctgggctttgagtgcgaatgttcccccggctggaccgggcccacatgctccaccaacatagacgattgtagccccaacaactgctcccacggggggacctgccaagacctggtcaacggattcaagtgcgtgtgtcccccccagtggacgggtaagacctgccaactggacgccaacgaatgcgaggccaagccctgtgtgaatgccaagagctgcaagaacctgatcgccagctactactgtgactgcctgcccggctggatgggccagaattgcgacatcaatatcaacgactgcctgggccagtgccagaatgacgcctcctgcagggacctggtgaacggctacaggtgcatatgcccccccggctacgccggcgaccactgcgaacgtgacatcgacgagtgcgcctcaaacccctgcctgaacggcggacactgccagaacgagatcaaccgattccagtgtctgtgccccaccgggtttagcgggaacctctgccagctcgatatcgactactgcgaacccaacccctgccagaacggcgcccagtgctacaaccgggccagcgactatttctgtaaatgccccgaggactacgaggggaaaaactgtagccacctgaaggaccactgcaggaccacaccctgcgaagtgatcgacagctgcaccgtggccatggccagcaatgacacccccgaaggcgtgaggtatataagcagcaacgtatgcggcccccacggcaagtgtaagagccagagcggcggcaagtttacgtgcgactgcaacaaaggcttcaccggcacctactgtcacgagaacatcaacgactgcgagagcaacccctgccgcaacgggggcacctgcatcgacggtgtgaacagctacaagtgcatctgcagcgacggctgggagggcgcctactgtgagacgaacatcaacgactgcagccagaacccgtgccataacgggggcacctgcagggatctggtgaacgacttttattgcgactgcaagaacggctggaagggcaagacctgccacagccgggacagccagtgtgacgaggccacctgcaacaacggcggcacctgctacgacgaaggggacgcctttaagtgcatgtgcccgggcgggtgggagggcaccacctgcaacatcgccaggaattcctcctgtctgcccaacccatgtcacaacggtggcacgtgcgtggtgaacggggagtcctttacctgtgtgtgcaaggaggggtgggagggacccatatgtgcgcagaataccaacgactgctccccccacccatgttataacagcggtacatgtgtggatggggacaactggtaccggtgtgagtgcgcccccggcttcgccggccccgattgcaggatcaacatcaatgagtgccagagctccccctgcgccttcggcgccacatgcgtcgacgaaatcaacggctacaggtgtgtgtgccccccgggacacagcggtgccaagtgccaggaagtgtcaggcaggccctgtattaccatgggcagcgtgatccccgacggagccaagtgggatgacgactgcaacacctgccagtgcctgaacggccgtatcgcctgcagcaaggtgtggtgcggcccccggccgtgcctgctgcacaaggggcactccgagtgccccagcgggcagagctgcatccccatcttggacgaccagtgcttcgtgcacccctgcaccggcgtgggcgaatgccgtagcagctccctgcagcccgtgaagaccaagtgcaccagcgattcctactatcaggataactgcgccaacatcaccttcaccttcaacaaggagatgatgagccccggcctgaccacggaacacatctgcagcgagctgaggaacctgaacatcctgaagaacgtgtccgccgaatacagcatctacatcgcctgcgagcccagccccagcgccaacaacgaaatccacgtcgccatctctgccgaggacatccgcgacgacggcaaccccattaaggagataaccgacaagatcatcgacctggtgtccaagcgagacggaaattctagcctgatcgccgccgtagccgaggtacgtgtgcagaggaggcccctcaagaataggaccgacttcctggtgcccctgctgagcagcgtgctcaccgtggcgtggatctgctgcctggtgaccgccttttactggtgcctgcgaaagaggaggaagcccggttcacacacgcacagcgccagcgaagacaacaccaccaacaatgtgcgcgagcagctcaaccagatcaagaatcccatcgagaagcacggcgccaacacggtccccatcaaggactacgagaacaaaaacagcaagatgtccaagatccgcacccataacagcgaggtcgaagaagacgacatggacaaacaccagcaaaaggccaggttcgccaagcagccggcctacaccctggtggacagggaggagaagcccccgaacggcacccccaccaagcaccccaactggaccaacaaacaggacaaccgggatctggagagtgcgcagagcctgaacaggatggagtacatcgtg

SEQ ID NO: 23 - DNA, 3654 bp, Artificial Sequence
  Synthetic polynucleotide
atgagaagcccaaggacgcgcggtaggagcggcaggcccctcagcctgctgctggctctactgtgcgccctgcgggccaaggtttgtggggccagtgggcaattcgagctggagatcctgagcatgcaaaacgtgaacggggagcttcagaatggtaactgctgcggcggggcccggaatcccggcgaccggaagtgtacgagggatgagtgtgacacctactttaaggtgtgcctgaaggagtaccagagcagggttacggcaggcggcccctgcagctttggcagcggctccaccccggtgatcggcggcaacacattcaacctgaaggccagccgcgggaacgatcgtaacaggatcgtgctcccctttagcttcgcctggccccgcagctacacgctgctggtggaggcctgggacagcagcaacgacaccgtccagcccgatagcattatcgagaaggcctcccacagcggtatgatcaacccgagccggcagtggcagaccctgaagcagaacaccggcgtggcccacttcgagtaccagatccgggtgacctgcgacgactactattacggtttcggctgcaacaagttttgccgaccccgggacgactttttcgggcattacgcctgcgaccaaaacggcaacaaaacctgcatggagggctggatgggcccggagtgcaaccgggccatctgccggcaggggtgtagccccaagcacggcagctgcaagctgcccggcgattgccggtgccagtacgggtggcagggcctgtactgcgacaagtgcatcccgcaccccggatgtgtgcacggcatctgcaacgagccctggcagtgcctgtgcgaaaccaactgggggggtcagctgtgtgacaaggatctgaactactgcggaacccaccaaccctgcctgaacggcggaacttgctcgaacacgggccccgacaagtaccagtgcagctgtcccgagggctacagcgggcccaactgtgagatcgccgaacacgcttgcctgagcgacccgtgtcacaaccggggcagctgcaaggagacctccctcggcttcgagtgcgagtgctccccagggtggaccggccccacctgcagcaccaacatcgacgattgcagccccaacaactgtagccacggcgggacgtgccaggacctggtcaacggcttcaaatgtgtctgtcccccccagtggaccggcaaaacctgccagctcgacgccaacgagtgcgaagccaagccgtgcgtgaacgcgaagagctgcaagaacctgatcgcctcctactactgcgactgcctgcccggctggatgggccagaactgcgacataaacatcaacgactgcctgggccagtgccagaacgatgccagctgtcgagacctggtgaacgggtaccggtgcatctgcccccccggatacgccggggaccactgcgagcgcgacatcgacgaatgtgcctcgaacccctgcctgaacgggggccactgccaaaacgagatcaatcgtttccagtgcctgtgccccaccggcttctctgggaacctgtgccagctggacatcgactactgcgagcccaacccctgccagaacggggcgcagtgctataaccgggcctccgattacttctgcaagtgccccgaggactatgagggaaaaaactgctcccacctgaaggatcactgtaggaccaccccctgtgaggtgatcgacagctgcaccgtggccatggccagcaacgacacccccgagggcgtgcgctacatcagctccaacgtgtgcggcccccatggtaagtgtaagtcgcagagcggcgggaagttcacctgcgactgcaacaagggctttacggggacctactgtcatgaaaacatcaacgactgcgagagcaacccctgtcgcaacggcggcacctgcatcgatggcgtcaacagctacaagtgcatctgctccgacggatgggagggcgcctactgcgagaccaacatcaacgactgcagccagaacccgtgccacaatggcggcacctgccgtgacctggtgaacgacttttactgcgactgcaagaacgggtggaaaggcaaaacctgccactccagggacagccagtgcgacgaggcgacctgcaacaatggcgggacgtgctacgacgagggcgacgccttcaagtgcatgtgccccggcggatgggaaggcactacctgtaacatcgcccggaatagctcctgcctgccgaacccctgccacaacgggggcacgtgcgtcgtgaacggcgaaagcttcacctgcgtgtgcaaggagggctgggagggccccatctgtgcccagaacaccaacgactgcagcccccacccctgctacaatagcggcacctgcgtggacggagacaactggtaccgatgcgagtgcgcccctggcttcgccggacccgattgccgcattaacatcaatgaatgccagagcagcccctgcgcctttggagccacctgcgtcgatgagatcaacggctaccgctgtgtctgcccccccggccacagcggggccaagtgccaggaggtctcaggtcggccctgcatcaccatgggcagcgtcatccccgacggggccaaatgggatgacgactgcaatacctgccagtgtctgaacggccgaatcgcctgctccaaggtgtggtgcgggcccaggccctgcctccttcacaaaggccatagcgagtgcccctccgggcaatcctgcatccccatcctggacgaccaatgcttcgtgcacccctgcaccggcgtgggggagtgcaggagcagcagcctgcagcccgtgaagaccaagtgcacctccgatagctattaccaggacaactgcgccaacatcaccttcacctttaacaaagaaatgatgtcacccggcctgacgaccgagcatatctgcagcgagctgcggaacctgaacatcctgaaaaacgtgtcggccgagtacagtatatacatcgcctgcgagcccagccccagcgccaacaacgagatacatgtggccataagcgccgaagacatcagggacgatggcaaccccatcaaggagatcaccgacaaaataatcgacctggtgagcaagcgggatggcaatagcagcctgatcgccgccgtggccgaggtgagggtgcagcggaggcccctgaagaatcgcaccgacttcctggtcccgctgcttagctccgtcctgacggtcgcctggatctgctgcctggtgaccgccttctactggtgcttgaggaagcggaggaagcccgggtcacatacccactccgccagcgaggacaacaccaccaataacgtgcgggaacagctgaaccagatcaagaaccccatcgagaagcatggtgccaacaccgtgcccatcaaggactatgaaaacaagaactccaagatgagcaagatcaggacccacaactccgaggtggaagaggacgacatggacaagcaccagcagaaagcccgtttcgccaagcagcccgcctacaccctggtggaccgagaggaaaagccgcccaacggcacccccaccaagcatcccaactggaccaacaagcaggacaaccgtgacctggagagcgcccagtcgctcaaccgcatggagtacatcgtg

SEQ ID NO: 24 - DNA, 3654 bp, Artificial Sequence
  Synthetic polynucleotide
atgcggtcgccgagaaccaggggccggagcggccggcccctgtcgctgctgctggccctgctctgcgcgctgagagccaaggtgtgtggcgccagcggccagttcgagcttgagatcctgtccatgcaaaacgtcaacggcgagctccagaacggaaactgttgcggcggcgcccgcaaccccggcgacaggaagtgcacccgcgacgagtgcgacacctacttcaaggtgtgcctgaaggagtaccagtcccgcgtgaccgctggcggaccgtgcagcttcggctcaggcagcacccccgtgatcgggggcaataccttcaatctcaaggccagccgaggaaacgacaggaacaggatcgtgctcccctttagctttgcctggcctcgtagctacaccctgctggtggaggcctgggactcaagcaatgacacggttcagcccgacagcatcatcgaaaaggcctctcacagcggaatgatcaaccccagcaggcagtggcagaccctcaagcagaacacgggcgtggcccacttcgagtaccagatccgtgtgacctgcgatgactactattacggtttcgggtgtaataagttctgcaggcccagggatgacttttttggccactacgcctgcgaccagaatggcaacaagacctgcatggagggatggatgggccccgagtgcaaccgtgccatctgtcggcagggctgctcgcccaagcacggcagctgcaagcttcccggcgactgtcggtgccagtacggatggcaagggctgtactgcgacaagtgcatcccccatcccggctgtgtccacggtatctgcaacgagccctggcagtgtctgtgcgagaccaactggggcggccagctgtgcgacaaggacctgaactactgcggcacccaccagccctgcctgaatgggggcacctgttctaacaccgggccggacaagtaccagtgttcctgccccgagggctacagcggccccaactgcgagatcgccgagcacgcctgcctgtccgacccctgccataataggggctcctgcaaggagacctccctgggctttgagtgcgagtgttcgcccggctggaccggccccacctgcagtaccaacatcgacgactgcagccccaacaactgtagccacggcggcacatgccaagacctggtgaacggcttcaagtgcgtctgcccgccgcagtggaccgggaagacctgtcagctggatgccaacgagtgcgaggctaaaccctgcgtgaacgcgaagagctgtaagaacctgattgccagctactactgcgactgcctgccgggctggatggggcagaattgcgacatcaacatcaacgactgtctgggccaatgccagaacgacgccagctgtcgggacctggtcaacggatacaggtgtatctgtccccccggctacgccggcgaccactgcgagcgggacatcgacgaatgcgccagcaacccttgtctgaacggaggccactgccagaacgagatcaacaggtttcagtgcctctgccccaccgggttcagcgggaacctgtgccagcttgacatcgattactgcgagcccaacccctgtcagaatggggcgcagtgctacaaccgagcttccgattacttctgcaagtgccccgaggattacgagggtaaaaattgcagccacctgaaggatcactgcaggaccaccccgtgcgaggtgatagacagctgcaccgtggccatggccagcaacgacacccccgagggcgtgcgatacatcagcagcaacgtgtgcggcccccacggcaagtgcaaaagccagagcggcggaaaattcacatgcgactgcaacaaggggttcacgggcacctattgccacgagaacatcaacgactgcgagtccaacccgtgccggaatggcggcacctgcatcgacggcgtgaactcctataagtgtatctgctcggacggctgggagggggcctattgcgagaccaacatcaacgactgcagccagaacccctgccacaacggcggcacctgcagggacctggtgaacgacttctattgcgactgcaagaacggctggaagggcaagacctgtcactccagggacagccagtgcgacgaggccacctgtaacaacggcgggacctgttacgacgagggggacgcgttcaagtgcatgtgccccggcggctgggagggcaccacgtgcaacatcgcgcgtaacagcagctgtctgccgaatccctgtcacaatggcggcacctgcgtcgtgaacggcgaaagcttcacctgcgtgtgtaaggaaggctgggagggccccatctgcgcccaaaacaccaacgactgtagcccccacccgtgctacaacagcggcacctgcgtggatggcgacaactggtatcggtgcgagtgtgcccctggctttgcgggccccgactgccggataaacataaacgagtgtcaatcgagcccctgcgccttcggggccacctgcgtggacgagatcaacggctacaggtgcgtgtgcccgcccggccacagcggcgcgaaatgccaagaggtgagcggcaggccctgcatcaccatgggttccgtgatccccgacggggcaaaatgggacgacgactgcaatacctgccagtgcctcaacgggaggatcgcctgcagcaaggtgtggtgcggccccaggccctgcctgctgcataaagggcacagcgagtgccccagcgggcagagctgcatccccatcctggacgaccagtgcttcgtgcacccgtgcaccggcgtgggcgagtgcagaagctctagcctgcaacccgtgaagaccaagtgcacgagcgacagctactaccaggacaactgcgcgaacatcaccttcaccttcaataaggagatgatgagcccgggactcaccaccgaacatatctgctccgagctgcgcaacctcaacatactgaagaatgtgagcgccgagtactccatttacattgcctgcgagcccagcccctccgccaataatgaaatacacgtcgccatcagcgccgaggacatcagggacgacggcaaccccatcaaggagatcaccgacaagatcatcgacctggtgagcaaaagggacggcaatagcagcctcatcgccgccgtggccgaggtgagggtgcagaggaggccgctgaaaaacagaaccgattttctcgtccccctgctgtcctccgtgctgaccgtcgcctggatctgttgcctggtgaccgccttctactggtgtctccgcaagaggcgcaagcccggcagccacacgcatagcgccagcgaggacaacactactaacaacgtgcgggagcagctgaatcagatcaagaaccccatcgagaaacacggcgccaacactgtgcccatcaaagactacgagaacaaaaactcgaaaatgagcaagatccgcacccacaacagcgaggtggaggaggacgacatggacaagcaccagcagaaagcgagattcgccaaacagcccgcctacaccctggtggacagggaggagaagcccccaaacggcacacccaccaagcacccgaactggaccaacaagcaggacaaccgtgacctggaaagcgcccagtccctgaatcgcatggaatatatcgtg

SEQ ID NO: 25 - DNA, 3654 bp, Artificial Sequence
  Synthetic polynucleotide
atgcgaagcccccgaacccggggcaggagcgggaggcccctgagcctgctgctggcccttctgtgcgcccttagggccaaggtgtgtggggcctccggccagttcgagctggagatcctgagcatgcagaacgtgaacggtgagctgcagaatggtaactgttgcggcggagccaggaacccgggcgataggaaatgtaccagggacgagtgcgacacctactttaaggtgtgcctcaaagagtaccagagccgggtcaccgccggcggcccctgctcgttcggcagcggtagcacccccgtgatcggcggcaacacattcaacctgaaagccagcagggggaacgacaggaaccggatcgtgctccccttctccttcgcctggcccaggtcgtacaccctgctcgtcgaggcctgggacagcagcaacgacaccgtgcagcccgacagcatcatcgaaaaggccagccacagcggaatgatcaaccccagccgacagtggcagaccctgaagcagaacaccggcgtggcccacttcgagtaccagatccgggtgacctgcgatgactattactatggcttcggctgtaacaagttctgtcgacccagggacgacttcttcggccactatgcctgcgaccagaacggtaataagacttgcatggagggctggatgggccccgagtgtaacagggccatctgcaggcagggctgctcccccaaacacggctcctgcaaactgcccggcgactgccgctgccagtacggctggcaggggctctactgcgataagtgcatcccccatcccggctgcgtgcatggcatctgcaacgaaccctggcagtgcctgtgcgagaccaactgggggggccagctatgcgataaggatctgaactactgtggcacccaccagccctgcctgaacgggggcacgtgctcaaacaccggccccgacaaataccaatgcagctgccccgagggctacagcggccccaactgcgagatcgccgagcatgcctgcctgagcgacccgtgccacaataggggctcctgtaaggagaccagcctgggcttcgagtgtgagtgcagccccggctggaccggccccacctgctcaactaacatcgacgactgttcccccaacaattgcagccacggcggcacctgccaggacctggtgaacggctttaagtgtgtgtgccccccccagtggaccgggaagacctgtcagctggacgctaacgagtgtgaggccaagccctgtgtcaacgccaaaagctgcaagaacctgatagcctcctactactgcgactgcctgcccggatggatgggccagaactgcgacatcaacatcaatgactgcctggggcagtgccagaacgacgccagctgccgggacctggtgaatgggtaccgctgcatctgcccccccggctacgcgggcgaccactgcgagagggacatcgacgagtgcgcctcgaacccctgcctcaacgggggccactgccagaacgagatcaaccggttccagtgtctgtgccctactggcttctctggcaacctgtgtcagctggatatcgattactgcgagccaaacccatgccagaacggggcccagtgctacaatagggcctccgactatttttgcaagtgccccgaggactacgagggtaagaactgttcccatctcaaggaccactgtcgaaccaccccctgcgaggtgatcgacagctgcaccgtggccatggccagcaatgacacccccgagggcgtgcggtacatctccagcaacgtgtgcggcccccacggcaagtgcaagagccagtccggcggcaaatttacctgcgattgcaacaaggggttcaccggcacctactgtcacgagaacatcaatgactgcgaatccaatccctgcaggaacggtggcacgtgcatcgacggggtgaatagctataagtgcatctgcagcgacgggtgggaaggggcctactgcgagaccaacatcaacgactgtagccagaacccgtgccacaatggcggcacttgtagggatctcgtgaatgacttctattgcgactgcaaaaatggatggaaggggaagacctgccactcccgggactcccagtgcgacgaggccacctgcaataacggcggtacctgctacgacgagggcgatgcctttaaatgcatgtgccccggcggctgggagggaaccacgtgcaacatcgcgaggaacagcagctgcctccccaatccctgtcacaatggcggtacctgcgtcgtgaacggggagagcttcacctgcgtgtgcaaggagggctgggagggcccgatctgcgcccagaacaccaacgactgcagcccacacccctgctacaatagcgggacctgcgtggacggagacaactggtaccggtgcgagtgcgcccccggcttcgccggccccgactgcaggatcaacatcaacgagtgccagagcagcccctgtgccttcggcgcgacctgcgtggatgaaatcaatggctaccggtgcgtgtgcccccccggccacagcggcgcgaagtgccaggaggttagcggcaggccctgcatcaccatgggatcggtgatccccgatggcgccaagtgggatgacgactgtaacacatgccaatgtctgaatggacggatcgcatgttccaaggtgtggtgcggccccaggccctgtctcctgcacaaaggccacagcgagtgtcccagcggccaaagctgcatccccatcctggacgaccagtgcttcgtgcatccctgcaccggcgtgggggagtgccgtagcagcagcctgcagcccgtgaagacgaagtgcacctcagacagctattaccaggataactgcgcgaacatcaccttcacctttaacaaggagatgatgtcccccggcctgaccaccgagcacatctgctcggagctgcgcaatcttaacatcctgaaaaacgtgtccgccgagtacagcatttacatcgcctgtgagccgagcccctccgccaacaatgagatccatgtcgccatcagcgccgaggacatccgggacgacggtaatccgatcaaggagatcacagataagatcatcgacctggtgtccaagcgggacggcaacagcagcctgatcgccgccgtcgccgaggtgcgtgtgcagagacggcccctcaagaaccgcaccgacttcctcgtgcccctcctgagctcggtgctgaccgtcgcctggatctgctgcctggtgaccgccttctactggtgcctgcgaaaacgccggaagccggggagccacacccacagcgccagcgaggataacaccaccaataacgtgagggaacagctgaaccagatcaagaaccccatcgaaaaacacggcgccaacaccgtgccgatcaaggactacgagaacaaaaatagcaagatgagcaagatcaggacacacaactctgaggtggaggaggacgacatggacaagcaccagcagaaggcccgcttcgccaagcagcccgcctacaccctggtcgaccgggaagagaagcccccgaacggcacccccaccaagcatcctaactggaccaacaagcaagacaacagggacctggaaagtgcccagagcctgaaccggatggagtacatcgtg

SEQ ID NO: 26 - DNA, 3654 bp, Artificial Sequence
  Synthetic polynucleotide
atgcgaagcccgaggacccggggcaggagcggcaggccgctaagcctgctgctggccctcctctgcgccctcagggccaaggtgtgcggcgcctccggccaattcgagctcgagatcctgtcaatgcagaacgtgaacggcgagctgcagaacggcaactgctgcggcggcgccaggaaccccggcgacaggaagtgcaccagggacgaatgtgacacctacttcaaggtgtgcctgaaggagtaccagagccgggtgaccgctggcggcccatgtagcttcgggagcggcagcaccccggtgatcgggggtaacacctttaacctcaaggcttcccgcggcaacgacaggaaccggatcgtgctgcccttctccttcgcctggcccaggagctataccctgctggtcgaggcctgggacagctccaacgacaccgtgcaacccgacagcatcatcgagaaggcctcccactccggcatgatcaaccccagcaggcagtggcagaccctcaagcaaaacaccggggtcgcgcacttcgagtaccagatcagggtcacctgcgacgactactactacggcttcggctgcaataagttttgccggcccagggacgatttcttcggacactacgcctgtgaccagaatggcaataagacctgtatggaagggtggatggggccagagtgcaatcgggccatctgcaggcaaggctgcagccccaaacacggctcgtgtaagctgcccggcgactgcaggtgccagtatggttggcagggcctctattgcgacaagtgcatcccccacccaggctgtgtgcatggcatctgtaacgaaccctggcagtgcctgtgcgagacgaactgggggggccaactgtgcgacaaggacctgaactattgcggcacccaccagccgtgcctgaatggcggaacctgttccaacaccggccccgacaagtaccagtgctcctgtcccgaggggtacagcggccccaactgcgagatcgccgagcatgcctgcctcagcgatccctgccacaacaggggcagctgcaaggagacgagcctgggcttcgagtgcgaatgcagccccggttggaccggccccacgtgctccaccaacatcgacgactgctcccccaacaattgcagccacgggggcacatgtcaggacctggtgaacggcttcaagtgcgtgtgcccgccccaatggaccggcaagacgtgccagctggacgccaacgagtgcgaagccaagccatgcgtgaacgccaagagctgcaagaacctgatcgccagctactactgcgactgcctcccaggctggatgggccagaactgtgatatcaacatcaacgactgcctcggccagtgccagaacgacgccagctgccgggacctggtgaacgggtaccgctgcatctgtccgcccggctacgccggagaccactgcgagcgcgacatcgacgagtgtgccagcaacccctgcttaaacggcggccactgccaaaatgaaatcaataggtttcagtgcctgtgccccaccgggttcagcggcaacctgtgccagctggacatcgactattgcgagccgaacccctgccagaacggggcccagtgctacaatagggccagcgattatttctgcaagtgtcccgaggactacgagggaaaaaactgcagccacctcaaggaccactgtaggaccacgccctgcgaagtgatcgactcctgcaccgtggccatggccagcaacgacacccccgagggcgtgcgctacatcagcagcaacgtgtgtggccctcacggcaaatgcaagagccaaagcggcggcaagttcacctgtgactgcaataagggcttcaccggcacctactgtcacgagaacatcaacgactgcgagagcaacccctgcagaaacggtggcacctgtatagatggcgtgaacagctacaagtgcatctgcagcgacggatgggaaggcgcctactgtgagaccaacattaacgactgcagccagaacccctgccacaatggcggcacctgccgcgacctggtcaatgacttttactgcgactgtaagaacgggtggaagggcaagacctgccatagccgcgactcccagtgcgacgaggcaacctgcaacaacggcggcacctgttatgatgagggggacgcattcaagtgcatgtgtccggggggctgggagggcacaacctgcaacatcgcccggaacagcagctgcctcccaaacccctgccacaacgggggcacctgcgtggtgaacggcgagagcttcacctgcgtgtgtaaggagggctgggagggccccatctgtgcccagaataccaacgattgctccccccacccctgctacaacagcggcacttgcgtggacggcgataactggtataggtgtgagtgcgcccccggcttcgcaggccccgactgccgcatcaacatcaacgagtgccagagcagcccctgtgccttcggggccacctgcgtggacgagatcaacggctaccggtgtgtgtgcccccccgggcactccggcgcgaaatgccaggaggtgtccggcaggccctgcatcaccatgggcagcgtgatccctgacggcgccaaatgggacgacgactgtaatacctgccagtgcctgaatggccgaatcgcctgctccaaggtgtggtgcggccccaggccttgcctgttgcacaagggccacagcgagtgccccagcggccagagctgtatccccatcctggacgaccaatgtttcgtgcatccctgcaccggcgtgggggagtgccggtcgtccagcctgcagcccgtgaagaccaagtgtaccagcgactcctactatcaggacaattgcgccaacatcaccttcacctttaacaaggagatgatgagccccggcctgaccaccgagcacatctgttccgagctgaggaacctgaacatcctgaagaacgtcagtgccgagtactccatctacatcgcctgtgaaccgtccccgtccgccaacaatgagattcacgtggccatcagcgccgaagacatcagggacgacggcaaccccatcaaggagatcaccgacaagatcatagaccttgtgtccaagagggacggcaactcgtccctgatcgccgccgtggcggaggtgagggtgcagaggaggcccctgaagaaccgcaccgacttcctggtgccgctcctgtcctccgtgctgaccgtggcctggatctgctgcctggtgaccgccttctactggtgcctgaggaagcgccgcaagcccgggtcccacacgcacagcgccagcgaggataacaccaccaacaacgtgcgggagcaactgaaccagataaagaaccccatcgaaaaacacggagcgaacaccgtccccatcaaggactacgaaaacaagaacagcaagatgagcaagatcaggacccataactccgaggtggaggaggacgacatggacaagcaccagcaaaaggcccggttcgccaagcagcccgcctacaccctggtggatcgggaggagaagccccccaacggtaccccgaccaaacaccccaactggaccaataaacaggacaatagggacctggagtccgcccagagcctgaacaggatggagtacatagtg

SEQ ID NO: 27 - DNA, 3654 bp, Artificial Sequence
  Synthetic polynucleotide
atgagaagccccaggacccgaggcaggagcggcaggccactgagcctgctccttgccctgctgtgcgccctgagggcaaaggtgtgcggcgccagcggccagttcgagctggaaatcctgtccatgcagaacgtgaacggggagctgcagaatggcaattgctgtggcggcgcgcggaaccccggcgacaggaagtgcacacgggacgaatgcgacacgtacttcaaggtgtgcctcaaggagtaccagtccagggtcaccgccggcgggccctgcagcttcggaagcggctccacccccgtgatcggcggcaacacattcaacctgaaagcgtcgagggggaatgaccgcaacaggatcgtgctgccgttttccttcgcctggccccgcagctacacgctgctggtggaggcatgggacagctccaacgataccgtgcagcccgacagcatcatcgagaaggcctcccacagcggcatgatcaacccgagcaggcagtggcagaccctcaagcagaacaccggcgtggcccacttcgagtatcagatccgggtgacctgcgacgactattactacggtttcggctgcaacaagttttgtaggccccgagacgacttcttcggccactacgcctgcgatcagaacgggaataaaacctgtatggaggggtggatgggccccgagtgcaacagggccatctgcaggcagggatgctcccccaagcacggcagctgcaagctgccaggagactgcaggtgtcagtatggctggcaggggctgtactgcgataagtgcattccgcacccaggatgtgtgcacggaatctgtaacgagccctggcagtgcctgtgcgaaaccaactgggggggccaactctgcgacaaggacctgaactactgcggcacccaccaaccctgtctgaacggcggcacctgcagcaacaccggccccgacaaataccagtgcagctgccccgagggctactccgggcccaactgcgagatcgccgaacacgcatgtctgagcgacccttgccacaacaggggcagctgcaaggagacctccctcggctttgagtgcgaatgcagccccggctggaccgggcccacctgcagcacgaacatcgacgactgcagccccaacaactgctcccacggcgggacgtgccaggatctcgtcaacggcttcaagtgcgtgtgccccccccagtggaccggcaaaacctgccagctggacgcaaacgagtgcgaagccaagccgtgcgtcaacgcgaagagctgcaagaacctcatcgccagctactattgcgactgcctgcccggctggatgggccagaactgcgacataaacatcaacgactgcctgggccagtgtcagaacgatgcctcctgcagggacctggtgaacgggtaccggtgtatctgcccccccgggtacgcgggggaccactgcgagagagacatcgatgagtgcgcctccaatccctgcctgaacggcggccattgccagaacgagatcaaccggttccagtgcctgtgccccaccggcttctccggcaacctgtgccaactagacatcgactactgcgagcccaatccctgccagaacggcgcccaatgctacaacagggccagcgactacttctgtaagtgccccgaggactacgagggcaagaactgctcccatctgaaggaccactgccggaccaccccctgcgaagtgatcgacagctgcaccgtggccatggccagcaatgacacccccgagggcgtgaggtatatcagcagcaacgtgtgcgggccccacgggaaatgcaagagccagagcggcggcaagttcacatgcgactgtaacaagggcttcacgggaacctactgtcacgagaacatcaacgactgcgagagcaacccctgccgcaacggcggcacctgcatcgacggcgtgaactcctataagtgcatctgtagcgatggctgggaaggggcctactgcgagaccaacataaacgactgcagccagaatccctgccataacgggggcacctgtcgtgacctggtcaacgacttctactgcgactgtaagaacggatggaagggtaagacctgccactccagggactcccagtgtgacgaagccacctgcaacaacggaggcacctgctacgacgagggtgacgcctttaagtgcatgtgccccggtggctgggaggggaccacgtgcaacatcgcccgcaacagcagctgccttccgaacccatgccataacggcggcacctgtgtcgtgaacggcgagtcgttcacctgtgtgtgcaaggaaggctgggaaggccccatatgcgcccagaacaccaacgactgcagcccccatccctgctacaactccggcacctgcgtggacggggacaactggtacaggtgtgagtgcgcccccggattcgccggtcccgactgccggatcaacatcaatgagtgtcaatccagcccctgcgccttcggcgccacctgcgtggatgagatcaacggctacaggtgcgtctgtccccccggccactccggcgccaaatgccaggaggtcagcggcaggccctgcatcaccatgggctccgttatccccgacggcgccaagtgggacgacgactgcaatacctgccagtgtctgaacgggaggatcgcctgctccaaggtgtggtgcggccccaggccctgcctgctgcacaagggccacagcgagtgccccagcggccagtcctgcatcccgatcctggacgaccagtgctttgtgcacccctgcaccggggtaggcgagtgccggtccagcagcctgcagcccgtgaaaaccaagtgcaccagcgacagctattaccaggacaactgcgccaatatcacctttacgttcaataaagagatgatgagccccggcctgaccaccgaacacatctgcagcgagctgcgcaacctgaacattctgaagaacgtgagcgccgagtacagcatctatatagcctgcgagcccagcccctcggctaataacgagatccacgtggccataagcgcggaggacatccgggacgacggcaaccccatcaaggagatcaccgacaagatcatcgacctggtgagcaagcgcgacgggaactcatcactgatcgccgccgtggccgaggtgagggtgcagaggcggcccctcaagaacaggaccgacttcctcgtccccctgctgtcgagcgtgctcaccgtggcctggatctgctgtctcgtgaccgcattctactggtgcctgaggaaacggcgcaagcccggctcgcacacccacagcgccagcgaagataacaccaccaacaacgtgagggagcagctcaaccagatcaagaaccccatagagaagcacggcgccaacacggtgccaatcaaggactatgagaacaagaacagcaagatgtccaagatccgcacccacaacagcgaagtcgaggaagacgacatggacaagcaccagcagaaagcgcgtttcgccaagcagcccgcctacaccctggtggacagggaggagaagccccccaacggaacccccacaaagcacccaaactggacgaataagcaggacaacagggacctggagagcgcccagagtctgaaccggatggagtacatcgtg

SEQ ID NO: 28 - DNA, 3654 bp, Artificial Sequence
  Synthetic polynucleotide
atgagaagtcccaggacccgcgggcggagcgggcgccccctgagcctgttactggccctcctgtgtgccctgcgcgcgaaggtgtgcggggccagcggccagttcgagctggagatcctgagcatgcagaacgtgaacggggaactacagaacggcaactgctgcggcggcgcccgcaatccgggagacaggaagtgtaccagggatgagtgcgacacctactttaaagtgtgcctgaaggagtaccagagcagggtgaccgccggcggcccctgtagcttcggcagcgggagcaccccggtgatcggcggcaacaccttcaacctcaaggcctccaggggcaacgacaggaaccggatcgtgctgcccttcagcttcgcctggccccgcagctacacgctgctggtggaggcctgggacagctctaatgacacggtgcagcctgactcaattatagagaaggccagccacagcggcatgatcaacccctcaagacagtggcagaccctgaagcagaacaccggtgtggcacacttcgagtatcagatcagggtgacatgcgatgactactactacgggtttggctgtaataagttctgcaggccccgagacgatttcttcgggcactatgcctgcgaccaaaatggcaacaagacctgcatggaggggtggatgggcccggagtgtaaccgagccatatgtaggcaaggctgcagcccgaagcacggctcctgcaagctgcccggtgattgcaggtgccagtacggctggcaaggcctctactgcgacaagtgcatcccgcaccccggttgcgtccacggcatctgcaacgagccctggcagtgcctgtgcgagaccaactgggggggccagctgtgcgacaaggacctcaattactgtggcacccaccagccctgcctcaacggtggcacctgctccaacaccggccccgacaagtaccagtgtagctgccccgaggggtacagcggcccgaactgcgagatcgccgagcacgcctgcctgtccgacccctgccacaatcgcggcagctgcaaggagaccagcctggggttcgaatgcgagtgttccccgggctggaccggccccacctgcagcaccaatatcgatgactgctcccccaacaactgcagccacggcggcacctgtcaggacctggtgaatggcttcaagtgtgtgtgcccaccgcagtggaccggcaaaacctgccagctcgacgccaacgagtgcgaggccaagccctgtgtgaatgccaagtcctgcaagaacctgatcgccagctactactgcgactgcctgcccgggtggatggggcaaaattgcgacataaacataaacgactgcctgggccagtgccagaacgacgcctcctgtcgggacctggtcaacggctacaggtgcatctgcccacccggctacgccggcgaccactgcgagcgagatatcgacgaatgcgccagcaacccctgcctgaacggggggcactgccagaatgagatcaacaggtttcagtgcctgtgccccaccggcttcagcggcaacctgtgtcaactggacatcgactattgtgagcccaacccttgccaaaacggggcccagtgctacaaccgggccagcgattacttctgcaagtgccccgaggactacgaaggcaagaactgcagccacctgaaggaccactgtcggaccaccccctgcgaagtgatcgacagctgcaccgtggccatggccagcaacgacacccccgagggcgtgaggtacatcagcagcaatgtgtgtggcccgcacggcaagtgcaagagccagagcggcggcaagttcacgtgcgactgcaacaagggctttaccggcacctactgccacgaaaacatcaatgactgcgagagcaacccgtgtcggaacggcggcacctgcatcgacggggtgaacagctacaagtgcatatgcagcgacggctgggagggcgcctactgtgaaaccaacatcaacgactgcagccagaacccctgccacaatggcgggacctgcagggacctggtgaatgacttctactgcgactgcaagaacggctggaagggcaaaacctgccacagcagggacagccagtgcgacgaggccacctgcaacaacggcggcacctgctatgacgagggcgacgccttcaagtgcatgtgccccggcggatgggagggcacgacctgcaatatcgcaaggaacagctcctgtctgcccaatccctgccacaacggcggtacctgcgtggtgaacggggaaagcttcacctgcgtgtgcaaggaggggtgggaggggcccatctgcgcccagaacaccaacgactgcagcccacacccctgctacaattccggcacctgtgtggacggcgacaactggtataggtgcgagtgcgcccccggtttcgccggcccggactgcaggatcaacatcaacgagtgtcagtccagcccctgcgccttcggggccacctgcgtggacgagatcaacggctatcgttgcgtgtgcccccccggccactccggcgccaagtgccaggaagtgtccgggcgcccctgcatcaccatgggctccgtgatccccgatggcgccaagtgggatgacgactgcaacacctgtcagtgcctgaacggcaggatcgcctgcagcaaggtgtggtgcggcccccgaccctgcctgctgcacaaggggcacagcgagtgcccctccggccagtcctgcatccccatactggacgatcagtgcttcgtgcacccctgcaccggcgtgggcgagtgtaggagctccagcctgcagcccgtgaaaaccaagtgcacctcggacagctactatcaggataactgcgccaacattacgttcaccttcaacaaggagatgatgtcccccggcctgaccacggagcacatctgttccgagctgaggaacctcaacatcctgaaaaatgtgagcgccgagtatagcatctatatagcctgtgagccgtccccctccgccaacaacgagatccacgtcgccatctccgcagaggacattcgcgacgacgggaaccccataaaggaaattacggacaaaatcatcgacctggtgagcaagagggacggcaactccagcctgatcgccgccgtggccgaggtgcgcgtgcaacgcaggccgctgaaaaacaggacggactttctggtgccgctgctgtcctcggtgctgaccgtcgcttggatctgctgcctggtgaccgccttctactggtgcctgcgcaaaaggcgcaagcccggtagccatacccactccgcctccgaagacaacaccaccaacaacgtgagggagcagctgaatcagatcaagaaccctatcgagaagcacggcgccaacacggtgcccatcaaggactatgaaaacaagaacagcaagatgtccaagatcaggacccacaacagcgaggtggaggaagacgacatggacaagcaccagcagaaggcccgattcgccaagcagcccgcttacaccctggtggacagggaggaaaagcccccgaacggcacccccaccaaacaccccaactggactaataaacaggacaaccgagacctggagagcgcccagagcctgaacaggatggaatatatcgtc

SEQ ID NO: 29 - DNA, 3654 bp, Artificial Sequence
  Synthetic polynucleotide
atgcgtagccccaggaccaggggtaggtccgggaggcccctgtcactcctcctggccctgctctgtgccctccgggccaaggtgtgcggcgccagcggacagtttgagctggagatcctgtccatgcagaacgtgaacggtgagctccagaacgggaactgctgcggcggcgccaggaaccccggcgatcgcaagtgtaccagggacgaatgtgacacctactttaaggtgtgcctgaaagagtaccagagccgcgtcaccgccggcgggccctgttcctttggctccggcagcactcccgtgatcggcggcaacaccttcaacctcaaggcgagcagggggaacgacaggaacaggatcgtgctgcccttcagcttcgcgtggccccggtcctacaccctgctcgtggaggcttgggactcctcaaacgacacggtccagccggatagcatcattgagaaggcgagccactccggcatgatcaaccccagccggcagtggcagaccctcaagcagaacaccggcgtggcccacttcgagtatcagatccgcgtgacctgcgatgattactactacggctttggatgcaacaagttctgccggccccgcgacgacttcttcggacactatgcctgtgaccagaacgggaacaagacctgcatggagggatggatgggtcccgagtgcaaccgggccatctgcaggcagggctgtagccccaagcacgggagctgcaagctgcccggcgactgcaggtgccagtacggctggcaggggctgtactgcgacaagtgcatcccccacccgggatgcgtgcacggcatctgcaacgagccctggcagtgcctctgcgagaccaactggggcggccagctgtgcgacaaggacctgaactactgtggcacgcatcagccatgcctcaatggtggcacctgcagcaacacgggccccgataagtaccaatgctcgtgccccgaagggtactccggcccaaattgcgagatcgccgagcacgcctgcctgtccgacccctgccacaacaggggctcctgtaaggagacctccctgggcttcgagtgtgagtgcagccccgggtggaccggccccacctgttccaccaacatcgacgactgcagccccaacaactgcagccatggaggcacctgtcaggacctggtgaatggtttcaagtgtgtgtgcccgccccagtggaccgggaagacctgccagctggacgccaacgagtgcgaggctaagccctgcgtcaacgccaagagctgcaagaacctcatcgcctcctactactgcgactgcctgccgggatggatgggccagaactgtgacatcaacatcaacgactgtctgggccagtgccagaatgacgccagctgccgagacctggtcaacggctacaggtgcatatgcccccccggatatgccggggatcactgcgagcgggacatcgacgagtgcgccagcaacccatgtctgaacggcgggcactgccagaacgagatcaacaggtttcaatgcctgtgccccaccggatttagtgggaacctctgtcagctggacatagactactgcgagccgaacccctgccaaaacggcgcgcagtgctacaacagggccagcgattacttctgcaagtgcccggaggactacgaggggaagaactgctcccacctgaaggaccactgcaggaccaccccctgcgaggtgatcgactcgtgcaccgtcgccatggcctcaaacgacacccccgagggggtccgctacatctcgagcaacgtctgtggcccccacggcaagtgcaagagccagagcggggggaagttcacctgcgactgcaacaaaggcttcaccggcacgtactgtcacgagaacatcaatgattgcgagagcaacccctgccggaacggcggcacctgcatcgacggcgtgaacagctacaagtgcatctgtagcgacggctgggagggggcctactgcgagaccaacatcaacgactgcagccagaacccctgtcacaacggcggcacctgcagggacctcgtgaatgacttctactgcgactgcaaaaacgggtggaaaggtaaaacctgccatagccgggacagccagtgcgacgaggccacctgtaataacggcggcacctgctacgacgagggtgacgcctttaagtgtatgtgccccggcggctgggagggcaccacctgcaatatcgcccgcaacagcagctgtctccccaacccctgccacaacgggggtacctgcgtggtcaacggcgagtcctttacctgcgtgtgcaaggagggctgggaagggcccatctgcgcccagaacaccaacgactgtagcccccatccctgctacaactccggtacctgcgtggacggcgacaattggtacaggtgtgaatgcgcaccaggcttcgcggggcccgactgcaggatcaacatcaacgaatgccagagcagcccctgcgcgttcggcgccacctgcgtggacgagatcaacgggtacaggtgcgtgtgcccccccgggcacagcggggccaagtgccaggaggtctccgggcggccctgcatcaccatgggctccgtgatcccggatggggcgaagtgggacgacgattgcaacacctgccaatgcctgaacgggaggatcgcctgtagcaaggtctggtgcggaccccggccctgcctcctgcacaaaggccactccgaatgccccagcggacaaagctgcataccgatcctggacgaccaatgcttcgtgcatccctgcacaggcgtgggtgaatgcaggagctccagcctgcagccagtgaagacgaagtgcaccagcgatagctactaccaggataattgtgccaacataaccttcaccttcaacaaggagatgatgtcccccggcctgaccaccgagcacatctgtagcgagctccgcaacctgaacatcctcaagaacgtgagcgccgagtactccatctacatcgcctgcgagccctcgcccagcgccaataacgagatccacgtggccatctccgccgaggacatccgcgacgacggcaatcccatcaaggagattaccgacaagatcatcgacctggtgagcaagcgcgatggcaacagcagcctgatcgccgcggtggccgaggtgagggtgcagaggcggcccctcaagaaccgcacggacttcctggtgccactgctgagctccgtgctgaccgtggcctggatctgctgtctggtcaccgccttctactggtgcctgcggaaacggaggaagcccggatcccacacccactccgcctccgaagacaacaccacgaacaacgtcagggagcagctgaaccagatcaagaaccccatcgagaagcatggcgccaacaccgtgccaatcaaagactacgagaacaagaacagcaagatgagcaagatccggacccacaacagcgaagtagaagaggacgacatggataagcaccagcagaaggccaggttcgccaagcaacccgcctacaccctcgtggaccgcgaggagaaaccccccaacggcacccccaccaagcaccccaattggaccaacaagcaagataaccgcgacctggagagcgcccagagcctcaaccggatggaatacatcgtg

SEQ ID NO: 30 - DNA, 3654 bp, Artificial Sequence
  Synthetic polynucleotide
atgaggagcccaaggaccagggggaggagcggcaggccgctcagcctgctgctcgccctgctgtgcgccctgcgggcaaaggtgtgcggggccagcggccagttcgagctggaaatcctgagcatgcagaacgtgaacggcgagctgcaaaatggtaattgctgcgggggcgccaggaacccgggcgacaggaagtgcaccagggacgagtgcgacacctatttcaaggtgtgcctgaaggaataccagagccgcgtcacggccgggggcccgtgctccttcggcagtggctccacccccgtgatcggcggcaacacctttaacctgaaggcctcccggggtaacgacaggaacaggatcgtgctgcccttctccttcgcctggccgaggtcctacaccctcctggtagaggcctgggacagcagcaatgatacggtgcagcccgactccatcatagaaaaggccagccactccgggatgatcaatccgagcaggcagtggcaaaccctcaagcagaacaccggtgtggcccactttgagtaccagatcagggtcacctgcgacgactactactacggcttcggctgcaacaagttttgcaggccgagggacgacttcttcggccactacgcctgcgaccagaatggcaacaagacctgcatggaaggctggatgggcccggaatgcaatcgcgccatctgtaggcaggggtgcagcccaaagcatgggagctgcaagctgcccggggactgcaggtgtcagtacggatggcaggggctgtactgtgacaagtgtatcccacatccgggctgcgtgcacggaatatgcaacgagccctggcagtgcctgtgtgaaacgaactggggcggtcagctgtgcgacaaggacctgaactactgcggcacccaccagccctgcctgaacggcgggacgtgttccaacaccggccccgacaagtatcagtgtagctgccccgagggctatagcggcccgaactgcgagatcgccgaacatgcctgtctcagcgacccctgtcacaacaggggtagctgtaaggaaaccagcctcgggtttgagtgtgaatgctccccgggctggaccgggcccacctgttccaccaacatcgacgactgctcccccaataactgcagccatggcggcacgtgtcaggacctcgtcaatggctttaagtgtgtgtgccccccgcagtggaccggcaagacgtgccagctggacgccaacgagtgtgaggccaagccctgcgtcaacgcaaagagctgcaagaacctgatcgcctcctactattgtgactgcctgcccgggtggatgggacagaactgcgacatcaatatcaacgattgcctggggcagtgccagaacgacgcgagctgcagggacctggtcaacggctaccgatgcatctgccccccgggctacgccggcgaccactgtgaaagggacatcgacgagtgcgccagcaacccctgcctgaacgggggccactgccagaacgagatcaataggttccagtgcctgtgcccgaccggttttagcggcaacctgtgccagctggacattgactattgcgagcccaacccctgccagaacggggcccagtgctacaacagggcctcggactacttctgtaagtgccccgaggactatgagggcaagaactgcagccatctgaaggaccactgcaggaccaccccgtgcgaggtcatcgacagctgcaccgtggccatggcctccaatgatacccccgagggcgtgaggtacatctcctccaacgtgtgtggcccccacggcaagtgcaaaagccagagcggcggcaagttcacctgtgactgtaacaagggcttcaccggcacctactgccatgaaaacatcaacgattgcgagtctaatccctgccggaacggcggcacctgcatcgatggcgtgaacagctataaatgtatctgctccgatgggtgggagggcgcatactgcgaaaccaacatcaacgactgctcccagaacccctgccataacggcggcacctgccgcgacctcgtcaacgatttctactgcgactgcaagaacggctggaagggcaagacctgccacagccgagacagccagtgcgacgaggccacgtgcaacaacggagggacctgttatgacgagggcgacgccttcaagtgcatgtgccccgggggctgggagggcacgacctgcaacattgcccgcaatagcagctgcttgcccaacccctgtcacaacggcggaacctgcgtcgtgaacggcgagtccttcacctgcgtttgcaaagagggctgggagggcccaatctgtgcccagaacaccaatgactgcagcccccacccctgctacaattccggtacctgcgtggacggcgacaactggtataggtgcgagtgcgccccgggattcgccggcccggactgcaggatcaacatcaacgagtgccagagcagcccctgcgccttcggggccacctgtgtggacgagatcaatggctacaggtgtgtctgcccccccggacactcgggcgcgaaatgccaagaggtgtccggcaggccctgcatcaccatgggttccgtgatacccgacggggcaaagtgggacgacgattgcaatacctgccaatgcctgaacggcaggatcgcctgtagcaaggtgtggtgtggcccgaggccttgcctcctgcataaaggccacagcgagtgtccctccggccagagctgtatccccatcctcgacgatcaatgctttgtgcacccttgcaccggggtgggcgagtgtcgcagcagcagcctgcagcccgtgaagaccaaatgcaccagcgatagctactaccaggacaactgcgcgaatatcacctttacgttcaacaaggagatgatgagcccgggcctgaccacagagcacatctgcagcgagctgcgcaacctgaacatcctgaagaacgtgtctgccgagtatagcatctacatcgcctgcgaacccagcccctccgcaaataatgagatccacgtggcgatctcggccgaggacatcagggacgacgggaaccccatcaaagagatcaccgacaagatcatcgatctggtgagcaagcgggacggcaacagctccctcatcgccgccgtggctgaggtccgagtgcagcggcgtccccttaagaacaggaccgacttcctggtgcccctcctgtcgtccgtgctcaccgtggcctggatctgttgcctggtgaccgccttctactggtgcctgcgtaagcgaaggaagcccggatcccacacccacagcgccagcgaagacaacaccaccaataacgtccgagagcagctgaaccagatcaagaaccccatagagaaacacggggccaacaccgtgcctatcaaggactacgagaacaaaaatagcaaaatgagcaagattaggacccacaactccgaggtggaggaggacgacatggacaagcatcagcagaaggcccgcttcgccaagcaacccgcctacaccctggtggaccgagaggaaaagccccccaacgggacccccacgaagcaccccaactggaccaataagcaggataacagggacctcgagagcgcccagtccctgaatcgcatggagtacatcgtg

SEQ ID NO: 31 - DNA, 3654 bp, Artificial Sequence
  Synthetic polynucleotide
atgaggagcccccgcaccagggggcgtagcggccgccccctgagcctgctgctggctctgctgtgtgccctgcgagccaaagtgtgcggggcctccggccagttcgagctggagatcctgagcatgcagaacgtgaacggcgagctccagaacggcaactgctgcggcggcgcccgcaaccccggcgacaggaagtgcactcgggacgagtgcgacacctatttcaaggtctgcctgaaggagtaccaaagccgtgtgaccgccggcgggccgtgcagcttcggaagcggctccaccccggtcatcggggggaacacctttaacctgaaggccagccggggtaacgacaggaaccgaatcgtactgcccttcagcttcgcctggccccggagctacaccctgctggtcgaggcatgggactccagcaacgataccgtgcagcccgacagcatcatcgagaaagccagccacagcgggatgattaatcccagcagacagtggcagaccctgaagcagaacaccggcgtggcccacttcgagtaccaaatccgggtgacctgcgacgattattactacgggtttggctgtaataaattctgccggccccgggatgactttttcggccattacgcctgcgatcagaacggtaacaagacctgcatggagggctggatgggaccggagtgtaacagggctatctgccgacagggttgtagccccaagcacggaagctgcaagctgcccggcgactgccggtgtcagtacggctggcagggcctgtactgcgataagtgcatcccccaccccggctgcgttcacggcatctgcaacgagccctggcagtgcctgtgtgaaaccaactggggtggacagctgtgcgacaaggatctgaactattgcggcacccaccagccctgcctgaacggcggaacctgcagcaacaccggccccgataagtaccagtgcagctgccccgaaggctactccggccccaactgcgagatcgccgagcacgcctgcctgagcgacccgtgccacaacagggggagctgcaaagagaccagcctgggtttcgagtgcgagtgcagccccggctggaccgggcccacttgctccaccaacattgacgactgtagcccgaacaattgcagccacggcggcacctgccaggacctggtgaatggcttcaagtgcgtgtgtcccccccagtggaccgggaagacctgccagctggacgccaacgagtgcgaggccaagccctgtgtgaacgccaagtcctgcaagaacctgatcgcctcctactactgtgactgtctccccgggtggatgggccagaactgcgacatcaacatcaacgattgcctcggccagtgccagaacgacgccagctgtagggacctcgtgaacggctaccggtgcatctgcccgcccgggtacgccggagaccactgcgagagggacattgacgagtgcgcctcgaacccctgcctgaacggcggccactgtcagaacgagatcaataggttccagtgtctgtgtcccaccggcttctccggcaacctgtgtcagctggacatcgactactgtgagcccaatccctgccagaatggcgcccagtgctataaccgggcctccgactacttttgcaagtgccccgaagattacgagggcaagaactgcagccatctgaaggaccactgcaggacgactccctgcgaggtgatcgacagctgtactgtcgccatggccagcaacgacacccccgagggggtccgctatatcagcagcaacgtgtgcgggccccatgggaaatgcaaatcccagtcagggggcaagtttacctgcgactgtaacaaaggcttcaccggcacctactgccacgaaaacatcaacgactgcgaatcgaacccctgccggaacggcgggacctgcatcgatggagtgaacagctacaagtgcatctgcagcgacgggtgggagggcgcgtactgcgaaaccaatatcaatgactgcagccagaacccctgccataacggaggcacctgcagggacctggtgaacgacttctactgcgattgcaagaacggctggaaggggaagacctgccatagcagggacagccagtgtgacgaggccacctgcaacaacggcggcacatgttacgatgagggcgacgccttcaaatgcatgtgccccggcggctgggagggcaccacatgcaacatcgcccggaacagcagctgcctccccaacccctgccataatggcggtacctgcgtggtgaacggcgagagtttcacctgcgtgtgcaaggagggctgggagggccccatctgcgcgcagaacaccaatgactgctcgccccacccctgctacaacagcggcacctgcgtggacggtgacaactggtaccgttgcgagtgcgccccaggcttcgccggcccggactgcaggatcaacatcaacgagtgccaaagctccccttgcgcctttggcgcaacctgtgtggacgagatcaatgggtacaggtgcgtgtgcccccccggccattccggggccaagtgccaagaggtgtccggccggccctgcattaccatgggcagcgttatccccgacggcgccaagtgggacgacgactgcaatacctgccagtgcctcaacggcaggatcgcctgcagcaaggtgtggtgcggacccaggccgtgcctgctgcataagggccacagcgagtgcccgagcggtcagtcctgcatccccatcctcgacgaccagtgtttcgtgcacccctgcacgggcgtgggtgagtgccgatcctccagcctgcagcccgtcaaaaccaagtgcacctccgacagctactaccaggacaactgcgccaacataaccttcacgtttaacaaggagatgatgagccccggcctgaccaccgagcacatctgcagcgagctgaggaacctgaacatcctgaagaacgtgtccgccgagtacagcatctacatcgcctgtgagcccagcccctccgccaacaacgagatccatgttgccatctcggccgaagatattagggacgacggcaaccccatcaaggagatcaccgacaagatcatagacctggtgagcaagcgggacggcaattccagcctgatcgccgccgtggccgaggtgagagtgcagaggaggcccctgaagaaccggaccgatttcctggtgcccctgctgagcagcgtgctgaccgtggcctggatctgctgcctggtgaccgcattttactggtgtctgaggaagcggaggaaacccggcagccacacccacagcgcaagcgaggataacaccacgaataacgtgcgcgagcagctgaaccaaatcaagaaccccatcgagaagcacggggccaacaccgtgcccatcaaggactacgagaataagaactcgaagatgagcaagatcaggacgcacaactccgaggtggaggaggacgacatggataagcaccagcagaaagcccggttcgccaagcagcccgcctacaccctggttgaccgcgaggagaaaccccccaacggcacccccaccaagcaccccaactggaccaacaagcaggacaaccgagacctggagagcgcccagagcctgaacaggatggagtatatcgtg

SEQ ID NO: 32 - DNA, 3654 bp, Artificial Sequence
  Synthetic polynucleotide
atgaggtcccccaggaccaggggcaggagcgggaggcccctgtcccttctgctggcgctgctgtgcgccctgcgcgccaaggtgtgcggggcaagcggccagttcgagctcgaaatactcagcatgcaaaacgtcaacggcgagctgcagaacggcaactgttgcggtggcgccaggaaccccggggatcgcaagtgcaccagggacgagtgtgatacctacttcaaagtgtgtctgaaggagtaccagagccgggtgaccgccgggggcccctgttccttcggcagcgggagcacccccgtcatcggcgggaatacgtttaacctgaaggcctccaggggcaacgataggaaccggatcgtgctccctttcagcttcgcctggcccaggtcctacaccctgctggtggaggcctgggactccagcaatgacactgtccagcctgacagtatcatagagaaagcctcccactccggcatgatcaaccccagtcgccagtggcagaccctgaagcagaacaccggcgtggcccacttcgagtaccagatccgggtgacctgcgacgactattactacggcttcggatgcaataagttctgtaggccccgcgacgatttcttcggccattatgcctgcgaccagaacggcaacaagacctgcatggagggctggatggggcccgagtgcaacagggccatctgcaggcaggggtgctcccccaaacacgggagctgcaaactgccgggggactgcaggtgccaatacggctggcagggcctgtactgcgacaagtgcatcccgcaccccgggtgcgtgcacggcatttgcaacgaaccctggcagtgcctctgcgaaaccaattggggaggccagctgtgcgacaaggatctgaactactgcggcacgcaccagccctgcctcaacggggggacctgtagcaacacgggccccgacaagtaccagtgctcctgcccggagggatactctggccccaactgcgagatcgccgagcacgcctgcctctccgatccgtgccacaataggggcagctgcaaggaaacgtccctgggcttcgaatgcgaatgcagtcccggatggaccggccccacctgcagcaccaacatcgacgactgcagccccaacaactgcagccacggcggcacctgccaagatctcgtgaacggcttcaagtgcgtgtgccccccccagtggaccgggaaaacctgccaactcgacgccaatgagtgtgaggccaagccctgcgtgaacgccaagtcgtgcaaaaacctgatcgccagctactactgcgactgcctgcccggctggatggggcagaactgcgacatcaacatcaacgactgcctggggcagtgccagaatgacgctagctgccgagacctggtcaatggataccggtgcatatgccccccgggctacgccggcgaccattgcgagcgggacatcgacgagtgcgccagcaacccatgcctgaacggcgggcactgccagaacgaaataaacaggttccagtgtctgtgcccgacgggctttagcggcaacctctgccagttggatatcgactattgcgagcctaacccttgccagaacggcgcccagtgctataaccgcgcaagcgattatttctgcaaatgccccgaggactacgagggcaagaattgcagccatctgaaagaccactgtcggacgaccccctgcgaggtgatcgacagctgcaccgtggccatggcctccaacgacacccccgaaggggtgcgctatatctccagcaacgtgtgcggcccccacggcaagtgcaagagccagtcagggggcaaattcacctgcgactgcaacaagggcttcaccgggacctactgccacgagaacatcaacgactgcgagagcaacccctgccggaacggcggcacctgcatcgatggggtgaactcctataagtgcatctgtagcgatggatgggagggggcctactgcgaaaccaacatcaacgactgcagccagaacccctgccacaacgggggcacctgcagggacctcgtgaacgacttctactgcgactgcaagaacggctggaagggcaagacatgccactcccgggactcacaatgcgacgaagcgacctgcaacaatggcggcacctgttacgatgagggggatgcctttaagtgcatgtgccccggtggctgggagggcaccacctgcaatatcgccaggaattcctcctgcctgcccaacccctgccataatggcgggacctgcgtcgtgaacggcgagagcttcacctgcgtgtgcaaagaggggtgggaaggacccatctgcgcccaaaatacgaacgactgcagcccccacccctgttacaacagcggcacgtgcgtggatggggacaactggtaccgctgcgagtgcgcccccggctttgcaggcccggactgtcggatcaacatcaacgagtgccagagcagcccctgcgccttcggagccacgtgcgtggacgagatcaatggctacagatgcgtgtgccccccgggacacagcggcgccaagtgccaggaagtgtccggccgtccctgcatcaccatgggtagcgtcatccccgacggcgccaagtgggacgatgactgcaacacgtgtcagtgtctgaacggccgaatcgcctgctccaaggtgtggtgcggcccccggccctgcctgctgcacaagggccacagcgagtgccccagcggccagtcgtgtatccccatcctcgacgaccaatgcttcgtgcacccctgcaccggcgtgggcgagtgccgcagctcgagcctgcagcccgtgaagaccaagtgcaccagcgatagctactaccaggacaattgcgccaacatcaccttcacctttaacaaggagatgatgagccccggcctgacgaccgaacacatctgctccgagctgaggaacctgaacatcctgaagaatgtcagcgctgagtactccatctacatcgcctgtgagcccagcccaagcgccaacaatgagatccacgtcgcgatctccgccgaggacatccgcgacgatggcaaccccatcaaggagatcaccgacaagatcatcgacctggtgagcaagagggacggcaacagctccctgatcgccgcggtggccgaggtgagggtccaaaggaggcccctgaagaacaggaccgacttcctggtgcccctgctgtcgagcgtgctgaccgtggcctggatctgctgcctggtgaccgcgttctactggtgcctgcgtaagaggaggaagcccggcagccacacccatagcgcgtccgaggataacaccaccaataacgtgagggagcagctcaaccagatcaagaacccaatcgagaagcacggtgccaacactgtgcccatcaaggactatgagaacaagaacagcaagatgagtaagatcaggacacacaactccgaggtggaagaagacgacatggacaagcaccagcagaaggcccggttcgccaagcagcccgcctacaccctggtggacagggaagagaaaccccccaacggtacacccacgaaacaccccaactggaccaataagcaggacaacagggacctggagtccgcccagagtctgaacaggatggagtacatcgtg

SEQ ID NO: 33 - DNA, 3654 bp, Artificial Sequence
  Synthetic polynucleotide
atgcggtccccccggaccaggggtaggagcggccgcccactgtccctgctgctggccctgctgtgtgccctgagggccaaggtgtgcggcgcctccggacaattcgagctggagattctctcgatgcagaacgtgaacggcgaactgcagaacggaaattgctgtggcggcgccaggaatcccggcgatagaaagtgcaccagggacgagtgtgacacgtacttcaaggtgtgcctgaaggagtaccagagccgcgtgaccgccggcgggccctgctccttcgggtcaggcagcacccccgtgatcggcgggaacaccttcaacctcaaggcctccaggggcaacgacaggaataggatcgtgctccccttcagcttcgcctggcccaggtcctacaccctgctggtagaggcctgggactccagcaacgacaccgtgcagcccgatagcatcatcgagaaggctagccacagcggaatgatcaaccccagccgccagtggcagaccctgaaacagaacaccggcgtagcccactttgagtaccagatcagggtgacctgcgacgactattactatggcttcggttgcaacaagttctgccggcctcgcgacgacttcttcggacactacgcctgtgatcagaacgggaacaagacctgtatggagggttggatgggccccgaatgcaacagggccatctgcaggcagggctgctcccccaagcacgggagctgcaagctgcccggcgactgccggtgccagtacggctggcagggtctgtactgcgacaagtgcatcccccatcctggctgcgtgcacggcatatgcaacgagccctggcagtgcctgtgcgagaccaattggggcggccagctgtgcgacaaggacctgaattactgtggcacccaccagccctgcctcaacggcggcacctgctccaacaccggccccgacaagtaccagtgcagctgccccgaaggctacagcggcccgaattgcgagatcgccgaacacgcctgcctcagcgacccctgccacaaccggggcagctgtaaggagacctccctgggctttgaatgcgaatgtagccccggttggaccggacccacctgttccaccaacatcgacgactgcagccccaataactgcagccacggtggcacgtgccaggacctcgtcaacggctttaagtgcgtgtgccccccccagtggaccgggaagacctgccagctggacgccaacgagtgcgaggccaagccctgcgtgaacgccaagagctgcaagaacctcatcgccagctactattgtgactgcctgcccgggtggatgggccagaactgtgacataaacatcaacgattgtctgggccagtgccagaacgatgccagctgtcgggacctggtgaacggctaccggtgcatctgtccccccggctacgccggagatcactgtgagcgagacatcgacgagtgcgcctccaacccctgcctcaacggcgggcactgtcagaatgagatcaacaggttccagtgcctgtgcccgacgggattctccggtaacctgtgccagctcgacatcgactactgtgagcccaacccctgtcaaaatggcgcccaatgctacaaccgggcctccgactacttctgtaagtgccccgaggattacgagggtaagaactgtagccatctgaaggaccactgcaggactaccccgtgcgaggtgatcgactcctgcaccgtcgccatggcctccaacgacacccccgagggcgtgcggtacatcagcagcaacgtgtgtgggccgcacggcaagtgcaagagccagagcgggggcaagttcacctgtgattgcaacaagggcttcaccgggacgtattgccacgagaacatcaacgactgcgagagcaacccctgcaggaacggggggacctgcatagacggcgtgaacagctacaaatgcatctgcagcgatgggtgggagggcgcctactgtgagaccaacattaacgactgcagccagaacccctgccacaacgggggtacctgtcgcgacctggtgaacgacttctactgtgactgcaagaacggctggaagggcaagacctgtcattcccgcgacagccagtgcgacgaagccacctgcaacaacggcggcacctgctacgacgagggcgatgccttcaagtgcatgtgcccgggcggctgggaggggaccacctgtaatatcgccaggaattccagctgcctccccaatccgtgccataatggcggcacctgcgtggtcaacggcgaaagctttacctgcgtctgtaaggaaggctgggaaggtccgatctgtgcccagaacaccaacgactgtagcccccacccctgctacaatagcggaacgtgcgtggacggcgacaactggtatcggtgcgagtgcgcccccggctttgcggggccggactgccggatcaatatcaacgagtgccagagcagcccctgcgccttcggcgccacctgcgtggacgagatcaacggctacaggtgcgtgtgtccccccggccactccggcgccaagtgccaggaggtgagcggtaggccctgcatcaccatgggcagcgtgatccccgacggggccaagtgggacgatgactgtaacacctgccagtgcctgaacgggaggatcgcctgttccaaagtgtggtgcggcccgcgtccctgcctactccacaaggggcattccgagtgtcccagcggacagagctgtatccccatcctggacgaccaatgcttcgtgcacccctgcaccggcgtgggtgagtgcaggtccagcagcctgcagcccgtgaagacaaagtgcaccagtgattcctactaccaggataactgcgccaacatcaccttcaccttcaataaggagatgatgagcccgggcctgaccacggagcacatctgcagcgagctgcgcaacctgaacatcctgaagaacgtctccgccgagtacagcatatacatcgcctgcgagcccagcccctccgccaataacgagatccacgtggccatctccgcggaggacatcagggacgatggcaaccccatcaaggagatcaccgacaagattatcgacctggtcagcaaaagggacggcaactccagcctcatcgccgccgtggccgaggtcagggtacagcgcaggccgctgaaaaaccggaccgacttcctggtgcccctgctttcctccgtgctcacggtggcctggatttgctgcctggtaaccgcgttttactggtgcctgaggaagaggaggaagcccggcagccatacccacagcgccagcgaggacaacacaaccaacaacgtgagggagcagctcaaccagataaagaaccccatcgagaaacacggcgccaacacggtgcccatcaaggactatgagaacaagaacagcaagatgagcaagatccgcacccacaacagcgaggttgaggaagacgacatggacaagcaccagcagaaggccaggttcgccaagcagcccgcctacaccctggtggatcgtgaggagaaaccgcccaacgggacccccaccaagcatcccaattggaccaacaaacaggacaacagggacctggagtccgcccaaagcctgaaccggatggagtacatcgtc

SEQ ID NO: 34 - DNA, 3654 bp, Artificial Sequence
  Synthetic polynucleotide
atgaggtcccccagaactcgggggaggtccggcaggccgctcagcctcctgctcgccctgctgtgcgccctgagggccaaggtgtgcggcgcctccggccagttcgagctggagattctgagcatgcagaacgtgaacggcgaactgcagaacggaaactgctgcggtggggccaggaaccccggcgaccggaagtgcaccagggatgaatgcgacacctacttcaaggtctgcctcaaggagtaccagagcagggtgaccgccgggggcccgtgtagcttcggctccggcagcacccccgtgataggcggcaacacgttcaaccttaaagcctccaggggcaacgaccgcaacaggatcgtgctgcccttctccttcgcgtggccccgcagctacaccctgctggtggaggcgtgggatagcagcaacgacaccgtccagcccgattcaatcatcgaaaaggccagccacagcggcatgatcaacccctccaggcagtggcagaccctgaagcaaaacaccggcgtggcccacttcgagtaccaaatcagggttacctgcgacgactactactatgggttcggctgcaataagttctgtcggccgcgggacgactttttcgggcattatgcctgcgaccagaatggcaataagacctgcatggagggctggatgggacccgagtgcaaccgcgccatctgcaggcagggctgctcccccaagcacggcagctgcaagctgcccggcgactgcaggtgccagtacgggtggcagggcctctactgcgacaagtgcatcccccaccccggctgcgtgcatgggatatgcaacgagccgtggcagtgcctgtgcgaaaccaactgggggggccagctgtgcgataaggacctcaactactgcggcacccaccagccctgcctcaacggcggcacctgctccaataccgggcccgataaataccagtgctcctgccctgagggctacagcgggcccaactgtgagatcgccgagcatgcctgcctctcggacccctgccataacaggggcagctgtaaggaaaccagcctgggcttcgagtgcgagtgcagccccgggtggaccgggccaacctgctccaccaacatcgacgactgtagcccgaacaactgctcccacggcgggacctgccaggacctggtgaatggcttcaagtgcgtatgtcccccacagtggaccggcaagacctgtcaactcgacgccaacgagtgcgaggccaaaccctgcgtgaacgccaagtcctgcaagaacctgatcgcctcctactactgcgactgtctgcccggctggatgggccagaactgcgatatcaacatcaacgattgcctcggccagtgtcagaacgacgcctcctgccgggacctggtgaacggctaccggtgcatttgccccccgggctacgccggcgatcactgcgagcgcgacatcgacgagtgcgcatccaacccctgtctgaacggggggcactgtcagaacgagatcaataggttccagtgcctgtgccccaccggcttctccgggaatctgtgccagctggacatcgattactgcgagcccaacccctgccagaacggcgcccagtgttacaacagggccagcgattacttctgcaagtgtcccgaagactatgagggcaagaattgcagccatctgaaagaccactgccgcaccaccccctgtgaggtgatcgactcgtgcaccgtggcgatggccagcaatgacaccccggagggcgtgcggtacatcagcagcaacgtgtgtgggccccacggcaagtgcaagtcccagagcgggggcaagttcacctgcgactgcaacaaaggctttacagggacatattgccacgaaaacatcaatgactgcgagagcaacccctgccgcaatggcggcacttgcatcgacggcgtgaacagctacaaatgtatctgctcagacgggtgggaaggcgcgtattgcgagaccaacatcaacgattgtagccagaatccctgccataacggtggtacctgccgggatctggtgaacgacttctattgcgactgcaagaacggctggaagggcaagacctgccattcgagggatagccagtgcgacgaggccacctgcaacaacggcggcacctgctacgacgagggcgatgccttcaagtgcatgtgccctggcggctgggagggcaccacctgcaacatcgccaggaacagctcctgcctgcccaacccctgccacaacggcgggacctgtgtcgtgaacggggagagcttcacgtgcgtgtgcaaggagggctgggaagggcccatctgcgcccaaaacaccaacgactgcagcccccatccctgttacaactccggcacctgcgtggacggcgacaactggtaccgatgcgagtgcgcccccggcttcgccggccccgactgccggatcaacatcaacgagtgccagagcagcccctgcgcgttcggcgccacctgcgtggatgaaatcaacggatataggtgcgtgtgcccccccggccacagcggggccaagtgccaggaggtcagcgggcgcccctgcatcaccatgggcagcgtgatacccgacggcgccaagtgggacgacgactgcaacacctgccagtgcctgaacggcaggatcgcctgctccaaggtgtggtgcgggccgcggccgtgcctgctgcacaagggccacagcgagtgccccagcggccagtcctgtatcccaatcctggacgaccagtgcttcgtgcatccctgcaccggcgtgggcgagtgcaggtcctcctccctgcagcccgtgaagaccaaatgcaccagcgactcgtactaccaggataactgcgccaacatcaccttcaccttcaacaaggaaatgatgagccccggcctgaccaccgagcacatctgcagcgagctccggaacctgaacatcctgaagaacgtgtccgccgagtatagcatctacatcgcgtgcgaaccaagtccgtccgccaacaacgagatccacgtggcaatctccgccgaggacatccgggacgacggcaaccccatcaaggagataaccgacaaaatcatcgacctggtgagcaaaagggacggcaattctagcctgatcgccgcagtggccgaagtgagggtgcagcgcaggcccctcaagaataggaccgacttcctggtgccgctcctcagcagcgtgctgaccgtggcctggatctgctgcctggtgaccgccttttactggtgcctgaggaagcgtaggaagcccggaagccacacacactccgccagcgaggacaacaccaccaacaacgtgcgggagcaactgaaccagatcaagaaccccatcgagaagcacggagccaacaccgtccctatcaaagactacgagaacaagaacagcaagatgagcaagatcaggacccacaacagcgaggttgaggaagacgacatggacaagcaccagcagaaagccaggttcgcgaagcagcccgcctacaccctggtggaccgggaggaaaagccccccaacggcacccccaccaagcacccgaactggaccaacaagcaggacaacagggacctggagagcgcccagagcctgaaccggatggagtacatcgtc

SEQ ID NO: 35 - DNA, 3654 bp, Artificial Sequence
  Synthetic polynucleotide
atgcgcagcccccggaccaggggaaggtccggcaggcccctgtccctgctgctggcgctgctctgcgccctgcgagccaaagtgtgtggtgcctccgggcagtttgagctggagatcctcagcatgcagaacgtgaacggggagctgcagaatgggaactgctgcggcggcgccaggaatcccggggacaggaagtgcacccgagatgagtgcgacacctatttcaaggtgtgcctgaaggagtaccagagccgtgtgacggccggcggcccctgcagctttggcagcggcagcacccccgtgatcggcggaaacacattcaacctgaaggccagcaggggcaacgacaggaacaggatcgtgctgcccttcagcttcgcctggcccaggtcctacaccctgctggtggaggcctgggatagcagcaatgacaccgtgcagcccgactccatcatcgagaaggccagtcactctggaatgatcaacccgagcaggcagtggcagaccctgaagcagaacaccggcgtggcccacttcgagtaccagatcagggtgacctgtgacgattactactacggttttggctgcaacaagttctgtaggccccgcgacgacttctttggtcattacgcctgcgatcagaacggcaataagacctgcatggaaggctggatgggccccgaatgcaacagggccatttgcaggcaggggtgcagcccgaagcacggcagctgcaagctgcccggcgactgcaggtgtcagtacggctggcagggcctgtactgcgacaaatgcatcccccaccctgggtgcgtgcacggcatctgtaacgagccctggcagtgcctgtgtgagaccaactggggtgggcaactgtgcgataaggacctgaactactgcggaacccaccagccctgcctgaacggcggcacatgcagcaacaccgggcccgacaagtaccagtgcagctgccccgaagggtatagcgggcccaattgcgaaatcgccgagcacgcctgcctgagcgatccctgtcataatcgcggatcctgcaaggagaccagcctcggctttgagtgcgaatgctcccccggctggaccggtcccacgtgcagcacgaacatcgacgactgttccccgaacaactgctcccacggcggcacctgccaggatctggtgaatggattcaaatgcgtgtgccccccccaatggaccgggaagacctgccaactggacgccaacgagtgcgaagccaagccctgtgtgaacgccaagagctgcaaaaacctcatcgctagctactactgcgactgcctgcccggctggatgggtcagaactgtgacatcaacatcaacgattgtctgggccagtgccagaacgacgccagctgcagggacctggtgaatgggtaccgctgcatctgcccccccggctacgccggagatcattgcgagcgggacatcgacgagtgcgccagcaacccctgcctgaacggcggtcactgtcagaatgagatcaaccgcttccagtgcctgtgccccaccggcttcagcggaaatctgtgccagctagacattgattactgcgaaccgaacccttgccagaacggcgcccagtgctacaacagggccagcgactacttttgcaagtgccccgaggactacgaggggaagaattgctcccacctaaaggaccactgccggaccaccccctgcgaggtgatcgacagctgcaccgtcgcgatggccagcaacgacacccccgagggcgtcaggtacatctccagcaacgtgtgcggtccccatggcaaatgcaagagccagagcggggggaagtttacctgcgactgcaacaagggcttcaccgggacctactgccatgagaacatcaatgactgcgagagcaacccctgcaggaacggcgggacatgcatcgacggggtgaactcctataagtgcatctgctccgacgggtgggaaggtgcctattgcgagacaaacatcaacgactgcagccaaaacccctgccacaacgggggcacctgcagggatctggtgaacgacttctactgtgactgcaagaacgggtggaagggaaagacctgtcacagccgggactcccagtgcgacgaggccacatgcaacaacggcggcacgtgctacgacgaaggagacgcctttaagtgcatgtgccccggcggctgggagggcaccacctgcaatatcgcccgcaactcctcctgcctgcccaacccgtgccacaacgggggcacctgcgtggtgaacggcgagtccttcacctgcgtctgcaaggagggctgggagggtcccatctgtgcccagaataccaatgactgcagcccccatccttgttacaattccggcacctgcgtggatggcgacaactggtatcggtgtgagtgcgcccccggcttcgcgggccccgactgtaggatcaacatcaacgagtgccagagctccccatgcgcgtttggggcgacctgtgtcgacgagatcaatgggtacaggtgcgtgtgtcccccggggcactccggggccaaatgccaggaggtaagcggccggccatgcattaccatgggctcggtgatcccagacggtgccaagtgggacgacgactgcaacacctgccagtgcctgaatggcaggatcgcctgcagcaaggtatggtgcggacccaggccgtgcctgctgcacaaaggacactccgagtgtccgagcggccagagctgcatccccatcctggacgaccagtgcttcgtgcatccctgcactggcgtcggcgagtgccgcagctccagcctgcagcccgtgaagaccaagtgtaccagcgacagctactaccaggacaattgtgccaacatcaccttcaccttcaacaaggagatgatgagccctggcctgaccaccgagcatatctgtagcgagctgaggaacttgaacatcctgaagaatgtgagcgccgagtattccatttacatagcctgtgagcccagcccaagcgctaacaatgagatccacgtggccatcagcgccgaggacatccgggacgacggcaaccccatcaaagaaatcaccgacaagatcatcgatctggtaagcaagagggacgggaacagcagcctcatcgccgccgtggccgaggtgcgcgtccagcggaggcccctcaaaaaccggaccgactttctggtgccgctgctcagctccgtgctgaccgtggcctggatatgctgcctggtgaccgccttctactggtgcctgcggaagaggaggaagcccggcagccacacgcacagcgcgagcgaggacaacaccaccaacaacgtgcgggagcaactgaaccagatcaagaaccccatcgagaagcacggcgccaacaccgtgcccatcaaggactacgagaacaagaatagcaagatgagtaagattaggacccacaacagcgaggtggaggaggacgacatggacaagcaccagcagaaggcccgcttcgccaagcagcccgcctataccctggtcgacagggaagagaagccgcccaatgggacccccaccaagcatcccaactggaccaacaagcaggacaaccgggatctggagagcgcccaaagcctgaataggatggagtacatcgtg

SEQ ID NO: 36 - RNA, 47 nt, Artificial Sequence
  Synthetic polynucleotide
gggaaauaagagagaaaagaagaguaagaagaaauauaagagccacc

SEQ ID NO: 37 - RNA, 47 nt, Artificial Sequence
  Synthetic polynucleotide
gggagaucagagagaaaagaagaguaagaagaaauauaagagccacc

SEQ ID NO: 38 - RNA, 145 nt, Artificial Sequence
  Synthetic polynucleotide
ggaauaaaagucucaacacaacauauacaaaacaaacgaaucucaagcaaucaagcauucuacuucuauugcagcaauuuaaaucauuucuuuuaaagcaaaagcaauuuucugaaaauuuucaccauuuacgaacgauagcaac

SEQ ID NO: 39 - RNA, 42 nt, Artificial Sequence
  Synthetic polynucleotide
gggagacaagcuuggcauuccgguacuguugguaaagccacc

SEQ ID NO: 40 - RNA, 47 nt, Artificial Sequence; identical to SEQ ID NO: 37
  Synthetic polynucleotide

SEQ ID NO: 41 - RNA, 145 nt, Artificial Sequence; identical to SEQ ID NO: 38
  Synthetic polynucleotide

SEQ ID NO: 42 - RNA, 42 nt, Artificial Sequence; identical to SEQ ID NO: 39
  Synthetic polynucleotide

SEQ ID NO: 43 - RNA, 47 nt, Artificial Sequence
  Synthetic polynucleotide
gggaauuaacagagaaaagaagaguaagaagaaauauaagagccacc

SEQ ID NO: 44 - RNA, 47 nt, Artificial Sequence
  Synthetic polynucleotide
gggaaauuagacagaaaagaagaguaagaagaaauauaagagccacc

SEQ ID NO: 45 - RNA, 47 nt, Artificial Sequence
  Synthetic polynucleotide
gggaaauaagagaguaaagaacaguaagaagaaauauaagagccacc

SEQ ID NO: 46 - RNA, 47 nt, Artificial Sequence
  Synthetic polynucleotide
gggaaaaaagagagaaaagaagacuaagaagaaauauaagagccacc

SEQ ID NO: 47 - RNA, 47 nt, Artificial Sequence
  Synthetic polynucleotide
gggaaauaagagagaaaagaagaguaagaagauauauaagagccacc

SEQ ID NO: 48 - RNA, 47 nt, Artificial Sequence
  Synthetic polynucleotide
gggaaauaagagacaaaacaagaguaagaagaaauauaagagccacc

SEQ ID NO: 49 - RNA, 47 nt, Artificial Sequence
  Synthetic polynucleotide
gggaaauuagagaguaaagaacaguaaguagaauuaaaagagccacc

SEQ ID NO: 50 - RNA, 47 nt, Artificial Sequence
  Synthetic polynucleotide
gggaaauaagagagaauagaagaguaagaagaaauauaagagccacc

SEQ ID NO: 51 - RNA, 47 nt, Artificial Sequence
  Synthetic polynucleotide
gggaaauaagagagaaaagaagaguaagaagaaaauuaagagccacc

SEQ ID NO: 52 - RNA, 47 nt, Artificial Sequence
  Synthetic polynucleotide
gggaaauaagagagaaaagaagaguaagaagaaauuuaagagccacc

SEQ ID NO: 53 - RNA, 92 nt, Artificial Sequence
  Synthetic polynucleotide
ucaagcuuuuggacccucguacagaagcuaauacgacucacuauagggaaauaagagagaaaagaagaguaagaagaaauauaagagccacc

SEQ ID NO: 54 - RNA, 142 nt, Artificial Sequence
  Synthetic polynucleotide
ugauaauaguccauaaaguaggaaacacuacagcuggagccucgguggccaugcuucuugccccuugggccuccccccagccccuccuccccuuccugcacccguacccccguggucuuugaauaaagucugagugggcggc

SEQ ID NO: 55 - RNA, 142 nt, Artificial Sequence
  Synthetic polynucleotide
ugauaauaggcuggagccucgguggcuccauaaaguaggaaacacuacacaugcuucuugccccuugggccuccccccagccccuccuccccuuccugcacccguacccccguggucuuugaauaaagucugagugggcggc

SEQ ID NO: 56 - RNA, 142 nt, Artificial Sequence
  Synthetic polynucleotide
ugauaauaggcuggagccucgguggccaugcuucuugccccuuccauaaaguaggaaacacuacaugggccuccccccagccccuccuccccuuccugcacccguacccccguggucuuugaauaaagucugagugggcggc

SEQ ID NO: 57 - RNA, 142 nt, Artificial Sequence
  Synthetic polynucleotide
ugauaauaggcuggagccucgguggccaugcuucuugccccuugggccuccccccaguccauaaaguaggaaacacuacaccccuccuccccuuccugcacccguacccccguggucuuugaauaaagucugagugggcggc

SEQ ID NO: 58 - RNA, 142 nt, Artificial Sequence
  Synthetic polynucleotide
ugauaauaggcuggagccucgguggccaugcuucuugccccuugggccuccccccagccccuccuccccuucuccauaaaguaggaaacacuacacugcacccguacccccguggucuuugaauaaagucugagugggcggc

SEQ ID NO: 59 - RNA, 142 nt, Artificial Sequence
  Synthetic polynucleotide
ugauaauaggcuggagccucgguggccaugcuucuugccccuugggccuccccccagccccuccuccccuuccugcacccguacccccuccauaaaguaggaaacacuacaguggucuuugaauaaagucugagugggcggc

SEQ ID NO: 60 - RNA, 142 nt, Artificial Sequence
  Synthetic polynucleotide
ugauaauaggcuggagccucgguggccaugcuucuugccccuugggccuccccccagccccuccuccccuuccugcacccguacccccguggucuuugaauaaaguuccauaaaguaggaaacacuacacugagugggcggc

SEQ ID NO: 61 - RNA, 371 nt, Artificial Sequence
  Synthetic polynucleotide
gcgccugcccaccugccaccgacugcuggaacccagccagugggagggccuggcccaccagaguccugcucccucacuccucgccccgcccccugucccagagucccaccugggggcucucuccacccuucucagaguuccaguuucaaccagaguuccaaccaaugggcuccauccucuggauucuggccaaugaaauaucucccuggcaggguccucuucuuuucccagagcuccaccccaaccaggagcucuaguuaauggagagcucccagcacacucggagcuugugcuuugucuccacgcaaagcgauaaauaaaagcauugguggccuuuggucuuugaauaaagccugaguaggaagucuaga

SEQ ID NO: 62 - RNA, 568 nt, Artificial Sequence
  Synthetic polynucleotide
gccccugccgcucccacccccacccaucugggccccggguucaagagagagcggggucugaucucguguagccauauagaguuugcuucugagugucugcuuuguuuaguagaggugggcaggaggagcugaggggcuggggcugggguguugaaguuggcuuugcaugcccagcgaugcgccucccugugggaugucaucacccugggaaccgggaguggcccuuggcucacuguguucugcaugguuuggaucugaauuaauuguccuuucuucuaaaucccaaccgaacuucuuccaaccuccaaacuggcuguaaccccaaauccaagccauuaacuacaccugacaguagcaauugucugauuaaucacuggccccuugaagacagcagaaugucccuuugcaaugaggaggagaucugggcugggcgggccagcuggggaagcauuugacuaucuggaacuugugugugccuccucagguauggcagugacucaccugguuuuaauaaaacaaccugcaacaucucauggucuuugaauaaagccugaguaggaagucuaga

SEQ ID NO: 63 - RNA, 289 nt, Artificial Sequence
  Synthetic polynucleotide
acacacuccaccuccagcacgcgacuucucaggacgacgaaucuucucaaugggggggcggcugagcuccagccaccccgcagucacuuucuuuguaacaacuuccguugcugccaucguaaacugacacaguguuuauaacguguacauacauuaacuuauuaccucauuuuguuauuuuucgaaacaaagcccuguggaagaaaauggaaaacuugaagaagcauuaaagucauucuguuaagcugcguaaauggucuuugaauaaagccugaguaggaagucuaga

SEQ ID NO: 64 - RNA, 379 nt, Artificial Sequence
  Synthetic polynucleotide
caucacauuuaaaagcaucucagccuaccaugagaauaagagaaagaaaaugaagaucaaaagcuuauucaucuguuuuucuuuuucguugguguaaagccaacacccugucuaaaaaacauaaauuucuuuaaucauuuugccucuuuucucugugcuucaauuaauaaaaaauggaaagaaucuaauagagugguacagcacuguuauuuuucaaagauguguugcuauccugaaaauucuguagguucuguggaaguuccaguguucucucuuauuccacuucgguagaggauuucuaguuucuugugggcuaauuaaauaaaucauuaauacucuucuaauggucuuugaauaaagccugaguaggaagucuaga

SEQ ID NO: 65 - RNA, 118 nt, Artificial Sequence
  Synthetic polynucleotide
gcugccuucugcggggcuugccuucuggccaugcccuucuucucucccuugcaccuguaccucuuggucuuugaauaaagccugaguaggaaggcggccgcucgagcaugcaucuaga

SEQ ID NO: 66 - RNA, 908 nt, Artificial Sequence
  Synthetic polynucleotide
gccaagcccuccccaucccauguauuuaucucuauuuaauauuuaugucuauuuaagccucauauuuaaagacagggaagagcagaacggagccccaggccucuguguccuucccugcauuucugaguuucauucuccugccuguagcagugagaaaaagcuccuguccucccauccccuggacugggagguagauagguaaauaccaaguauuuauuacuaugacugcuccccagcccuggcucugcaaugggcacugggaugagccgcugugagccccugguccugaggguccccaccugggacccuugagaguaucaggucucccacgugggagacaagaaaucccuguuuaauauuuaaacagcaguguuccccaucuggguccuugcaccccucacucuggccucagccgacugcacagcggccccugcauccccuuggcugugaggccccuggacaagcagagguggccagagcugggaggcauggcccuggggucccacgaauuugcuggggaaucucguuuuucuucuuaagacuuuugggacaugguuugacucccgaacaucaccgacgcgucuccuguuuuucuggguggccucgggacaccugcccugcccccacgagggucaggacugugacucuuuuuagggccaggcaggugccuggacauuugccuugcuggacggggacuggggaugugggagggagcagacaggaggaaucaugucaggccugugugugaaaggaagcuccacugucacccuccaccucuucaccccccacucaccaguguccccuccacugucacauuguaacugaacuucaggauaauaaaguguuugccuccauggucuuugaauaaagccugaguaggaaggcggccgcucgagcaugcaucuaga

SEQ ID NO: 67 - RNA, 835 nt, Artificial Sequence
  Synthetic polynucleotide
acucaaucuaaauuaaaaaagaaagaaauuugaaaaaacuuucucuuugccauuucuucuucuucuuuuuuaacugaaagcugaauccuuccauuucuucugcacaucuacuugcuuaaauugugggcaaaagagaaaaagaaggauugaucagagcauugugcaauacaguuucauuaacuccuucccccgcucccccaaaaauuugaauuuuuuuuucaacacucuuacaccuguuauggaaaaugucaaccuuuguaagaaaaccaaaauaaaaauugaaaaauaaaaaccauaaacauuugcaccacuuguggcuuuugaauaucuuccacagagggaaguuuaaaacccaaacuuccaaagguuuaaacuaccucaaaacacuuucccaugagugugauccacauuguuaggugcugaccuagacagagaugaacugagguccuuguuuuguuuuguucauaauacaaaggugcuaauuaauaguauuucagauacuugaagaauguugauggugcuagaagaauuugagaagaaauacuccuguauugaguuguaucgugugguguauuuuuuaaaaaauuugauuuagcauucauauuuuccaucuuauucccaauuaaaaguaugcagauuauuugcccaaaucuucuucagauucagcauuuguucuuugccagucucauuuucaucuucuuccaugguuccacagaagcuuuguuucuugggcaagcagaaaaauuaaauuguaccuauuuuguauaugugagauguuuaaauaaauugugaaaaaaaugaaauaaagcauguuugguuuuccaaaagaacauau

SEQ ID NO: 68 - RNA, 297 nt, Artificial Sequence
  Synthetic polynucleotide
cgccgccgcccgggccccgcagucgagggucgugagcccaccccguccauggugcuaagcgggcccgggucccacacggccagcaccgcugcucacucggacgacgcccugggccugcaccucuccagcuccucccacgggguccccguagccccggcccccgcccagccccaggucuccccaggcccuccgcaggcugcccggccucccucccccugcagccaucccaaggcuccugaccuaccuggccccugagcucuggagcaagcccugacccaauaaaggcuuugaacccau

SEQ ID NO: 69 - RNA, 602 nt, Artificial Sequence
  Synthetic polynucleotide
ggggcuagagcccucuccgcacagcguggagacggggcaaggagggggguuauuaggauuggugguuuuguuuugcuuuguuuaaagccgugggaaaauggcacaacuuuaccucugugggagaugcaacacugagagccaaggggugggaguugggauaauuuuuauauaaaagaaguuuuuccacuuugaauugcuaaaaguggcauuuuuccuaugugcagucacuccucucauuucuaaaauagggacguggccaggcacgguggcucaugccuguaaucccagcacuuugggaggccgaggcaggcggcucacgaggucaggagaucgagacuauccuggcuaacacgguaaaacccugucucuacuaaaaguacaaaaaauuagcugggcgugguggugggcaccuguagucccagcuacucgggaggcugaggcaggagaaaggcaugaauccaagaggcagagcuugcagugagcugagaucacgccauugcacuccagccugggcaacaguguuaagacucugucucaaauauaaauaaauaaauaaauaaauaaauaaauaaauaaaaauaaagcgagauguugcccucaaa

SEQ ID NO: 70 - RNA, 785 nt, Artificial Sequence
  Synthetic polynucleotide
ggcccugccccgucggacugcccccagaaagccuccugcccccugccagugaaguccuucagugagccccuccccagccagcccuucccuggccccgccggauguauaaauguaaaaaugaaggaauuacauuuuauaugugagcgagcaagccggcaagcgagcacaguauuauuucuccauccccucccugccugcuccuuggcacccccaugcugccuucagggagacaggcagggagggcuuggggcugcaccuccuacccucccaccagaacgcaccccacugggagagcugguggugcagccuuccccucccuguauaagacacuuugccaaggcucuccccucucgccccaucccugcuugcccgcucccacagcuuccugagggcuaauucugggaagggagaguucuuugcugccccugucuggaagacguggcucugggugagguaggcgggaaaggauggaguguuuuaguucuugggggaggccaccccaaaccccagccccaacuccaggggcaccuaugagauggccaugcucaaccccccucccagacaggcccucccugucuccagggcccccaccgagguucccagggcuggagacuuccucugguaaacauuccuccagccuccccuccccuggggacgccaaggaggugggccacacccaggaagggaaagcgggcagccccguuuuggggacgugaacguuuuaauaauuuuugcugaauuccuuuacaacuaaauaacacagauauuguuauaaauaaaauugu

SEQ ID NO: 71 - RNA, 3001 nt, Artificial Sequence
  Synthetic polynucleotide
auauuaaggaucaagcuguuagcuaauaaugccaccucugcaguuuugggaacaggcaaauaaaguaucaguauacauggugauguacaucuguagcaaagcucuuggagaaaaugaagacugaagaaagcaaagcaaaaacuguauagagagauuuuucaaaagcaguaaucccucaauuuuaaaaaaggauugaaaauucuaaaugucuuucugugcauauuuuuuguguuaggaaucaaaaguauuuuauaaaaggagaaagaacagccucauuuuagauguaguccuguuggauuuuuuaugccuccucaguaaccagaaauguuuuaaaaaacuaaguguuuaggauuucaagacaacauuauacauggcucugaaauaucugacacaauguaaacauugcaggcaccugcauuuuauguuuuuuuuuucaacaaaugugacuaauuugaaacuuuuaugaacuucugagcuguccccuugcaauucaaccgcaguuugaauuaaucauaucaaaucaguuuuaauuuuuuaaauuguacuucagagucuauauuucaagggcacauuuucucacuacuauuuuaauacauuaaaggacuaaauaaucuuucagagaugcuggaaacaaaucauuugcuuuauauguuucauuagaauaccaaugaaacauacaacuugaaaauuaguaauaguauuuuugaagaucccauuucuaauuggagaucucuuuaauuucgaucaacuuauaauguguaguacuauauuaagugcacuugaguggaauucaacauuugacuaauaaaaugaguucaucauguuggcaagugauguggcaauuaucucuggugacaaaagaguaaaaucaaauauuucugccuguuacaaauaucaaggaagaccugcuacuaugaaauagaugacauuaaucugucuucacuguuuauaauacggauggauuuuuuuucaaaucaguguguguuuugaggucuuauguaauugaugacauuugagagaaaugguggcuuuuuuuagcuaccucuuuguucauuuaagcaccaguaaagaucaugucuuuuuauagaaguguagauuuucuuugugacuuugcuaucgugccuaaagcucuaaauauaggugaaugugugaugaauacucagauuauuugucucucuauauaauuaguuugguacuaaguuucucaaaaaauuauuaacacaugaaagacaaucucuaaaccagaaaaagaaguaguacaaauuuuguuacuguaaugcucgcguuuagugaguuuaaaacacacaguaucuuuugguuuuauaaucaguuucuauuuugcugugccugagauuaagaucuguguaugugugugugugugugugugcguuuguguguuaaagcagaaaagacuuuuuuaaaaguuuuaagugauaaaugcaauuuguuaauugaucuuagaucacuaguaaacucagggcugaauuauaccauguauauucuauuagaagaaaguaaacaccaucuuuauuccugcccuuuuucuucucucaaaguaguuguaguuauaucuagaaagaagcaauuuugauuucuugaaaagguaguuccugcacucaguuuaaacuaaaaauaaucauacuuggauuuuauuuauuuuugucauaguaaaaauuuuaauuuauauauauuuuuauuuaguauuaucuuauucuuugcuauuugccaauccuuugucaucaauuguguuaaaugaauugaaaauucaugcccuguucauuuuauuuuacuuuauugguuaggauauuuaaaggauuuuuguauauauaauuucuuaaauuaauauuccaaaagguuaguggacuuagauuauaaauuauggcaaaaaucuaaaaacaacaaaaaugauuuuuauacauucuauuucauuauuccucuuuuuccaauaagucauacaauugguagauaugacuuauuuuauuuuuguauuauucacuauaucuuuaugauauuuaaguauaaauaauuaaaaaaauuuauuguaccuuauagucugucaccaaaaaaaaaaaauuaucuguagguagugaaaugcuaauguugauuugucuuuaagggcuuguuaacuauccuuuauuuucucauuugucuuaaauuaggaguuuguguuuaaauuacucaucuaagcaaaaaauguauauaaaucccauuacuggguauauacccaaaggauuauaaaucaugcugcuauaaagacacaugcacacguauguuuauugcagcacuauucacaauagcaaagacuuggaaccaacccaaauguccaucaaugauagacuugauuaagaaaaugugcacauauacaccauggaauacuaugcagccauaaaaaaggaugaguucauguccuuuguagggacauggauaaagcuggaaaccaucauucugagcaaacuauugcaaggacagaaaaccaaacacugcauguucucacucauaggugggaauugaacaaugagaacacuuggacacaagguggggaacaccacacaccagggccugucaugggguggggggaguggggagggauagcauuaggagauauaccuaauguaaaugaugaguuaaugggugcagcacaccaacauggcacauguauacauauguagcaaaccugcacguugugcacauguacccuagaacuuaaaguauaauuaaaaaaaaaaagaaaacagaagcuauuuauaaagaaguuauuugcugaaauaaaugugaucuuucccauuaaaaaaauaaagaaauuuugggguaaaaaaacacaauauauuguauucuugaaaaauucuaagagaguggaugugaaguguucucaccacaaaagugauaacuaauugagguaaugcacauauuaauuagaaagauuuugucauuccacaauguauauauacuuaaaaauauguuauacacaauaaauacauacauuaaaaaauaaguaaaugua

SEQ ID NO: 72 - RNA, 1037 nt, Artificial Sequence
  Synthetic polynucleotide
cccacccugcacgccggcaccaaacccuguccucccaccccuccccacucaucacuaaacagaguaaaaugugaugcgaauuuucccgaccaaccugauucgcuagauuuuuuuuaaggaaaagcuuggaaagccaggacacaacgcugcugccugcuuugugcaggguccuccggggcucagcccugaguuggcaucaccugcgcagggcccucuggggcucagcccugagcuagugucaccugcacagggcccucugaggcucagcccugagcuggcgucaccugugcagggcccucuggggcucagcccugagcuggccucaccuggguuccccaccccgggcucuccugcccugcccuccugcccgcccucccuccugccugcgcagcuccuucccuaggcaccucugugcugcaucccaccagccugagcaagacgcccucucggggccugugccgcacuagccucccucuccucuguccccauagcugguuuuucccaccaauccucaccuaacaguuacuuuacaauuaaacucaaagcaagcucuucuccucagcuuggggcagccauuggccucugucucguuuugggaaaccaaggucaggaggccguugcagacauaaaucucggcgacucggccccgucuccugaggguccugcuggugaccggccuggaccuuggcccuacagcccuggaggccgcugcugaccagcacugaccccgaccucagagaguacucgcaggggcgcuggcugcacucaagacccucgagauuaacggugcuaaccccgucugcuccucccucccgcagagacuggggccuggacuggacaugagagccccuuggugccacagagggcugugucuuacuagaaacaacgcaaaccucuccuuccucagaauagugauguguucgacguuuuaucaaaggcccccuuucuauguucauguuaguuuugcuccuucuguguuuuuuucugaaccauauccauguugcugacuuuuccaaauaaagguuuucacuccucuc

SEQ ID NO: 73 - RNA, 577 nt, Artificial Sequence
  Synthetic polynucleotide
agaggccugccuccagggcuggacugaggccugagcgcuccugccgcagagcuggccgcgccaaauaaugucucugugagacucgagaacuuucauuuuuuuccaggcugguucggauuugggguggauuuugguuuuguuccccuccuccacucucccccacccccuccccgcccuuuuuuuuuuuuuuuuuuaaacugguauuuuaucuuugauucuccuucagcccucaccccugguucucaucuuucuugaucaacaucuuuucuugccucuguccccuucucucaucucuuagcuccccuccaaccuggggggcagugguguggagaagccacaggccugagauuucaucugcucuccuuccuggagcccagaggagggcagcagaaggggguggugucuccaaccccccagcacugaggaagaacggggcucuucucauuucaccccucccuuucuccccugcccccaggacugggccacuucuggguggggcagugggucccagauuggcucacacugagaauguaagaacuacaaacaaaauuucuauuaaauuaaauuuugugucucc

SEQ ID NO: 74 - RNA, 2212 nt, Artificial Sequence
  Synthetic polynucleotide
cucccuccaucccaaccuggcucccucccacccaaccaacuuuccccccaacccggaaacagacaagcaacccaaacugaacccccucaaaagccaaaaaaugggagacaauuucacauggacuuuggaaaauauuuuuuuccuuugcauucaucucucaaacuuaguuuuuaucuuugaccaaccgaacaugaccaaaaaccaaaagugcauucaaccuuaccaaaaaaaaaaaaaaaaaaagaauaaauaaauaacuuuuuaaaaaaggaagcuugguccacuugcuugaagacccaugcggggguaagucccuuucugcccguugggcuuaugaaaccccaaugcugcccuuucugcuccuuucuccacaccccccuuggggccuccccuccacuccuucccaaaucugucuccccagaagacacaggaaacaauguauugucugcccagcaaucaaaggcaaugcucaaacacccaaguggcccccacccucagcccgcuccugcccgcccagcacccccaggcccugggggaccugggguucucagacugccaaagaagccuugccaucuggcgcucccauggcucuugcaacaucuccccuucguuuuugagggggucaugccgggggagccaccagccccucacuggguucggaggagagucaggaagggccacgacaaagcagaaacaucggauuuggggaacgcgugucaaucccuugugccgcagggcugggcgggagagacuguucuguuccuuguguaacuguguugcugaaagacuaccucguucuugucuugaugugucaccggggcaacugccugggggcggggaugggggcaggguggaagcggcuccccauuuuauaccaaaggugcuacaucuaugugaugggugggguggggagggaaucacuggugcuauagaaauugagaugcccccccaggccagcaaauguuccuuuuuguucaaagucuauuuuuauuccuugauauuuuucuuuuuuuuuuuuuuuuuuuguggauggggacuugugaauuuuucuaaaggugcuauuuaacaugggaggagagcgugugcggcuccagcccagcccgcugcucacuuuccacccucucuccaccugccucuggcuucucaggccucugcucuccgaccucucuccucugaaacccuccuccacagcugcagcccauccucccggcucccuccuagucuguccugcguccucuguccccggguuucagagacaacuucccaaagcacaaagcaguuuuucccccuaggggugggaggaagcaaaagacucuguaccuauuuuguauguguauaauaauuugagauguuuuuaauuauuuugauugcuggaauaaagcauguggaaaugacccaaacauaauccgcaguggccuccuaauuuccuucuuuggaguugggggagggguagacauggggaaggggcuuuggggugaugggcuugccuuccauuccugcccuuucccuccccacuauucucuucuagaucccuccauaaccccacuccccuuucucucacccuucuuauaccgcaaaccuuucuacuuccucuuucauuuucuauucuugcaauuuccuugcaccuuuuccaaauccucuucuccccugcaauaccauacaggcaauccacgugcacaacacacacacacacucuucacaucugggguuguccaaaccucauacccacuccccuucaagcccauccacucuccacccccuggaugcccugcacuugguggcggugggaugcucauggauacugggagggugaggggaguggaacccgugaggaggaccugggggccucuccuugaacugacaugaagggucaucuggccucugcucccuucucacccacgcugaccuccugccgaaggagcaacgcaacaggagaggggucugcugagccuggcgagggucugggagggaccaggaggaaggcgugcucccugcucgcuguccuggcccugggggagugagggagacagacaccugggagagcuguggggaaggcacucgcaccgugcucuugggaaggaaggagaccuggcccugcucaccacggacugggugccucgaccuccugaauccccagaacacaaccccccugggcugggguggucuggggaaccaucgugcccccgccucccgccuacuccuuuuuaagcuu

SEQ ID NO: 75 - RNA, 729 nt, Artificial Sequence
  Synthetic polynucleotide
uuggccaggccugacccucuuggaccuuucuucuuugccgacaaccacugcccagcagccucugggaccucggggucccagggaacccaguccagccuccuggcuguugacuucccauugcucuuggagccaccaaucaaagagauucaaagagauuccugcaggccagaggcggaacacaccuuuauggcuggggcucuccgugguguucuggacccagccccuggagacaccauucacuuuuacugcuuuguagugacucgugcucuccaaccugucuuccugaaaaaccaaggcccccuucccccaccucuuccauggggugagacuugagcagaacaggggcuuccccaaguugcccagaaagacugucugggugagaagccauggccagagcuucucccaggcacagguguugcaccagggacuucugcuucaaguuuugggguaaagacaccuggaucagacuccaagggcugcccugagucugggacuucugccuccauggcuggucaugagagcaaaccguaguccccuggagacagcgacuccagagaaccucuugggagacagaagaggcaucugugcacagcucgaucuucuacuugccuguggggaggggagugacagguccacacaccacacugggucacccuguccuggaugccucugaagagagggacagaccgucagaaacuggagaguuucuauuaaaggucauuuaaacca

SEQ ID NO: 76 - RNA, 847 nt, Artificial Sequence
  Synthetic polynucleotide
uccuccgggaccccagcccucaggauuccugaugcuccaaggcgacugaugggcgcuggaugaaguggcacagucagcuucccugggggcuggugucauguugggcuccuggggcgggggcacggccuggcauuucacgcauugcugccaccccagguccaccugucuccacuuucacagccuccaagucuguggcucuucccuucuguccuccgaggggcuugccuucucucguguccagugaggugcucagugaucggcuuaacuuagagaagcccgcccccuccccuucuccgucugucccaagagggucugcucugagccugcguuccuagguggcucggccucagcugccuggguuguggccgcccuagcauccuguaugcccacagcuacuggaauccccgcugcugcuccgggccaagcuucugguugauuaaugagggcaugggguggucccucaagaccuuccccuaccuuuuguggaaccagugaugccucaaagacaguguccccuccacagcugggugccaggggcaggggauccucaguauagccggugaacccugauaccaggagccugggccucccugaaccccuggcuuccagccaucucaucgccagccuccuccuggaccucuuggcccccagccccuuccccacacagccccagaagggucccagagcugaccccacuccaggaccuaggcccagccccucagccucaucuggagccccugaagaccagucccacccaccuuucuggccucaucugacacugcuccgcauccugcuguguguccuguuccauguuccgguuccauccaaauacacuuucuggaacaaa

SEQ ID NO: 77 - RNA, 110 nt, Artificial Sequence
  Synthetic polynucleotide
gcuggagccucgguggccaugcuucuugccccuugggccuccccccagccccuccuccccuuccugcacccguacccccguggucuuugaauaaagucugagugggcggc

SEQ ID NO: 78 - RNA, 119 nt, Artificial Sequence
  Synthetic polynucleotide
ugauaauaggcuggagccucgguggccuagcuucuugccccuugggccuccccccagccccuccuccccuuccugcacccguacccccguggucuuugaauaaagucugagugggcggc

SEQ ID NO: 79 - RNA, 87 nt, Artificial Sequence
  Synthetic polynucleotide
gacagugcagucacccauaaaguagaaagcacuacuaacagcacuggaggguguaguguuuccuacuuuauggaugaguguacugug

SEQ ID NO: 80 - RNA, 23 nt, Artificial Sequence
  Synthetic polynucleotide
uguaguguuuccuacuuuaugga

SEQ ID NO: 81 - RNA, 23 nt, Artificial Sequence
  Synthetic polynucleotide
uccauaaaguaggaaacacuaca

SEQ ID NO: 82 - RNA, 21 nt, Artificial Sequence
  Synthetic polynucleotide
cauaaaguagaaagcacuacu

SEQ ID NO: 83 - RNA, 21 nt, Artificial Sequence
  Synthetic polynucleotide
aguagugcuuucuacuuuaug

SEQ ID NO: 84 - DNA, 92 bp, Artificial Sequence
  Synthetic polynucleotide
tcaagcttttggaccctcgtacagaagctaatacgactcactatagggaaataagagagaaaagaagagtaagaagaaatataagagccacc

SEQ ID NO: 85 - DNA, 119 bp, Artificial Sequence
  Synthetic polynucleotide
tgataataggctggagcctcggtggccatgcttcttgccccttgggcctccccccagcccctcctccccttcctgcacccgtacccccgtggtctttgaataaagtctgagtgggcggc

SEQ ID NO: 86 - DNA, 18 bp, Artificial Sequence
  Synthetic polynucleotide
attgggcacccgtaaggg

SEQ ID NO: 87 - RNA, 3654 nt, Artificial Sequence
  Synthetic polynucleotide
augcgaagccccaggacccgcggccguagcgguaggccccugucccugcugcuggcccugcugugcgcccucagggccaaggugugcggcgccagcggccaguucgagcucgagauccugagcaugcagaacgugaacggcgagcuccagaaugggaauuguugcggcggcgccaggaaccccggugacaggaaaugcacccgcgacgagugcgacaccuacuucaaagugugccucaaggaguaccagagcagggugaccgccggcgggcccugcagcuucgggagcggcuccacgcccgugaucggcgggaacaccuucaaccugaaggccagcaggggcaacgaucggaaccggaucgugcugccguucuccuucgccuggccgcgaagcuacacccugcugguggaagcgugggacagcagcaacgacaccgugcagcccgacagcaucaucgagaaggccucacacuccgguaugaucaaccccagcaggcaguggcagacccugaagcagaacaccggaguggcccacuucgaauaccagaucagggugacaugcgacgacuacuacuacggcuucgggugcaacaaguucugcaggccccgcgacgacuucuucggacacuacgccugugaccagaacgggaacaagacguguauggagggguggauggggcccgaaugcaacagggccaucugucggcaggguugcucccccaagcacggcuccugcaaacugcccggcgauugccggugccaguacggguggcaaggucuguacugcgacaagugcaucccgcaucccggcugcgugcacggcaucugcaacgagcccuggcagugccugugcgaaaccaacuggggcggccagcucugugacaaggaccuuaacuacugcggcacccaccagcccugccugaacggcgggaccugcagcaacaccgggcccgacaaguaccaguguagcugccccgaaggguacucgggucccaacugcgagaucgccgagcacgccugccuguccgaccccugccauaacaggggcagcuguaaggagaccucccugggcuucgagugugagugcucccccggauggaccggccccaccugcagcaccaauauugacgacugcagcccaaauaacugcucccacggcggcaccugccaggaccucgugaacggcuuuaagugcgucugucccccccaguggaccggcaagaccugccagcuggacgccaaugagugcgaggccaagcccuguguaaacgccaagagcugcaagaaccugaucgccagcuacuacugugacugccugcccggcuggaugggccagaacugcgacaucaacaucaacgacugccucgggcagugccagaacgacgccagcugcagggaucuggugaacggcuacaggugcaucugcccccccggauacgccggcgaccauugcgaaagggacaucgaugagugcgccuccaaucccugucugaacggcggccacugccagaacgagaucaacagguuccagugccugugccccaccggcuucagcgggaaccugugccagcuggacaucgacuauugcgagcccaaucccugccagaacggggcgcagugcuacaacagggccagcgacuacuucugcaagugccccgaggacuacgagggcaagaauugcagccaccugaaagaccacugccgcaccacccccugugagguuaucgacagcuguacggucgccauggccucgaacgacacccccgaaggcgugagguauaucuccagcaacgugugcgggccacacggcaaauguaagucccagagcggcgggaaguucaccugcgacugcaacaagggcuucacaggcacguacugccaugagaacaucaacgauugugagagcaaccccugcaggaacggcgggaccugcauagacggcgugaacagcuauaagugcaucugcagcgauggcugggagggagccuacugcgaaaccaacaucaaugacugcagccagaaccccugucacaacgggggcacaugccgggaccuggugaaugauuucuacugcgacugcaagaauggcuggaagggcaagaccugccacagcagggacucccagugugacgaggccaccugcaauaacgggggcaccugcuacgacgagggcgacgccuuuaagugcaugugccccggcgguugggaggguaccaccugcaacaucgcgcggaacagcagcugucugcccaaccccugccacaacgggggcacgugcguggugaacggcgagagcuucaccugcguguguaaggaggggugggagggccccaucugcgcccagaacaccaacgauugcucgccccaccccuguuacaacagcgggaccugcguggacggugauaacugguacaggugcgagugcgcaccaggcuucgccgggccggacugcaggaucaacaucaacgaaugucagagcuccccgugcgccuucggcgccacgugcguagacgagaucaauggcuacaggugcgugugccccccaggccacagcggggccaaaugccaggaagucagcggccgacccugcaucaccauggguuccguuaucccagacggagccaagugggaugacgauuguaacaccugucagugucugaauggccggaucgcgugcagcaagguguggugcggccccaggccgugccugcugcacaagggccacuccgaaugucccuccggucagagcugcauccccauccucgacgaccagugcuuuguacaccccugcaccggagucggcgagugcagguccucgucucugcagcccgugaaaaccaagugcaccagcgacuccuacuaccaggacaacugcgccaacaucacguucaccuuuaacaaggagaugaugagccccgggcugaccacggagcacaucugcucggagcugaggaaccugaacauacugaagaacgugagcgccgaguacagcaucuacauugccugcgagcccagccccagcgccaacaacgagauccacguggcgaucuccgccgaagacauccgggacgacggcaaccccaucaaggagauaaccgacaagaucaucgaccuggugagcaagcgggacggcaacagcucccugaucgccgccguggccgaggugcggguacagaggcggccccucaagaacaggacggacuuccucgugccgcuccugucguccgugcugaccguggccuggaucugcugucuggugaccgccuucuacuggugccugcggaagcggcgcaagccggggagccacacccacucggccagcgaagacaacacgaccaacaacgugagggagcagcugaaucagaucaagaaucccauagagaaacacggcgccaacaccgugcccaucaaggauuacgagaacaagaacagcaagauguccaaaaucagaacccacaauagcgaaguggaggaagacgacauggauaagcaccagcagaaggccagguucgccaagcagcccgccuacacccugguagacagggaggagaagccccccaacggcacccccacgaaacacccgaacuggaccaacaagcaggauaauagggaccuggaguccgcgcagagccugaaccgcauggaguacaucgug

SEQ ID NO: 88 - RNA, 3654 nt, Artificial Sequence
  Synthetic polynucleotide
augaggagccccaggacccggggccguagcgggaggccgcucucgcugcugcuggcccugcucugcgcccugagggccaagguguguggcgccuccgggcaguucgagcuggaaauccugagcaugcagaacgucaacggcgagcugcagaacggcaacugcugcggcggagcgcggaaccccggggacaggaagugcaccagggacgagugugacacguacuucaaagucugccucaaggaguaccagagccgggugaccgccgggggcccaugcuccuucggcagcggcagcacccccgucaucggaggcaacaccuuuaaucugaaggccagcagggggaacgacaggaauaggaucguccugcccuuuagcuucgccuggcccagguccuacacccugcuggucgaggccugggacagcuccaacgacaccguccagcccgacaguaucaucgagaaggcgucccacuccggcaugaucaaucccagcaggcaguggcagacgcugaagcagaacaccggcguggcccacuucgaguaucagauccgggugacgugcgacgacuacuacuacggguucggcugcaacaaguucuguaggccccgggacgauuucuucggccacuacgcaugcgaccagaacggcaacaagaccugcauggagggcuggaugggccccgagugcaacagggcuaucugccgccagggcugcucccccaagcacggcagcuguaagcugcccggcgauugccggugucaguacggguggcagggacuguauugcgacaagugcauaccccacccaggcugcgugcacggcaucuguaacgagcccuggcaaugccucugcgagaccaacugggggggacaacugugcgacaaggaccugaacuacugcgguacccaccagcccugccugaacggcggcaccugcaguaacaccggccccgacaaguaucagugcagcugccccgagggguauuccggcccgaacugcgagaucgccgagcacgccugccucagcgacccaugccacaauagaggcagcugcaaggaaaccucccugggguucgagugugagugcucccccggguggaccgggcccaccugcuccaccaacaucgacgacugcagccccaauaacugcagccacgggggcaccugucaggaccuggugaacggcuuuaagugcgucugccccccccaguggaccgguaagacgugccagcuggacgccaaugagugcgaagccaagcccugcgucaaugccaagagcuguaagaaccucaucgcguccuacuauugcgacugccugcccggguggaugggacagaacugcgacaucaacaucaacgacugccucgggcagugccagaacgacgccagcugccgggaccuggugaacggcuauagaugcaucugcccccccggcuacgccggggaccacugcgagagggacaucgacgagugcgccuccaaccccugccugaauggaggccacugccagaacgaaaucaacagguuccagugucugugccccaccggauucagcggaaaccugugccagcuggacaucgacuauugcgaacccaaccccugucagaacggcgcccagugcuacaaccgggcaagcgacuacuucugcaagugcccugaggacuacgagggcaagaacugcagccaccucaaggaccacugcaggacgacccccugugaggugaucgacagcuguaccguggccauggccucgaacgacaccccugagggcgugagguauaucuccagcaacgucugcggcccccacggcaaauguaagagccaauccgggggcaaguucaccugcgacugcaacaagggauuuaccggcaccuacugccacgagaacaucaacgacugcgaguccaaucccugccguaacggcggcaccugcaucgacggugucaacagcuacaagugcaucugcagcgacggcugggagggagcguacugcgaaaccaacauaaacgauuguucccagaaccccugccacaacggcggcaccugccgggaccuugugaacgacuuuuacugugacugcaagaauggguggaagggcaaaacgugccacagcagagacagccagugcgacgaagccaccuguaacaacggcggcaccugcuacgacgagggcgacgccuuuaaguguaugugcccgggcggcugggaaggcacgaccugcaacaucgcccggaacagcagcugccucccgaacccuugccacaacggcgggaccugcguggugaauggcgaauccuucaccugcgugugcaaggagggcugggagggccccaucugcgcccaaaacaccaaugacuguagcccccaccccugcuacaacuccggcacauguguggauggcgacaacugguacaggugugagugcgcccccggauucgccggccccgacugccggaucaacauuaacgagugucagagcagccccugcgccuucggcgccaccugcgucgaugagauaaacggauauaggugcgugugcccccccggacacagcggcgcgaagugccaggaggugagcggcaggcccugcaucacaaugggcagcgugaucccggacggcgccaagugggacgacgauugcaacaccugccagugccugaacggccggauagccugcuccaaaguguggugcggcccccgccccugccugcugcacaagggccacagcgagugccccuccggccagagcugcauccccauacuggacgaccaauguuucgugcaucccugcaccggcgugggcgagugucggagcagcagccugcagcccgugaagacuaagugcaccuccgacuccuacuaucaggacaacugugccaacaucaccuucaccuucaacaaggagaugaugagccccggccugacaacggagcacaucugcagcgagcugcgcaaucugaacauccugaaaaaugugagcgccgaguacagcaucuacaucgccugugagccgagccccagcgcuaauaacgagauccacguggccaucuccgccgaggacaucagggaugacggcaaccccaucaaagagaucaccgacaagaucaucgaccugguguccaagcgggacggcaacuccagccugaucgcagccguggccgaagugaggguccagcggcggccccugaagaaccgaaccgacuuccuggucccccugcugagcagcgugcugaccgucgcauggaucuguugccuggugacggccuucuacuggugccucaggaaaagacggaagcccgggagccacacccacagcgccagcgaggacaacaccaccaacaacgugcgggagcagcugaaccaaaucaagaaccccaucgagaagcauggcgccaauaccgugcccaucaaagacuacgagaacaagaacagcaagaugagcaagauccgcacccauaacucggagguggaagaagacgauauggauaagcaccagcaaaaggcccgguucgcgaagcagcccgccuauacccucguggaccgggaagaaaagccgcccaacggcacccccaccaagcaccccaacuggaccaacaaacaggacaacagggaccucgagagcgcccagucccucaaccguauggaguacaucguc

SEQ ID NO: 89 - RNA, 3654 nt, Artificial Sequence
  Synthetic polynucleotide
augagguccccgcguacccgaggcagguccgggaggccccugucccugcugcucgccuuacuuugcgcccugagggccaaagucugcggcgccuccggccaauucgagcuggagauccucagcaugcagaacgugaacggcgagcugcaaaacgggaacugcugcgggggagcccgcaaccccggcgaccggaagugcaccagggacgagugcgacaccuacuucaaggugugccucaaggaguaucagucaagggugaccgccggaggccccuguagcuucggcuccgggucgacccccgugauaggcggaaacaccuucaaccugaaggccagcagggggaacgacaggaauaggaucgugcuccccuucucguucgccuggcccaggagcuacacccuccucguggaggccugggacagcagcaacgauacggugcagcccgacuccaucaucgagaaggccagccacuccggcaugaucaaccccagccgccaguggcagacccugaagcaaaacacgggcguggcacacuucgaguaccagauaagggucacuugcgacgacuacuacuacggguucgggugcaacaaguuuugcaggccccgggacgacuucuucggacacuaugccugcgaccagaacggcaacaagaccuguauggaggguuggaugggccccgaaugcaaucgcgccauuugccggcaggggugcagcccuaagcacggaagcuguaagcuccccggcgacugccgcugccaguacggcuggcagggacuguacugugacaaguguaucccccaccccggcugcgugcacggcaucugcaaugagccuuggcagugccugugcgagaccaauuggggcggccagcugugcgacaaggaccugaacuacugcggcacccaccagcccugccugaacggugggaccugcagcaacaccgggccagacaaguaccagugcagcugccccgagggcuauagcgggcccaauugcgagaucgccgagcacgccugccuguccgaccccugucacaaccggggcuccugcaaggagaccucccugggguuugagugcgagugcucccccgguuggaccggccccaccugcuccaccaacaucgacgacugcucccccaacaauugcagccacggcggcacaugccaggaucuggugaacggcuucaagugugugugucccccccaguggaccggcaagaccugccagcuggacgcgaacgagugcgaagcaaagcccugcgugaacgccaaguccugcaaaaaccugaucgccagcuauuacugcgacugccugcccggcuggauggggcagaacugugacauaaacauaaacgacugccucggccagugccagaaugacgcgagcugccgggaccucgugaacggcuaccgaugcaucugccccccgggcuacgccggcgaccauugcgaacgggauaucgacgagugugccagcaaccccugccugaacggggggcacugccagaacgagauaaacagguuccagugccugugccccaccggcuucagcggcaaccugugccaacucgacaucgacuacugcgagcccaaccccugccaaaacggugcccaaugcuacaaccgggccucggacuacuuuugcaagugcccggaggacuaugagggcaagaauuguucccaccucaaggaccacugccggaccacccccugcgaggugaucgacuccugcaccguggccauggcuaguaacgauacccccgagggcguuagguacaucuccuccaacgugugcggcccccacgggaagugcaagucgcagagcggcggcaaguucaccugcgacugcaauaagggcuucaccgguaccuacugccacgagaacaucaacgacugcgagagcaaucccugccggaacggggguaccugcaucgacggcgugaacuccuacaaguguaucugcucagauggcugggaaggcgcguacugugagaccaacauaaacgacuguagccagaaccccugucauaacgggggcaccugcagggaccuggugaacgacuucuacugcgacugcaagaacggguggaaaggcaaaacuugccacuccagggacucccagugcgaugaggccaccugcaauaacggcggcacgugcuacgacgagggggacgccuucaagugcaugugccccgggggcugggaggggaccaccugcaacaucgccaggaacagcuccugccugcccaacccaugccacaauggaggcaccugcguagugaauggcgaguccuucaccugugugugcaaggagggcugggaggggcccaucugcgcccagaacaccaacgacugcagcccacacccgugcuacaacuccggcaccugcgucgacggcgacaacugguacaggugcgagugcgcccccggcuucgcgggcccggacugccggauuaauaucaacgagugccagagcagccccugcgccuucggggccaccugcgucgacgaaaucaacggguaccggugcgugugcccccccggccacagcggggcaaagugccaggaagucagcggcaggcccugcaucaccaugggcagcgucauucccgauggcgcaaagugggacgacgacugcaacacuugccagugccugaauggcaggaucgccugcagcaagguguggugcggcccaaggcccugccugcugcacaaaggccacagcgaaugcccaagcggucagagcugcauccccauccuggaugaccagugcuucgugcaccccugcaccggggucggugaguguaggagcagcagccugcagcccgugaagaccaagugcaccuccgauuccuacuaccaggacaauugcgccaacauaacuuuuaccuucaacaaggagaugaugagccccggccucaccacggagcacaucugcagcgagcugcgcaaccucaacauccugaagaacgugagcgccgaguacagcauuuacaucgccugcgagcccagccccuccgccaacaacgagauccacguggccaucagcgccgaggacauaagggaugacgggaaucccaucaaggagaucaccgacaagaucaucgaccugguguccaagcgggacggcaauagcagccugaucgccgccgucgcggaggugcgggugcagaggcgcccgcugaagaaccggaccgacuuccucgugccccugcugagcagcgugcugacgguggccuggaucugcugccuggugacagccuucuacuggugccugcggaagaggaggaagcccgggagccacacccauagcgcguccgaggacaacacgacaaacaacgucagagagcagcugaaccaaaucaagaaucccaucgaaaaacacggcgccaacaccgugcccaucaaagauuacgagaacaagaacagcaagaugagcaaaauccggacccacaacucggagguggaggaggacgacauggacaagcaccaacagaaggcccgcuuugccaagcagcccgccuacacccugguggaccgggaggaaaagccgccgaaugguacaccgaccaagcaucccaauuggacaaacaagcaggauaacagggaccuggaaagcgcccagagccugaaccggauggaguacaucgua

SEQ ID NO: 90 - RNA, 3654 nt, Artificial Sequence
  Synthetic polynucleotide
augaggagccccaggaccagggggaggagcgggaggccgcugagccugcuccuggcccugcugugugcccugcgcgccaaggugugcggcgcguccggacaguuugagcuggagauccuguccaugcagaacgugaacggcgagcuccagaacgggaacugcugcgggggcgcaaggaaccccggugacaggaagugcacccgcgacgagugcgacacguacuuuaaggugugccugaaagaguaccagagcagggugacugccggcggacccugcucguuuggaagcggcagcacuccugugaucgguggcaacaccuucaaucugaaggccuccagggggaacgauaggaacaggaucgugcugccauucagcuuugccuggccccggucauacacccugcugguggaggccugggacuccagcaacgacaccgugcagcccgacuccaucauagagaaggcgagccacagcggcaugaucaaccccuccaggcaguggcagacccucaagcagaacaccggcgucgcccacuucgaauaccagaucagggucacgugcgacgacuacuacuacggcuuuggcugcaauaaguucugcaggccccgggacgacuucuucgggcacuacgccugcgaccagaacgggaacaaaaccuguauggagggguggaugggccccgaaugcaaccgagccaucugccgccaggggugcucccccaagcacggcuccuguaaacuccccggcgauugcaggugucaguacggcuggcagggucucuacugcgacaagugcaucccgcaccccggcugcguccacggcaucuguaaugagcccuggcaaugccugugcgagaccaacuggggcggccagcugugcgacaaggaccucaauuauuguggcacccaccagccaugccugaaugguggcaccugcagcaacacaggcccagacaaguaccagugcagcugucccgagggcuacucgggccccaacugcgaaaucgccgagcacgcuugccugagcgaccccugucacaacaggggcagcugcaaggaaaccagccugggguucgagugcgagugcagccccggguggaccggccccaccugcagcaccaacaucgacgacugcagccccaacaacuguagccauggcggcaccugccaggaucuggucaacggcuucaagugcgugugucccccccaguggaccggcaagaccugccagcucgacgccaacgagugugaagcaaagcccugcgugaaugccaaguccugcaagaaccugauagccuccuacuacugcgacugccugcccggcuggaugggccagaacugugacaucaacaucaacgacugccuggggcagugucagaaugacgccagcugccgcgaccuggugaauggcuauaggugcaucugcccccccggauacgccggcgaccacugcgagagggauaucgaugagugcgccagcaacccuugccugaacggcgggcacugccagaacgagauuaacagguuccagugccugugccccaccggcuucagcggcaaucugugccagcuggauaucgacuacugcgagcccaacccgugccagaacggcgcccagugcuacaacagggccuccgacuacuucuguaagugucccgaggacuaugagggcaagaacuguucccaccugaaagaccacugcaggaccacccccugcgaggugaucgacucgugcaccguggccauggcgagcaaugacaccccggaaggcgugcgcuauaucagcagcaaugugugcgggccccacggcaagugcaagagccagagcggcgggaaguucaccugcgacugcaacaagggcuucaccggcacguacugccacgagaacaucaacgauugcgaguccaaccccugccggaacggcggcaccugcauagauggagugaacuccuauaagugcaucugcuccgaugggugggagggcgccuacugugaaaccaacaucaacgacugcagccagaaccccugccauaaugguggcacgugccgggaccugguuaaugacuucuacugcgacugcaagaacggcuggaagggcaagaccugccacagcagagauagccagugcgacgaggccacgugcaacaauggcgggaccugcuacgacgagggggacgccuucaaaugcaugugccccggcggaugggaggggaccaccugcaacaucgccaggaacuccagcugccugcccaacccgugccauaacgguggcaccugcguggugaacggcgaaagcuucaccugcgugugcaaggagggcugggagggccccaucugcgcccagaacaccaaugacugcuccccccacccaugcuacaacuccgggaccuguguggacggcgacaacugguauaggugcgagugugcccccggcuucgccggccccgacugcaggaucaacaucaacgaaugucagagcucccccugcgccuuuggcgccacaugugucgaugagauuaacggcuaccggugcgucugcccccccggccacagcggcgcgaagugccaggaagucuccggcaggcccuguaucaccaugggcagcgugauccccgacggcgccaagugggacgacgacugcaacaccugucaaugccugaauggcaggaucgccugcagcaaagucuggugcgggccccggcccugccugcugcacaagggccacagcgagugcccuuccggccagagcugcaucccgauccuggacgaucaguguuuuguccauccaugcaccggcgugggcgaguguaggucgagcagccugcagcccgugaaaacaaagugcaccagcgacagcuacuaccaggauaacugugccaacaucaccuuuaccuucaacaaggagaugaugagccccggacugaccaccgagcauaucuguucagagcugaggaaccugaacauccucaagaacgucagcgccgaguacagcaucuacaucgccugcgagcccagccccuccgccaacaacgaaauccacguggccauaagcgccgaggacaucagggacgacggcaauccgaucaaggagauaaccgacaagaucaucgaccucgugaguaagagggacgggaacaguagccucaucgccgccgucgccgaggugagggugcagcggaggccccugaagaacaggaccgauuuucuggucccccugcugagcuccgugcugaccguggccuggaucugcugccuggugacggcguucuacuggugccuccggaaacgacggaagcccgggagccauacccacuccgccagcgaggacaacaccaccaauaacgugagggagcagcugaaucagaucaagaauccgaucgagaagcacggcgccaacaccgugccgaucaaagacuacgagaacaagaauuccaagaugagcaagaucaggacccacaacuccgagguggaggaagaugacauggacaagcaccagcagaaagccagguuugccaagcagcccgccuauacccugguggacagggaggagaaacccccgaauggcacccccaccaaacacccaaacuggaccaacaagcaggacaacagggaucuggagagcgcccagagccucaaccguauggaguacaucgug

SEQ ID NO: 91 - RNA, 3654 nt, Artificial Sequence
  Synthetic polynucleotide
augaggucaccccggacccggggacgcuccggcaggccccugagccugcugcuggcccugcugugcgcccucagggccaaggucugcggcgccuccggucaguucgaacucgagauccugagcaugcagaacgugaacggugaacugcagaacggcaacugcugcggcggcgccaggaaucccggcgaccgaaagugcaccagggacgagugcgacaccuacuuuaaggugugccuaaaggaguaccagagccgggugacggccggcggccccuguuccuucggcagcggcagcacgcccgugaucggcggcaacaccuucaaccucaaggccucgcgcggcaacgaucggaacaggaucgugcugccguuuuccuuugccuggcccaggucguacacccugcugguggaggccugggacagcuccaaugacaccgugcagccagacuccauaaucgagaaggccagccacagcgggaugauuaauccaagcaggcaguggcaaacccugaagcagaacaccggaguggcccauuucgaguaccagaucagggugaccugcgacgacuacuacuacggcuucggaugcaacaaguucugcaggccccgggacgacuucuucggccauuacgccugcgaccagaacggcaacaagaccugcauggaggguuggaugggccccgaaugcaauagggccaucugcaggcaaggcuguucccccaaacacgggagcuguaaacuccccggcgacugccgaugccaguacggguggcaaggccucuacugcgacaagugcaucccccaucccggcugcgugcauggcauuugcaacgaacccuggcaaugccucugcgagaccaacugggggggccagcucugcgacaaggaucugaacuacugcggcacacaccagccuugccugaacggagggaccugcaguaauaccggccccgacaaguaccagugcagcugccccgagggcuauagcggccccaacugcgaaauugccgagcacgccugccugagcgaccccugucacaacaggggcagcugcaaggagaccagucugggcuucgagugcgagugcagcccaggcuggacgggccccaccugcuccaccaacaucgacgacugcucccccaacaauugcagccacggcggcaccugccaagaucucgugaacggcuucaagugcguguguccgccgcaguggaccgggaaaaccugccaacuggacgccaacgagugugaggcaaagcccugcgugaacgcgaaguccuguaagaaccugaucgccagcuacuauugcgacugccugccgggcuggauggggcagaacugugacaucaacaucaacgauugccugggccagugucagaacgacgccagcugcagggaccuggucaacggcuacaggugcaucugucccccgggguaugccggggaccacugcgaacgagauaucgacgagugcgccucgaacccuugccucaauggcggccacugccagaacgagaucaacagguuccagugccugugccccaccggcuucagcggcaaucugugccagcuggacaucgacuauugugaacccaacccgugccagaacggcgcccagugcuacaaccgcgccuccgacuacuucugcaagugcccggaggacuacgagggcaagaacugcagccaucugaaggaccacuguagaaccacgcccugcgaggugaucgacuccugcaccgucgccauggccucaaacgacacccccgagggagugcgcuacaucagcucgaacgugugcggcccccauggaaaaugcaagagccaguccgggggcaaguucaccugcgacugcaacaagggcuucaccggcacguauugccaugagaacaucaaugacugcgagagcaacccgugccguaacgggggcaccuguaucgauggcgugaacagcuacaagugcaucuguagcgacggcugggagggcgccuauugcgaaaccaacaucaacgacuguucccagaacccaugccacaacgggggcaccuguagggaccuggucaacgacuuuuacugugacugcaagaacgguuggaaaggcaagaccugccacucgagggacagccagugugacgaggccacgugcaacaauggcggcaccuguuacgacgagggcgacgccuuuaagugcaugugucccggggguugggaggguaccaccuguaacaucgccaggaacucaagcugccugcccaaucccugccauaacggugggaccugcguggugaacggcgaaagcuucaccugcgugugcaaggagggcugggagggccccaucugugcccagaacaccaaugacugcagcccccaccccuguuacaacagcgggaccugcguggauggugacaacugguacaggugugagugcgcccccggguuugccggccccgacugcaggaucaacaucaacgagugccagagcagccccugugccuucggcgccaccugcguggacgagaucaacggguaccggugcgugugcccccccggccacuccggcgccaagugccaggagguguccggcaggcccugcaucaccaugggcagcgucauccccgacggcgccaaaugggacgacgacugcaacaccugucagugccugaacggcaggaucgccugcuccaagguuuggugcgggcccaggcccugccugcugcacaagggacauagcgaaugccccagcggccagagcugcauccccauccuggacgaccagugcuucgugcaucccugcaccggggugggcgagugccggagcuccucgcugcaacccgucaagaccaagugcaccucggacagcuauuaccaggacaacugcgccaacaucaccuucaccuucaacaaggaaaugaugagccccggccugaccaccgagcauaucugcagcgagcugcggaaccugaacauacugaagaacguuagcgccgaguacuccaucuacaucgccugcgagcccagcccgagcgcgaauaaugagauccacgucgccaucagcgccgaggacauccgggacgacggcaaccccaucaaggagaucaccgacaagaucaucgaccuggucagcaagcgugacggcaacuccagccugaucgccgcgguggcugaggugcgaguccagaggaggccccugaagaacaggacggacuuccucgucccucugcugagcagcgugcugaccguggccuggaucuguugccuggugaccgccuuuuacuggugccugcgaaagaggaggaagccgggcagccacacccacagcgccucagaagacaacaccacaaacaacguccgcgagcagcucaaccagaucaaaaaccccaucgaaaagcacggcgccaacaccgugcccaucaaggacuacgagaacaagaauagcaagaugagcaagauccgcacucacaacagcgagguggaggaggacgacauggacaagcaccagcagaaggccagguuugccaagcagcccgccuacacccugguggaccgggaggagaagccgcccaauggcacccccacgaagcacccgaacuggaccaacaaacaggacaacagggaccuggagagcgcccagagccugaaccgcauggaguacaucgug

SEQ ID NO: 92 - RNA, 3654 nt, Artificial Sequence
  Synthetic polynucleotide
augcggucccccaggaccagggggcgcagcgggaggccccugagccugcugcuggccuuacugugugcccugagggccaaggugugcggcgccagcgggcaguucgagcuggagauacuguccaugcaaaacgugaacggcgaacugcagaaugggaauugcugcgguggcgccaggaacccuggggaccgcaaguguacccgggacgagugcgacaccuacuucaaggugugucucaaggaauaucagucccgcgugaccgccgggggccccugcagcuucggcucaggcagcaccccagucaucgggggcaacaccuucaaccugaaggccagccguggcaacgacaggaacaggauagugcugcccuucuccuucgcguggcccagguccuacacccugcugguggaggcgugggauagcucgaaugauaccguccagcccgacuccaucaucgagaaagccucccacuccgguaugaucaauccaagcaggcaguggcagacccugaagcagaacacgggcguggcccacuuugaguaccagaucagggucaccugcgacgacuacuacuacggcuucggcuguaauaaauuuugccggccucgggacgacuucuucggccacuacgccugcgaccagaacggcaauaagacguguauggagggcuggaugggcccggaguguaauagggccaucugccgacaggggugcagccccaagcacggcagcugcaagcugcccggcgacugcaggugucaguacggcuggcaaggacuguauugugacaagugcauuccccauccgggcugugugcacggaaucugcaaugagcccuggcagugccugugcgagaccaacuggggcggccagcugugugacaaggaucugaacuacuguggcacccaccagcccugccugaacggcgggaccugcuccaauaccgggcccgacaaguaccaguguuccugccccgagggcuacagcgguccaaacugcgagaucgccgagcacgccugccugagcgaccccugccauaacaggggcuccugcaaggagaccagccugggcuucgaaugcgagugcucccccggguggaccggccccaccugcaguaccaacaucgaugacugcagccccaauaacuguucccacggcggcaccugccaggaccuggugaacggcuucaaaugcgucuguccgccccaguggaccggaaagaccugucagcucgacgcaaacgagugcgaggccaagcccugcgugaacgccaagagcugcaagaaucugaucgccuccuacuacugcgauugucugcccggauggaugggccaaaacugcgacaucaacaucaacgauugucuggggcagugccagaacgacgccagcugcagggaccuggucaacggcuacaggugcaucugcccccccggcuaugccggagaccauugcgagcgagacaucgacgagugugccucgaaccccugccugaacggggggcacugccagaacgaaaucaacagguuccaaugccucugccccaccggguucagcggcaaccugugccagcuggacaucgacuauugcgagcccaaccccugccagaacggggcgcaguguuauaaccgggccucggacuacuucuguaagugucccgaggacuacgagggcaaaaacugcucccaccugaaggaccacugccguaccacacccugcgaagucaucgacuccugcaccguggccauggccagcaacgacacccccgagggagugcgguacaucagcagcaacgugugcgggccgcauggcaaguguaagucccagagcgggggcaaguuuacaugugacuguaacaagggcuucaccggcacauacugccacgagaacaucaacgauugcgagagcaaccccugccggaaugggggcaccugcaucgacggggugaacagcuauaaguguaucugcuccgauggcugggagggcgccuacugcgagacuaacaucaaugacugcucgcagaacccgugccacaacgggggaaccugcagggaucucgugaacgacuucuacugcgacugcaagaacggguggaaggggaagaccugccacagccgcgacucccagugcgacgaggccaccugcaacaaugggggcaccugcuacgacgagggcgacgccuucaagugcaugugccccggcgggugggagggcaccaccugcaacaucgcccggaacuccagcugccugcccaauccgugucacaaugggggcaccugcguggugaacggcgagucguucacgugcgugugcaaggaaggcugggagggaccgaucugcgcccaaaauaccaacgacuguagcccccaccccuguuauaacagcggcaccugcgucgacggggacaauugguaccggugcgagugcgcccccggcuucgccggccccgacugccgaaucaacaucaacgaaugucaaagcucacccugugccuucggggcaaccuguguggacgagaucaacggcuaccggugugugugccccccgggacacuccggggccaagugccaggaggugagcgggcgaccaugcaucaccaugggcuccgugauccccgacggcgccaagugggacgacgacugcaacaccugccagugccugaacggcaggaucgccugcuccaaggugugguguggcccccggcccugucuccugcacaaaggucacagcgagugccccagcggccagagcugcaucccgauccuugacgaccagugcuucgugcacccguguacaggcguaggggagugcaggagcuccucgcuccagcccgugaaaaccaaguguaccagcgacucauacuaucaggacaacugugccaauaucaccuuuaccuucaacaaggaaaugaugagccccgggcugaccaccgagcacaucugcagcgagcugcggaaccuuaacauucugaaaaauguguccgccgaguacagcauauacaucgccugcgagccgagcccuagcgccaacaaugagauacacguggccaucagcgcugaggacaucagggaugacggcaacccgaucaaggagaucaccgacaagauaauagaccucgucagcaaaagggacggcaacagcagccugaucgccgccgucgccgaggugagggugcagcgccggccccugaagaacaggaccgacuuccuggugccccuccugagcuccgugcugaccguggccuggaucugcugccuggugaccgccuucuacuggugucugaggaaaaggaggaagccuggcagccacacccauagcgccuccgaggacaauaccaccaacaacgucagggaacagcucaaccaaaucaagaaccccaucgagaagcacggcgccaauaccgugcccaucaaggauuacgagaacaagaauagcaagauguccaagauccgcacacauaauuccgaggucgaggaagacgacauggauaagcaccagcagaaggccagauucgccaagcagcccgccuacacccugguggacagggaggagaagccccccaacggcacacccaccaagcaucccaacuggaccaacaagcaggacaacagggaccuggagagcgcccagucccugaaccguauggaguacaucguc

SEQ ID NO: 93 - RNA, 3654 nt, Artificial Sequence
  Synthetic polynucleotide
augaggagccccaggacaaggggccggagcggcaggccccugagccugcugcucgcccuccucugugcccugcgcgccaaagugugcggggccucaggccaguucgagcucgagauccuguccaugcaaaacgugaacggcgaacugcagaacggaaauugcugcgguggcgcccguaaccccggcgaccgcaagugcaccagggacgagugcgacaccuacuucaaggugugucugaaggaguaccagagcagggucaccgccggcggccccugcagcuuuggcuccggcagcacccccgugaucggcggcaacaccuucaaccugaaggcuagccgcggcaacgacaggaacaggaucgugcuuccauuuagcuucgccuggcccaggagcuacacccugcuuguggaggccugggacagcuccaacgacaccgugcagcccgacagcaucaucgagaaggccagccacuccggcaugaucaaccccagccggcaguggcagacccugaagcagaacaccggcgucgcgcacuucgaguaccagaucagggugacaugugacgacuauuacuauggcuuuggauguaacaaguucugcaggcccagagacgacuucuucggccacuacgccugcgaccagaacggaaauaagaccuguauggaaggcuggauggggcccgagugcaaccgagccaucugcaggcaaggcugcagccccaagcacggcagcugcaagcugcccggggacugccggugccaguacggcuggcagggcuuguauugcgacaagugcaucccgcaccccggcugcgugcacgggaucugcaacgagcccuggcagugccugugcgagacgaacuggggcggccagcugugcgacaaggaccugaacuacugcgggacgcaucaacccugucucaacggcgguaccugcagcaauaccggccccgacaaguaccagugcucuugccccgagggcuauagcgggcccaacugugagaucgccgagcacgcuugccuguccgaccccugccacaaccggggcuccugcaaggagaccucccugggcuucgagugcgaaugcagccccggguggaccggucccacgugcagcaccaacaucgaugacuguagccccaacaacugcagccacggcggcacgugccaggaccucgugaacggcuucaagugcgugugccccccccaguggaccggcaagaccugccagcucgacgccaaugagugcgaagccaagcccugcgucaacgccaaguccugcaagaaccugaucgccaguuacuacugcgacugucugcccggauggaugggccagaauugcgacaucaacaucaaugacugccugggccagugccagaaugacgcguccuguagggaucuggugaacggguacaggugcauauguccccccggcuaugccggggaucacugcgagagggauaucgaugagugcgccagcaaccccugucugaacgguggccacugccagaacgagauuaacagguuccagugccugugccccaccggcuucagcggcaaccugugccagcuggauaucgacuacugugagcccaacccgugccagaacggcgcccagugcuacaaccgagccagcgauuauuuuugcaaaugucccgaggauuacgaagggaagaauugcagccaccugaaggaccauugcaggaccacccccugcgaagugaucgacagcugcaccguggccauggccucgaaugacacgcccgagggagugagguacaucaguagcaaugugugcggcccccaugggaagugcaagagccagucgggcggaaaguuuaccugcgacuguaacaagggcuucaccgggaccuacugucacgaaaacaucaacgacugcgaguccaacccguguaggaacggcgggaccugcauagacggggugaauagcuauaagugcaucuguucagacggaugggagggggccuacugcgagaccaacaucaacgauugcucgcagaaccccugccacaacggcggcaccugccgggaccuggugaacgacuucuacugcgacuguaaaaacggcuggaaggggaagaccugccacuccagggacagccagugcgacgaggcgaccugcaacaacggcggcaccugcuacgacgagggcgaugccuucaaguguaugugccccggaggcugggagggcaccaccugcaacaucgcccgcaacagcagcugccugcccaaucccugccacaaugguggaacaugcguggugaacggggagagcuuuacgugcgugugcaaggagggaugggagggccccaucugugcccagaacaccaacgacugcuccccccaucccuguuacaacagcggcaccuguguggacggggacaacugguaccgcugcgagugcgcccccggcuucgccggcccggacugccguaucaacaucaacgagugucagagcagccccugcgcauucggcgccaccugcguggaugaaauaaacggcuacaggugugugugcccccccggccacagcggagccaaaugccaggaggugagcgggcgcccaugcaucaccauggggagcgugaucccagacggggcgaagugggaugacgacuguaacaccugccagugccugaacggccgaaucgccugcagcaagguguggugcgggccccggcccugccugcugcacaaaggccacagcgagugccccagcggccagagcugcauaccgauccuggacgaccagugcuucguacaccccugcaccggggugggcgagugccgguccuccucgcuccagcccgucaagaccaagugcaccagcgauagcuacuaccaggacaacugcgccaacaucaccuuuaccuuuaacaaggagaugaugagccccggccugaccacggagcacaucugcagcgagcugcgcaaccucaacauccugaaaaacgugucggccgaguacuccaucuacaucgccugcgagcccucccccuccgccaacaaugaaauccacguggccaucagcgccgaggacauccgagacgaugggaaccccaucaaggaaaucaccgacaagauaaucgaccuggugaguaaaagggacgggaacagcagccugaucgcugccguggcggaggugaggguccagaggaggccgcugaaaaaucggaccgacuuucuggugccccugcugagcuccgugcugaccgucgccuggaucugcugccuggucaccgccuucuacuggugccugaggaagcguaggaagcccggcagccacacgcacagcgccagcgaggacaacaccaccaacaacgugcgggagcagcugaaccagaucaagaaccccaucgagaagcacggcgcgaacacagugccgaucaaggauuacgagaacaagaauuccaagaugagcaagaucaggacccacaacagcgagguggaggaggacgacauggauaaacaccagcagaaggccagguucgccaagcagcccgccuauacccuggucgacagggaggagaaacccccuaauggcacccccaccaagcaccccaacuggacaaacaagcaggacaacagggaccuggagagcgcccagagccugaaccguauggaguauaucgug

SEQ ID NO: 94 - RNA, 3654 nt, Artificial Sequence
  Synthetic polynucleotide
augcggagccccagaacccguggccggagcggcaggccccugucacuacugcuggcccugcugugcgcgcuuagggccaaggucugcggcgccagcggccaguucgagcuggagauccugagcaugcagaacgugaacggcgagcugcagaacggcaacugcugcggcggggccaggaaccccggagaccgcaaaugcacccgggacgagugcgacaccuauuuuaaagugugccugaaggaguaccagagcagggugaccgccggcggccccugcagcuucggcagcggcagcacccccgugaucggcgggaauaccuucaaccugaaggccagccgcggcaacgacaggaaccgaaucgugcugcccuuuagcuucgccuggccucggagcuacacccugcugguggaagccugggacuccuccaacgacaccgugcaacccgacuccauuaucgagaaggccucccacagcggcaugauaaaccccagccggcaguggcagacacugaagcaaaacaccggggucgcacauuucgaguaccagaucagggugacgugugacgacuacuacuacggguucggaugcaacaaguucugcaggcccagggacgacuucuucggccacuacgccugugaccagaacggcaauaagaccugcauggagggguggaugggcccggagugcaacagggccauaugccggcagggcugcuccccaaaacacggguccugcaagcugccuggcgacugcaggugucaguacggcuggcaggggcuguacugcgauaagugcaucccccaccccggcugcguccacggcaucugcaacgagccauggcagugucugugcgagaccaacuggggugggcagcugugcgacaaggaucugaacuacugcggcacccaccagcccugccucaacgggggaacgugcucgaacaccgggcccgauaaguaccagugcuccugccccgaaggcuacucgggaccuaacugugagaucgcugagcacgcaugccugagcgacccaugccauaacagggguaguugcaaggagaccucccucgguuuugaaugcgagugcagccccggcuggaccggccccaccugcucgaccaacaucgacgacugcagcccaaacaacugcucccacggcggcacgugucaggaccuggugaauggcuucaagugugugugccccccccaguggaccggaaaaaccugccagcuggaugccaacgagugugaggccaagcccugcgugaacgcgaaguccugcaagaaccugaucgccuccuacuacugugacugccugcccgguuggaugggccaaaacugcgacaucaacaucaacgacugccugggccagugccagaacgacgccagcugcagggaccuagugaacggguaucggugcaucugcccccccggcuacgccggcgaucacugcgaaagggacaucgacgagugcgccagcaacccgugccugaacggggggcacugccagaacgagaucaacagguuccagugccucugccccaccggguucagcgggaaccucugccagcucgacaucgacuacugcgagcccaaucccugccagaacggcgcgcaaugcuacaauagggccucggacuacuucugcaagugccccgaggacuacgagggcaaaaacugcagccaccugaaggaccacuguaggacaacccccugcgaagucaucgacuccugcaccguggccauggccuccaacgacaccccagaaggcguacguuacaucagcuccaacgucugcgggccccacgggaagugcaagagccagagcggcggcaaguucacgugugacugcaacaaaggguucaccggcaccuacugccaugagaacauaaaugacugcgaguccaaccccugucggaacggcggcaccugcaucgacggcguaaacucuuacaaauguaucugcagcgacggcugggagggcgccuacugcgagaccaacaucaacgacugcagccaaaaccccugucacaacggcgggaccugccgcgaccucgucaacgacuucuacugcgacugcaagaacggcuggaagggcaagaccugccacagccgggacucgcagugugaugaggccaccugcaacaauggcggcaccugcuaugaugagggggacgccuucaaauguaugugccccggcgggugggagggcaccacuugcaacaucgccaggaacuccuccugccuccccaaccccugccacaacggagggacgugcguggugaacggggagagcuucaccugcgugugcaaggagggcugggaaggccccauuugcgcgcagaacacuaacgauugcagcccccaccccugcuacaacuccggcaccugcguggacggggacaacugguaccggugcgagugcgcccccggcuucgccggcccggacugcaggaucaacaucaacgaaugucagagcagccccugcgccuucggagccaccugcguggacgagauaaacggcuaccggugcgucugcccccccggucacucuggugccaagugccaagaggucagcggcaggccgugcaucaccaugggcuccgugaucccggauggcgccaaaugggacgaugacugcaacaccugccagugccuuaacggucggaucgcgugcagcaaggugugguguggccccaggcccugccuccugcacaaggggcacagcgagugccccuccggacaguccuguauccccauccuggacgaccagugcuucguccaccccugcaccggagugggcgaaugcaggagcagcucccugcagccggugaagaccaagugcaccagcgacuccuacuaccaggacaauugcgccaacaucaccuucaccuucaacaaggagaugaugagccccggccugaccaccgagcacaucugcagcgagcugcgcaaccugaacaucuugaagaacgugagcgccgaguauuccaucuacaucgccugcgagcccagcccgagcgccaauaacgagauccacguggccaucagcgccgaggacauccgggaugacggcaaucccaucaaggagaucaccgauaagaucaucgaccuggucagcaagcgcgacggcaauagcucgcugaucgcggccguggccgaggugagggugcagcggcggccccugaagaacaggaccgacuuucugguaccccuccugagcucggugcugaccguugccuggaucuguugucuggugaccgccuucuacuggugccugcggaaaaggcggaagcccggcucccauacccauagcgcauccgaagacaacaccaccaacaacguccgugagcagcugaaccagaucaagaaccccauagagaaacacggcgccaacaccgugcccaucaaggacuacgaaaacaagaacuccaagauguccaaaaucaggacccacaacagcgagguggaagaggacgacauggauaaacaccagcagaaggcccguuucgccaagcagcccgccuacaccuuaguggacagggaggagaaaccccccaacgggacccccaccaagcacccaaacuggacgaacaagcaggauaaccgggaccuggaaucagcgcagucccugaacagaauggaauacaucguc

SEQ ID NO: 95 - RNA, 3654 nt, Artificial Sequence
  Synthetic polynucleotide
augagguccccccgaaccaggggcagguccggucggccccugagccugcuccuggcccuccugugcgcccugagagccaagguguguggagccagcgggcaguucgagcucgagauccucuccaugcagaacgugaacggcgagcugcagaacggcaacugcugcggaggcgccaggaaucccggcgaucggaagugcaccagggacgagugcgacaccuauuucaaggugugccucaaggaguaccaaagcagggugaccgccggcggccccugcuccuucggcagcggcagcacccccgugauagggggcaacacguucaaccucaaggccagcaggggcaacgacaggaaccgcaucgugcugcccuucagcuuugcguggccccguuccuacacccugcuggucgaggccugggacagcuccaacgauaccgugcagcccgacuccaucauugagaaggccagccacagcggcaugaucaaccccagcaggcaguggcaaacccugaagcagaacaccggaguggcccauuucgaauaccagaucagggugaccugcgaugacuacuauuaugguuuugggugcaacaaauucugccggccccgagacgacuucuucggucacuaugccugcgaccagaacggcaacaagaccuguauggagggguggaugggcccugagugcaaccgggccaucugucgccaggggugcucccccaagcacggcagcugcaagcugccuggcgauugccggugucaguacggguggcagggucucuacugcgacaagugcaucccccacccgggcugugugcacggcaucugcaacgagcccuggcagugccugugcgaaaccaauuggggcggccaacugugcgacaaggaccugaacuacuguggcacccaccagcccugccugaacgggggcacuugcuccaacacgggccccgacaaguaucagugcagcuguccugagggcuacagcggccccaacugugagaucgccgagcaugccugccugagcgacccgugccacaaucguggcagcuguaaggagaccagccugggcuucgagugcgagugcagcccggguuggaccggacccaccugcagcaccaacaucgacgauugcagccccaacaacuguucacacgggggcacgugccaagaccuggugaacggguucaagugugucugccccccccaguggaccggcaaaaccugucagcucgacgccaacgaaugugaggccaagcccugcgugaaugcgaagagcugcaagaaccugaucgcgucguacuauugcgauugccugcccggcuggaugggccagaacugcgacaucaacaucaacgacugccugggccagugccaaaacgacgccucuugccgcgaucuggucaacggguaccgcugcaucugcccuccgggguacgccggggaucacugugagagggacauagaugagugcgcguccaaccccugccugaacggggggcacugccagaacgagaucaacagguuucagugccugugccccaccggcuucuccggcaaccugugccagcuugacaucgacuacugcgagcccaaucccugccagaauggcgcccagugcuacaacagggccagcgacuauuucugcaagugucccgaggacuacgaggggaagaauugcucccaccugaaagaccacugcaggacgacccccugugaggugaucgacagcugcaccguggccauggccuccaacgacacccccgagggcgugagguacaucagcagcaacgucugcggcccccacggcaagugcaagagccagagcggcggaaaguucaccugcgacugcaacaagggguucacgggcaccuacugccacgagaacaucaacgacugcgaguccaaccccugcaggaacggcggcacgugcauagacgggguuaacagcuauaaguguaucugcucggacgggugggaaggcgccuacugcgagaccaacaucaacgacugcucacagaauccgugccacaacgggggcaccugcagggaccuggugaacgacuucuauugcgacugcaagaacggcuggaaagguaagacaugccacucccgggacucccagugcgacgaggccaccugcaacaacggaggaaccugcuacgaugagggcgacgccuucaagugcaugugccccgggggaugggaaggcaccaccugcaacaucgccaggaacuccagcugucuccccaacccgugccacaacggcgggacgugcguggugaauggcgaguccuucacgugcgugugcaaggagggcugggagggccccaucugcgcgcagaacaccaacgauugcagcccccacccgugcuacaacucaggcaccugcgucgacggugacaacugguaccggugcgagugcgccccaggguucgcgggccccgacugcaggaucaacaucaacgagugccaguccagccccugcgccuuuggcgccaccugcguggacgagaucaacggcuacaggugcgugugcccccccggccauagcggcgccaagugccaggaggugagcggcaggcccugcaucaccaugggcagcgugauccccgacggcgccaagugggacgacgacugcaauacgugccagugccugaacggacgcauugccugcuccaagguguggugcggcccccggccgugccugcuccacaaggggcacagcgagugccccuccggccagagcugcauccccauccucgacgaccagugcuucguccaccccugcaccggcgugggcgagugcagguccuccagccugcagccagugaaaaccaaguguaccagcgacuccuacuaccaggacaacugcgccaacaucacauucacauucaacaaggagaugaugagcccgggccugaccaccgagcacaucugcagcgaacucagaaaccugaacauccugaagaacgugucggccgaguacagcaucuauaucgcgugcgagcccagccccagcgcgaauaacgagauccacguggccauaagcgcggaggacauccgggacgacggcaaccccaucaaggagaucaccgacaagauuauugaccuggucuccaagagggacggcaauagcucccugauugccgccgucgccgaagugcgggugcaaagaaggccccugaaaaaccggacggauuuccuggucccccuccugagcagcgugcugaccgucgccuggaucugcugucuggugacggccuucuacuggugccucagaaagaggcgcaaacccggcucgcacacccauagcgccucagaggacaacaccacgaauaacgugcgggaacagcugaaccaaauaaaaaaccccaucgagaagcacggggcuaacaccgugccgaucaaggacuacgagaacaagaacagcaagauguccaagauccgaacccacaacagcgaggucgaggaggacgacauggacaagcaccagcagaaggcgagguucgccaagcagcccgccuacacccugguagaccgggaggagaagccgcccaacggcacccccacgaaacaccccaacuggaccaacaaacaagacaacagggaccuggagagcgcccagucccugaacaggauggaauauauuguc

SEQ ID NO: 96 - RNA, 3654 nt, Artificial Sequence
  Synthetic polynucleotide
augaggagccccaggacacggggccggagcgggcgaccucugucccugcuccuggcccugcugugcgcccugagagccaaagugugcggcgccagcgggcaguucgagcuggagauacugagcaugcagaacgugaacggcgagcugcagaacggcaacuguugugggggcgcgcggaaccccggggacaggaagugcacccgggacgagugcgacaccuacuucaaggugugccucaaggaauaccaaagccgugugacagcugggggccccugcagcuucggguccggauccacccccgucaucggcggcaacaccuucaaccucaaggccagcaggggcaacgacaggaaccgaaucgugcugcccuuuucguuugccuggccccgcagcuacacccuccuaguggaggccugggacagcagcaacgacaccgugcagcccgacuccaucaucgagaaggcaucccacagcgggaugaucaaucccucccgccaguggcagacgcugaagcagaacaccggcguggcccacuucgaauaccaaaucagggugacgugcgaugacuacuauuacggcuucgggugcaacaaguucugcaggccgagggaugacuucuucggccacuaugccugcgaccagaacggaaacaaaaccugcauggaggguuggaugggacccgagugcaacagggccaucugccgccagggcugcucaccaaagcacggcagcuguaagcuacccggcgacugucggugccaguacgguuggcagggccuguacugugacaagugcaucccccaccccggcugcgugcacggcaucugcaaugagccguggcagugccugugugaaaccaacuggggugggcagcugugcgacaaggaccugaauuacugcggcacccaccagcccugucugaacggcggcaccugcuccaacaccggcccggacaaguaucagugcaguugccccgagggcuauagcggccccaacugcgagaucgccgagcacgccugccuguccgacccgugccacaacagggggagcugcaaagagaccagccugggguucgagugcgagugcagccccggguggaccggacccaccugcagcaccaacaucgaugauugcagcccuaacaacugcucccacggcggcaccugccaggaccuggugaacggcuuuaagugcguaugccccccccaauggacggggaagaccugucagcucgacgccaaugaaugcgaggcaaaaccgugugugaacgccaagagcugcaaaaaccucaucgcguccuacuacugcgacugccugcccggcuggauggggcagaacugugacaucaacaucaacgauugccugggccaaugccagaaugaugccuccugcagggaccuugugaacggcuacaggugcauaugcccccccggcuacgccggcgaucacugcgagcgggauauagacgagugugccagcaaccccugccucaacggggggcacugccagaaugagaucaacagauuucaaugccugugccccacaggauuuagcggaaaucugugccaacuggacaucgacuacugcgagcccaaucccugccagaacggggcccagugcuacaaccgggccagcgacuacuuuugcaagugccccgaggacuacgagggaaaaaacugcagccaccugaaggaccauugcaggaccacccccugugaggugauugacagcugcaccguggccauggccucaaacgacacccccgagggugugagguauaucagcucgaacgugugcggcccccacggcaagugcaagucacaaagcgggggaaaguucaccugcgacugcaacaagggcuucaccgguaccuacugccacgagaacaucaacgacugugagagcaaccccuguagaaacggggggaccugcaucgacggagugaauuccuauaagugcaucuguagcgacgggugggagggcgccuacugcgagaccaauaucaacgauugcagccagaaccccugccacaacgggggcaccugccgagaucucgugaacgacuucuacugcgacuguaaaaacgguuggaaaggcaaaaccugccacucccgcgauucccagugcgaugaggcgaccugcaauaauggaggcaccugcuacgacgagggcgacgccuuuaagugcaugugccccggcggcugggaaggcaccaccugcaauaucgcgagaaauagcagcugccugcccaaccccugccauaacggcgggaccugcguggugaauggcgagagcuucaccugcgucuguaaggagggcugggaaggucccaucugugcccagaacaccaacgacugcagcccccaucccugcuacaacagcggcaccugcguggacggcgacaauugguacaggugcgagugcgcccccggguuugccggccccgacugcaggaucaacaucaacgagugccagaguagccccugugccuucggcgccaccugcguggacgagaucaacggcuaccggugcgugugcccccccggccacuccggcgccaagugucaagaggugagcggacgacccuguaucaccaugggcucggugauccccgacggcgccaagugggacgacgacugcaacacgugccagugccucaacgggaggaucgccugcagcaagguguggugcggucccaggcccugccugcugcacaaaggccacuccgagugccccagcggccagagcuguauccccauccuggaugaucagugcuucguccaucccuguacuggcgugggcgagugcaggagcagcagccuccagcccgugaaaaccaagugcacgagcgacuccuauuaccaagauaacugugccaacaucaccuucaccuuuaacaaggagaugaugucgcccggacugaccaccgagcauaucugcagcgagcugaggaaccugaacauacugaagaauguguccgccgaauauuccaucuacaucgccugugagccuagcccgagcgccaacaacgagauccacguggccaucuccgccgaggauaucagggacgacgggaaccccaucaaagagaucaccgauaagaucaucgaccuggugucuaagcgcgacgguaacagcucccuaaucgccgccguggccgaggugcgcgugcagcgcaggccgcugaagaaccgcaccgacuuccuggugccccugcugagcagcgugcucaccguggccuggauaugcugccuggugaccgccuucuacuggugccugcggaagcggcguaaaccgggaagccauacccacagcgccagcgaggauaauaccaccaauaacgugcgggagcagcugaaccagaucaagaaccccaucgaaaagcacggggcgaacaccgugcccaucaaggacuacgagaauaagaacuccaagaugagcaagauccgcacacacaacagcgagguggaggaggacgauauggacaagcaccagcagaaggccagguucgccaagcagcccgccuacacccuuguggaccgcgaagagaagcccccgaacggcacccccaccaagcaccccaacuggaccaacaaacaggauaaccgugaccuggaaagcgcgcagucccugaaccgcauggaguacauagug

SEQ ID NO: 97 - RNA, 3654 nt, Artificial Sequence
  Synthetic polynucleotide
augaggagcccccggaccagggggcggagcggcaggccccugagccuccugcuggcccugcuuugcgcacugagggccaagguguguggggccagcgggcaguucgagcucgaaauccugagcaugcagaacgugaacggcgagcugcagaauggcaauuguugcggcggcgccaggaaccccggcgaccggaagugcacccgggacgaaugcgacaccuacuucaaggugugccucaaggaguaccagagccgcgugaccgccggcggacccugcagcuucggcagcggcagcacccccgugaucgggggcaacaccuucaaccugaaggcaucccgcgggaacgacaggaacaggaucgugcugccguucagcuucgccuggccgcgauccuacacgcugcugguugaggccugggacagcagcaaugacacggugcaacccgacagcauuaucgagaaggccagccacuccggcaugaucaaccccucccggcaguggcagacccugaagcagaacacuggaguugcacacuucgaguaccaaaucagggucacgugcgacgacuacuauuacggguucggcuguaacaaguucugcaggccccgugaugacuucuuuggacacuacgccugcgaccagaacggaaacaagaccugcauggaaggguggaugggccccgagugcaacagggccaucuguagacaaggcugcagccccaaacacggcuccuguaagcugcccggcgacugccggugccaguacggcuggcaggggcucuacugcgacaagugcauuccccaucccggcugcgugcacggcauauguaacgaacccuggcaaugccucugcgagaccaacuggggcgggcagcugugcgacaaagaccugaacuacuguggcacccaucagcccugccugaacggggggacuugcuccaauaccggucccgacaaguaucagugcagcugccccgagggcuacuccgggcccaacugcgagaucgccgaacacgccugucuguccgaccccugccacaacagaggcagcugcaaggagaccagccugggcuuugagugcgagugcucccccggcuggaccgggcccaccugcagcaccaacaucgacgauugcagccccaacaauugcucccacggcggcacuugccaagaccuggugaacggcuucaagugcgugugccccccccaguggaccgguaaaacaugccagcuggacgccaacgagugcgaggccaagcccugcgugaacgccaagagcugcaaaaaccugaucgccaguuacuacugcgacugccugccuggauggaugggccagaacugcgacaucaacaucaacgacugccugggccagugccagaacgacgcaagcugccgugaccuggugaacggcuacaggugcaucugcccccccggguacgccggugaccacugcgaacgggacauagaugagugcgccagcaaccccugccugaacggcggacacugccagaaugagaucaauagguuccaaugccucugccccaccggcuuuagcggcaaucugugccagcuggacaucgauuacugugagcccaaccccugccagaauggagcccagugcuacaaccgggccuccgacuauuucuguaagugucccgaagacuacgaggguaagaacugcucccaccugaaggaccacugccggaccacuccgugcgaggucaucgacagcugcaccgucgccauggccagcaaugacacacccgagggcgugagguacaucuccuccaacguguguggcccccacggcaagugcaagagccagagcggaggcaaguucaccugcgacugcaacaagggguucaccggcacuuacugccacgagaacaucaacgacugcgaauccaaccccugucgaaacgggggcaccugcauugacggcgugaacagcuauaagugcaucugcuccgacgggugggagggggccuacugcgaaaccaauauaaacgauugcagccagaaccccugucacaacgggggcacaugcagggaccuggucaacgacuucuacugugacugcaagaacggcuggaagggcaagacaugucacagcagggacagccagugcgacgaggccaccuguaacaauggcggcaccugcuaugacgaaggcgacgccuucaaauguaugugccccggcgguugggaggggacgacgugcaauauugcgaggaacuccagcugucugcccaaccccugccacaacggaggcaccuguguggugaacggcgagagcuuuacgugcgucuguaaagagggcugggaaggccccaucugcgcccaaaacacgaacgacugcagcccccaccccuguuacaauagcggcaccugcgucgacggugacaacugguauaggugcgagugugccccgggcuuugccgggcccgacugccggaucaauaucaacgagugccaguccagcccaugugcguucggcgccaccugcguggacgaaaucaacggcuacaggugcgucugccccccggggcacagcggagccaaaugucaggaagucucugggaggcccugcaucaccaugggcagcguaauccccgacggggcuaagugggacgacgacugcaauaccugucagugucugaacggcaggauugccugcagcaaagugugguguggcccgcggcccugucuccugcacaagggccacuccgagugucccagcggccaauccugcauccccauccucgacgaccagugcuuugugcaccccugcacaggcgugggagaguguaggucgagcucccugcagcccgugaagaccaagugcaccagcgauuccuacuaccaggacaacugcgcgaauaucaccuuuaccuuuaacaaggagaugaugagccccgggcugaccaccgagcacaucugcagcgagcugcggaaccugaacauccucaaaaacgucagcgccgaguauagcaucuacauugccugcgagcccagccccagcgccaacaacgaaauacacguggccaucagcgccgaggacaucagggacgacggcaacccgaucaaggagaucaccgauaagauaaucgaccugguguccaagagggacggcaauagcucccugaucgccgccguggccgaagugagggugcagaggaggccccugaaaaacaggaccgauuuccugguuccccugcugagcagcgugcugacaguggcuuggaucugcugccucguaacugcauucuacuggugccugaggaagaggaggaagcccggcagucacacccacagcgccuccgaggauaacaccacuaacaaugugcgggagcagcugaaccagaucaagaaucccauagaaaaacauggcgccaacaccgugcccauuaaagauuacgagaacaaaaauagcaagauguccaagauccgcacccacaacagcgagguggaggaggacgacauggacaagcaccagcagaaggccagguucgccaagcagcccgcguacacccugguggaccgugaggagaagccccccaacggcacccccaccaagcaccccaacuggaccaacaagcaagauaaucgggaccuggaauccgcccagagccugaacaggauggaguacaucgug

SEQ ID NO: 98 - RNA, 3654 nt, Artificial Sequence
  Synthetic polynucleotide
augaggagcccgagaacgagggggcgguccggcaggccgcugagccuccugcuggcccugcugugcgcccugcgggcaaagguguguggcgccuccgggcaguucgagcuggagauccugagcaugcaaaacgugaacggcgaacuccagaacggcaauugcugcggcggcgccagaaaccccggggaucgaaagugcacccgggacgagugcgacaccuacuucaaagugugucucaaagaauaccagagcagggugaccgccggcgggcccugcagcuucggcagcggcagcacccccgugaucggcgggaacaccuucaaccugaaggccagccgcggcaacgacaggaaucggaucguguugccguucagcuucgccuggccccguuccuacacccugcugguggaggccugggacagcagcaacgauaccgugcagccagacagcauaaucgagaaggccagccacuccgguaugaucaaccccagcaggcaguggcagacccugaagcaaaacaccggcguggcccauuucgaguaccagaucagggucacgugcgacgacuauuacuacggguucgggugcaacaaguucugcaggccccgggaugacuucuuuggacacuacgccugugaccagaacggaaacaaaacuugcauggagggcuggaugggcccggagugcaauagggccauuugcaggcaaggcugcagccccaagcacggcuccugcaagcuccccggcgacugccgaugccaauauggcuggcagggccucuacugugacaagugcaucccccacccgggcugcguccacggaaucugcaaugagcccuggcagugucugugcgagacgaacugggguggccagcugugcgacaaggaccugaacuacugcgggacccaccagcccugccugaacggcgggaccuguuccaacaccggcccggacaaguaucagugcagcugcccggaaggguacuccggcccgaacugcgaaaucgccgaacacgcuugccucagcgaccccugccacaaccgcgggagcugcaaggagaccagccugggcuuugagugcgaauguucccccggcuggaccgggcccacaugcuccaccaacauagacgauuguagccccaacaacugcucccacggggggaccugccaagaccuggucaacggauucaagugcgugugucccccccaguggacggguaagaccugccaacuggacgccaacgaaugcgaggccaagcccugugugaaugccaagagcugcaagaaccugaucgccagcuacuacugugacugccugcccggcuggaugggccagaauugcgacaucaauaucaacgacugccugggccagugccagaaugacgccuccugcagggaccuggugaacggcuacaggugcauaugcccccccggcuacgccggcgaccacugcgaacgugacaucgacgagugcgccucaaaccccugccugaacggcggacacugccagaacgagaucaaccgauuccagugucugugccccaccggguuuagcgggaaccucugccagcucgauaucgacuacugcgaacccaaccccugccagaacggcgcccagugcuacaaccgggccagcgacuauuucuguaaaugccccgaggacuacgaggggaaaaacuguagccaccugaaggaccacugcaggaccacacccugcgaagugaucgacagcugcaccguggccauggccagcaaugacacccccgaaggcgugagguauauaagcagcaacguaugcggcccccacggcaaguguaagagccagagcggcggcaaguuuacgugcgacugcaacaaaggcuucaccggcaccuacugucacgagaacaucaacgacugcgagagcaaccccugccgcaacgggggcaccugcaucgacggugugaacagcuacaagugcaucugcagcgacggcugggagggcgccuacugugagacgaacaucaacgacugcagccagaacccgugccauaacgggggcaccugcagggaucuggugaacgacuuuuauugcgacugcaagaacggcuggaagggcaagaccugccacagccgggacagccagugugacgaggccaccugcaacaacggcggcaccugcuacgacgaaggggacgccuuuaagugcaugugcccgggcgggugggagggcaccaccugcaacaucgccaggaauuccuccugucugcccaacccaugucacaacgguggcacgugcguggugaacggggaguccuuuaccugugugugcaaggaggggugggagggacccauaugugcgcagaauaccaacgacugcuccccccacccauguuauaacagcgguacauguguggauggggacaacugguaccggugugagugcgcccccggcuucgccggccccgauugcaggaucaacaucaaugagugccagagcucccccugcgccuucggcgccacaugcgucgacgaaaucaacggcuacaggugugugugccccccgggacacagcggugccaagugccaggaagugucaggcaggcccuguauuaccaugggcagcgugauccccgacggagccaagugggaugacgacugcaacaccugccagugccugaacggccguaucgccugcagcaagguguggugcggcccccggccgugccugcugcacaaggggcacuccgagugccccagcgggcagagcugcauccccaucuuggacgaccagugcuucgugcaccccugcaccggcgugggcgaaugccguagcagcucccugcagcccgugaagaccaagugcaccagcgauuccuacuaucaggauaacugcgccaacaucaccuucaccuucaacaaggagaugaugagccccggccugaccacggaacacaucugcagcgagcugaggaaccugaacauccugaagaacguguccgccgaauacagcaucuacaucgccugcgagcccagccccagcgccaacaacgaaauccacgucgccaucucugccgaggacauccgcgacgacggcaaccccauuaaggagauaaccgacaagaucaucgaccugguguccaagcgagacggaaauucuagccugaucgccgccguagccgagguacgugugcagaggaggccccucaagaauaggaccgacuuccuggugccccugcugagcagcgugcucaccguggcguggaucugcugccuggugaccgccuuuuacuggugccugcgaaagaggaggaagcccgguucacacacgcacagcgccagcgaagacaacaccaccaacaaugugcgcgagcagcucaaccagaucaagaaucccaucgagaagcacggcgccaacacgguccccaucaaggacuacgagaacaaaaacagcaagauguccaagauccgcacccauaacagcgaggucgaagaagacgacauggacaaacaccagcaaaaggccagguucgccaagcagccggccuacacccugguggacagggaggagaagcccccgaacggcacccccaccaagcaccccaacuggaccaacaaacaggacaaccgggaucuggagagugcgcagagccugaacaggauggaguacaucgug

SEQ ID NO: 99 - RNA, 3654 nt, Artificial Sequence
  Synthetic polynucleotide
augagaagcccaaggacgcgcgguaggagcggcaggccccucagccugcugcuggcucuacugugcgcccugcgggccaagguuuguggggccagugggcaauucgagcuggagauccugagcaugcaaaacgugaacggggagcuucagaaugguaacugcugcggcggggcccggaaucccggcgaccggaaguguacgagggaugagugugacaccuacuuuaaggugugccugaaggaguaccagagcaggguuacggcaggcggccccugcagcuuuggcagcggcuccaccccggugaucggcggcaacacauucaaccugaaggccagccgcgggaacgaucguaacaggaucgugcuccccuuuagcuucgccuggccccgcagcuacacgcugcugguggaggccugggacagcagcaacgacaccguccagcccgauagcauuaucgagaaggccucccacagcgguaugaucaacccgagccggcaguggcagacccugaagcagaacaccggcguggcccacuucgaguaccagauccgggugaccugcgacgacuacuauuacgguuucggcugcaacaaguuuugccgaccccgggacgacuuuuucgggcauuacgccugcgaccaaaacggcaacaaaaccugcauggagggcuggaugggcccggagugcaaccgggccaucugccggcagggguguagccccaagcacggcagcugcaagcugcccggcgauugccggugccaguacggguggcagggccuguacugcgacaagugcaucccgcaccccggaugugugcacggcaucugcaacgagcccuggcagugccugugcgaaaccaacugggggggucagcugugugacaaggaucugaacuacugcggaacccaccaacccugccugaacggcggaacuugcucgaacacgggccccgacaaguaccagugcagcugucccgagggcuacagcgggcccaacugugagaucgccgaacacgcuugccugagcgacccgugucacaaccggggcagcugcaaggagaccucccucggcuucgagugcgagugcuccccaggguggaccggccccaccugcagcaccaacaucgacgauugcagccccaacaacuguagccacggcgggacgugccaggaccuggucaacggcuucaaaugugucugucccccccaguggaccggcaaaaccugccagcucgacgccaacgagugcgaagccaagccgugcgugaacgcgaagagcugcaagaaccugaucgccuccuacuacugcgacugccugcccggcuggaugggccagaacugcgacauaaacaucaacgacugccugggccagugccagaacgaugccagcugucgagaccuggugaacggguaccggugcaucugcccccccggauacgccggggaccacugcgagcgcgacaucgacgaaugugccucgaaccccugccugaacgggggccacugccaaaacgagaucaaucguuuccagugccugugccccaccggcuucucugggaaccugugccagcuggacaucgacuacugcgagcccaaccccugccagaacggggcgcagugcuauaaccgggccuccgauuacuucugcaagugccccgaggacuaugagggaaaaaacugcucccaccugaaggaucacuguaggaccacccccugugaggugaucgacagcugcaccguggccauggccagcaacgacacccccgagggcgugcgcuacaucagcuccaacgugugcggcccccaugguaaguguaagucgcagagcggcgggaaguucaccugcgacugcaacaagggcuuuacggggaccuacugucaugaaaacaucaacgacugcgagagcaaccccugucgcaacggcggcaccugcaucgauggcgucaacagcuacaagugcaucugcuccgacggaugggagggcgccuacugcgagaccaacaucaacgacugcagccagaacccgugccacaauggcggcaccugccgugaccuggugaacgacuuuuacugcgacugcaagaacggguggaaaggcaaaaccugccacuccagggacagccagugcgacgaggcgaccugcaacaauggcgggacgugcuacgacgagggcgacgccuucaagugcaugugccccggcggaugggaaggcacuaccuguaacaucgcccggaauagcuccugccugccgaaccccugccacaacgggggcacgugcgucgugaacggcgaaagcuucaccugcgugugcaaggagggcugggagggccccaucugugcccagaacaccaacgacugcagcccccaccccugcuacaauagcggcaccugcguggacggagacaacugguaccgaugcgagugcgccccuggcuucgccggacccgauugccgcauuaacaucaaugaaugccagagcagccccugcgccuuuggagccaccugcgucgaugagaucaacggcuaccgcugugucugcccccccggccacagcggggccaagugccaggaggucucaggucggcccugcaucaccaugggcagcgucauccccgacggggccaaaugggaugacgacugcaauaccugccagugucugaacggccgaaucgccugcuccaagguguggugcgggcccaggcccugccuccuucacaaaggccauagcgagugccccuccgggcaauccugcauccccauccuggacgaccaaugcuucgugcaccccugcaccggcgugggggagugcaggagcagcagccugcagcccgugaagaccaagugcaccuccgauagcuauuaccaggacaacugcgccaacaucaccuucaccuuuaacaaagaaaugaugucacccggccugacgaccgagcauaucugcagcgagcugcggaaccugaacauccugaaaaacgugucggccgaguacaguauauacaucgccugcgagcccagccccagcgccaacaacgagauacauguggccauaagcgccgaagacaucagggacgauggcaaccccaucaaggagaucaccgacaaaauaaucgaccuggugagcaagcgggauggcaauagcagccugaucgccgccguggccgaggugagggugcagcggaggccccugaagaaucgcaccgacuuccuggucccgcugcuuagcuccguccugacggucgccuggaucugcugccuggugaccgccuucuacuggugcuugaggaagcggaggaagcccgggucacauacccacuccgccagcgaggacaacaccaccaauaacgugcgggaacagcugaaccagaucaagaaccccaucgagaagcauggugccaacaccgugcccaucaaggacuaugaaaacaagaacuccaagaugagcaagaucaggacccacaacuccgagguggaagaggacgacauggacaagcaccagcagaaagcccguuucgccaagcagcccgccuacacccugguggaccgagaggaaaagccgcccaacggcacccccaccaagcaucccaacuggaccaacaagcaggacaaccgugaccuggagagcgcccagucgcucaaccgcauggaguacaucgug

SEQ ID NO: 100 - RNA, 3654 nt, Artificial Sequence
  Synthetic polynucleotide
augcggucgccgagaaccaggggccggagcggccggccccugucgcugcugcuggcccugcucugcgcgcugagagccaagguguguggcgccagcggccaguucgagcuugagauccuguccaugcaaaacgucaacggcgagcuccagaacggaaacuguugcggcggcgcccgcaaccccggcgacaggaagugcacccgcgacgagugcgacaccuacuucaaggugugccugaaggaguaccagucccgcgugaccgcuggcggaccgugcagcuucggcucaggcagcacccccgugaucgggggcaauaccuucaaucucaaggccagccgaggaaacgacaggaacaggaucgugcuccccuuuagcuuugccuggccucguagcuacacccugcugguggaggccugggacucaagcaaugacacgguucagcccgacagcaucaucgaaaaggccucucacagcggaaugaucaaccccagcaggcaguggcagacccucaagcagaacacgggcguggcccacuucgaguaccagauccgugugaccugcgaugacuacuauuacgguuucggguguaauaaguucugcaggcccagggaugacuuuuuuggccacuacgccugcgaccagaauggcaacaagaccugcauggagggauggaugggccccgagugcaaccgugccaucugucggcagggcugcucgcccaagcacggcagcugcaagcuucccggcgacugucggugccaguacggauggcaagggcuguacugcgacaagugcaucccccaucccggcuguguccacgguaucugcaacgagcccuggcagugucugugcgagaccaacuggggcggccagcugugcgacaaggaccugaacuacugcggcacccaccagcccugccugaaugggggcaccuguucuaacaccgggccggacaaguaccaguguuccugccccgagggcuacagcggccccaacugcgagaucgccgagcacgccugccuguccgaccccugccauaauaggggcuccugcaaggagaccucccugggcuuugagugcgaguguucgcccggcuggaccggccccaccugcaguaccaacaucgacgacugcagccccaacaacuguagccacggcggcacaugccaagaccuggugaacggcuucaagugcgucugcccgccgcaguggaccgggaagaccugucagcuggaugccaacgagugcgaggcuaaacccugcgugaacgcgaagagcuguaagaaccugauugccagcuacuacugcgacugccugccgggcuggauggggcagaauugcgacaucaacaucaacgacugucugggccaaugccagaacgacgccagcugucgggaccuggucaacggauacagguguaucuguccccccggcuacgccggcgaccacugcgagcgggacaucgacgaaugcgccagcaacccuugucugaacggaggccacugccagaacgagaucaacagguuucagugccucugccccaccggguucagcgggaaccugugccagcuugacaucgauuacugcgagcccaaccccugucagaauggggcgcagugcuacaaccgagcuuccgauuacuucugcaagugccccgaggauuacgaggguaaaaauugcagccaccugaaggaucacugcaggaccaccccgugcgaggugauagacagcugcaccguggccauggccagcaacgacacccccgagggcgugcgauacaucagcagcaacgugugcggcccccacggcaagugcaaaagccagagcggcggaaaauucacaugcgacugcaacaagggguucacgggcaccuauugccacgagaacaucaacgacugcgaguccaacccgugccggaauggcggcaccugcaucgacggcgugaacuccuauaaguguaucugcucggacggcugggagggggccuauugcgagaccaacaucaacgacugcagccagaaccccugccacaacggcggcaccugcagggaccuggugaacgacuucuauugcgacugcaagaacggcuggaagggcaagaccugucacuccagggacagccagugcgacgaggccaccuguaacaacggcgggaccuguuacgacgagggggacgcguucaagugcaugugccccggcggcugggagggcaccacgugcaacaucgcgcguaacagcagcugucugccgaaucccugucacaauggcggcaccugcgucgugaacggcgaaagcuucaccugcguguguaaggaaggcugggagggccccaucugcgcccaaaacaccaacgacuguagcccccacccgugcuacaacagcggcaccugcguggauggcgacaacugguaucggugcgagugugccccuggcuuugcgggccccgacugccggauaaacauaaacgagugucaaucgagccccugcgccuucggggccaccugcguggacgagaucaacggcuacaggugcgugugcccgcccggccacagcggcgcgaaaugccaagaggugagcggcaggcccugcaucaccauggguuccgugauccccgacggggcaaaaugggacgacgacugcaauaccugccagugccucaacgggaggaucgccugcagcaagguguggugcggccccaggcccugccugcugcauaaagggcacagcgagugccccagcgggcagagcugcauccccauccuggacgaccagugcuucgugcacccgugcaccggcgugggcgagugcagaagcucuagccugcaacccgugaagaccaagugcacgagcgacagcuacuaccaggacaacugcgcgaacaucaccuucaccuucaauaaggagaugaugagcccgggacucaccaccgaacauaucugcuccgagcugcgcaaccucaacauacugaagaaugugagcgccgaguacuccauuuacauugccugcgagcccagccccuccgccaauaaugaaauacacgucgccaucagcgccgaggacaucagggacgacggcaaccccaucaaggagaucaccgacaagaucaucgaccuggugagcaaaagggacggcaauagcagccucaucgccgccguggccgaggugagggugcagaggaggccgcugaaaaacagaaccgauuuucucgucccccugcuguccuccgugcugaccgucgccuggaucuguugccuggugaccgccuucuacuggugucuccgcaagaggcgcaagcccggcagccacacgcauagcgccagcgaggacaacacuacuaacaacgugcgggagcagcugaaucagaucaagaaccccaucgagaaacacggcgccaacacugugcccaucaaagacuacgagaacaaaaacucgaaaaugagcaagauccgcacccacaacagcgagguggaggaggacgacauggacaagcaccagcagaaagcgagauucgccaaacagcccgccuacacccugguggacagggaggagaagcccccaaacggcacacccaccaagcacccgaacuggaccaacaagcaggacaaccgugaccuggaaagcgcccagucccugaaucgcauggaauauaucgug

SEQ ID NO: 101 - RNA, 3654 nt, Artificial Sequence
  Synthetic polynucleotide
augcgaagcccccgaacccggggcaggagcgggaggccccugagccugcugcuggcccuucugugcgcccuuagggccaagguguguggggccuccggccaguucgagcuggagauccugagcaugcagaacgugaacggugagcugcagaaugguaacuguugcggcggagccaggaacccgggcgauaggaaauguaccagggacgagugcgacaccuacuuuaaggugugccucaaagaguaccagagccgggucaccgccggcggccccugcucguucggcagcgguagcacccccgugaucggcggcaacacauucaaccugaaagccagcagggggaacgacaggaaccggaucgugcuccccuucuccuucgccuggcccaggucguacacccugcucgucgaggccugggacagcagcaacgacaccgugcagcccgacagcaucaucgaaaaggccagccacagcggaaugaucaaccccagccgacaguggcagacccugaagcagaacaccggcguggcccacuucgaguaccagauccgggugaccugcgaugacuauuacuauggcuucggcuguaacaaguucugucgacccagggacgacuucuucggccacuaugccugcgaccagaacgguaauaagacuugcauggagggcuggaugggccccgaguguaacagggccaucugcaggcagggcugcucccccaaacacggcuccugcaaacugcccggcgacugccgcugccaguacggcuggcaggggcucuacugcgauaagugcaucccccaucccggcugcgugcauggcaucugcaacgaacccuggcagugccugugcgagaccaacugggggggccagcuaugcgauaaggaucugaacuacuguggcacccaccagcccugccugaacgggggcacgugcucaaacaccggccccgacaaauaccaaugcagcugccccgagggcuacagcggccccaacugcgagaucgccgagcaugccugccugagcgacccgugccacaauaggggcuccuguaaggagaccagccugggcuucgagugugagugcagccccggcuggaccggccccaccugcucaacuaacaucgacgacuguucccccaacaauugcagccacggcggcaccugccaggaccuggugaacggcuuuaagugugugugccccccccaguggaccgggaagaccugucagcuggacgcuaacgagugugaggccaagcccugugucaacgccaaaagcugcaagaaccugauagccuccuacuacugcgacugccugcccggauggaugggccagaacugcgacaucaacaucaaugacugccuggggcagugccagaacgacgccagcugccgggaccuggugaauggguaccgcugcaucugcccccccggcuacgcgggcgaccacugcgagagggacaucgacgagugcgccucgaaccccugccucaacgggggccacugccagaacgagaucaaccgguuccagugucugugcccuacuggcuucucuggcaaccugugucagcuggauaucgauuacugcgagccaaacccaugccagaacggggcccagugcuacaauagggccuccgacuauuuuugcaagugccccgaggacuacgaggguaagaacuguucccaucucaaggaccacugucgaaccacccccugcgaggugaucgacagcugcaccguggccauggccagcaaugacacccccgagggcgugcgguacaucuccagcaacgugugcggcccccacggcaagugcaagagccaguccggcggcaaauuuaccugcgauugcaacaagggguucaccggcaccuacugucacgagaacaucaaugacugcgaauccaaucccugcaggaacgguggcacgugcaucgacggggugaauagcuauaagugcaucugcagcgacgggugggaaggggccuacugcgagaccaacaucaacgacuguagccagaacccgugccacaauggcggcacuuguagggaucucgugaaugacuucuauugcgacugcaaaaauggauggaaggggaagaccugccacucccgggacucccagugcgacgaggccaccugcaauaacggcgguaccugcuacgacgagggcgaugccuuuaaaugcaugugccccggcggcugggagggaaccacgugcaacaucgcgaggaacagcagcugccuccccaaucccugucacaauggcgguaccugcgucgugaacggggagagcuucaccugcgugugcaaggagggcugggagggcccgaucugcgcccagaacaccaacgacugcagcccacaccccugcuacaauagcgggaccugcguggacggagacaacugguaccggugcgagugcgcccccggcuucgccggccccgacugcaggaucaacaucaacgagugccagagcagccccugugccuucggcgcgaccugcguggaugaaaucaauggcuaccggugcgugugcccccccggccacagcggcgcgaagugccaggagguuagcggcaggcccugcaucaccaugggaucggugauccccgauggcgccaagugggaugacgacuguaacacaugccaaugucugaauggacggaucgcauguuccaagguguggugcggccccaggcccugucuccugcacaaaggccacagcgagugucccagcggccaaagcugcauccccauccuggacgaccagugcuucgugcaucccugcaccggcgugggggagugccguagcagcagccugcagcccgugaagacgaagugcaccucagacagcuauuaccaggauaacugcgcgaacaucaccuucaccuuuaacaaggagaugaugucccccggccugaccaccgagcacaucugcucggagcugcgcaaucuuaacauccugaaaaacguguccgccgaguacagcauuuacaucgccugugagccgagccccuccgccaacaaugagauccaugucgccaucagcgccgaggacauccgggacgacgguaauccgaucaaggagaucacagauaagaucaucgaccugguguccaagcgggacggcaacagcagccugaucgccgccgucgccgaggugcgugugcagagacggccccucaagaaccgcaccgacuuccucgugccccuccugagcucggugcugaccgucgccuggaucugcugccuggugaccgccuucuacuggugccugcgaaaacgccggaagccggggagccacacccacagcgccagcgaggauaacaccaccaauaacgugagggaacagcugaaccagaucaagaaccccaucgaaaaacacggcgccaacaccgugccgaucaaggacuacgagaacaaaaauagcaagaugagcaagaucaggacacacaacucugagguggaggaggacgacauggacaagcaccagcagaaggcccgcuucgccaagcagcccgccuacacccuggucgaccgggaagagaagcccccgaacggcacccccaccaagcauccuaacuggaccaacaagcaagacaacagggaccuggaaagugcccagagccugaaccggauggaguacaucgug

SEQ ID NO: 102 - RNA, 3654 nt, Artificial Sequence
  Synthetic polynucleotide
augcgaagcccgaggacccggggcaggagcggcaggccgcuaagccugcugcuggcccuccucugcgcccucagggccaaggugugcggcgccuccggccaauucgagcucgagauccugucaaugcagaacgugaacggcgagcugcagaacggcaacugcugcggcggcgccaggaaccccggcgacaggaagugcaccagggacgaaugugacaccuacuucaaggugugccugaaggaguaccagagccgggugaccgcuggcggcccauguagcuucgggagcggcagcaccccggugaucggggguaacaccuuuaaccucaaggcuucccgcggcaacgacaggaaccggaucgugcugcccuucuccuucgccuggcccaggagcuauacccugcuggucgaggccugggacagcuccaacgacaccgugcaacccgacagcaucaucgagaaggccucccacuccggcaugaucaaccccagcaggcaguggcagacccucaagcaaaacaccggggucgcgcacuucgaguaccagaucagggucaccugcgacgacuacuacuacggcuucggcugcaauaaguuuugccggcccagggacgauuucuucggacacuacgccugugaccagaauggcaauaagaccuguauggaaggguggauggggccagagugcaaucgggccaucugcaggcaaggcugcagccccaaacacggcucguguaagcugcccggcgacugcaggugccaguaugguuggcagggccucuauugcgacaagugcaucccccacccaggcugugugcauggcaucuguaacgaacccuggcagugccugugcgagacgaacugggggggccaacugugcgacaaggaccugaacuauugcggcacccaccagccgugccugaauggcggaaccuguuccaacaccggccccgacaaguaccagugcuccugucccgagggguacagcggccccaacugcgagaucgccgagcaugccugccucagcgaucccugccacaacaggggcagcugcaaggagacgagccugggcuucgagugcgaaugcagccccgguuggaccggccccacgugcuccaccaacaucgacgacugcucccccaacaauugcagccacgggggcacaugucaggaccuggugaacggcuucaagugcgugugcccgccccaauggaccggcaagacgugccagcuggacgccaacgagugcgaagccaagccaugcgugaacgccaagagcugcaagaaccugaucgccagcuacuacugcgacugccucccaggcuggaugggccagaacugugauaucaacaucaacgacugccucggccagugccagaacgacgccagcugccgggaccuggugaacggguaccgcugcaucuguccgcccggcuacgccggagaccacugcgagcgcgacaucgacgagugugccagcaaccccugcuuaaacggcggccacugccaaaaugaaaucaauagguuucagugccugugccccaccggguucagcggcaaccugugccagcuggacaucgacuauugcgagccgaaccccugccagaacggggcccagugcuacaauagggccagcgauuauuucugcaagugucccgaggacuacgagggaaaaaacugcagccaccucaaggaccacuguaggaccacgcccugcgaagugaucgacuccugcaccguggccauggccagcaacgacacccccgagggcgugcgcuacaucagcagcaacguguguggcccucacggcaaaugcaagagccaaagcggcggcaaguucaccugugacugcaauaagggcuucaccggcaccuacugucacgagaacaucaacgacugcgagagcaaccccugcagaaacgguggcaccuguauagauggcgugaacagcuacaagugcaucugcagcgacggaugggaaggcgccuacugugagaccaacauuaacgacugcagccagaaccccugccacaauggcggcaccugccgcgaccuggucaaugacuuuuacugcgacuguaagaacggguggaagggcaagaccugccauagccgcgacucccagugcgacgaggcaaccugcaacaacggcggcaccuguuaugaugagggggacgcauucaagugcauguguccggggggcugggagggcacaaccugcaacaucgcccggaacagcagcugccucccaaaccccugccacaacgggggcaccugcguggugaacggcgagagcuucaccugcguguguaaggagggcugggagggccccaucugugcccagaauaccaacgauugcuccccccaccccugcuacaacagcggcacuugcguggacggcgauaacugguauaggugugagugcgcccccggcuucgcaggccccgacugccgcaucaacaucaacgagugccagagcagccccugugccuucggggccaccugcguggacgagaucaacggcuaccggugugugugcccccccgggcacuccggcgcgaaaugccaggagguguccggcaggcccugcaucaccaugggcagcgugaucccugacggcgccaaaugggacgacgacuguaauaccugccagugccugaauggccgaaucgccugcuccaagguguggugcggccccaggccuugccuguugcacaagggccacagcgagugccccagcggccagagcuguauccccauccuggacgaccaauguuucgugcaucccugcaccggcgugggggagugccggucguccagccugcagcccgugaagaccaaguguaccagcgacuccuacuaucaggacaauugcgccaacaucaccuucaccuuuaacaaggagaugaugagccccggccugaccaccgagcacaucuguuccgagcugaggaaccugaacauccugaagaacgucagugccgaguacuccaucuacaucgccugugaaccguccccguccgccaacaaugagauucacguggccaucagcgccgaagacaucagggacgacggcaaccccaucaaggagaucaccgacaagaucauagaccuuguguccaagagggacggcaacucgucccugaucgccgccguggcggaggugagggugcagaggaggccccugaagaaccgcaccgacuuccuggugccgcuccuguccuccgugcugaccguggccuggaucugcugccuggugaccgccuucuacuggugccugaggaagcgccgcaagcccgggucccacacgcacagcgccagcgaggauaacaccaccaacaacgugcgggagcaacugaaccagauaaagaaccccaucgaaaaacacggagcgaacaccguccccaucaaggacuacgaaaacaagaacagcaagaugagcaagaucaggacccauaacuccgagguggaggaggacgacauggacaagcaccagcaaaaggcccgguucgccaagcagcccgccuacacccugguggaucgggaggagaagccccccaacgguaccccgaccaaacaccccaacuggaccaauaaacaggacaauagggaccuggaguccgcccagagccugaacaggauggaguacauagug

SEQ ID NO: 103 - RNA, 3654 nt, Artificial Sequence
  Synthetic polynucleotide
augagaagccccaggacccgaggcaggagcggcaggccacugagccugcuccuugcccugcugugcgcccugagggcaaaggugugcggcgccagcggccaguucgagcuggaaauccuguccaugcagaacgugaacggggagcugcagaauggcaauugcuguggcggcgcgcggaaccccggcgacaggaagugcacacgggacgaaugcgacacguacuucaaggugugccucaaggaguaccaguccagggucaccgccggcgggcccugcagcuucggaagcggcuccacccccgugaucggcggcaacacauucaaccugaaagcgucgagggggaaugaccgcaacaggaucgugcugccguuuuccuucgccuggccccgcagcuacacgcugcugguggaggcaugggacagcuccaacgauaccgugcagcccgacagcaucaucgagaaggccucccacagcggcaugaucaacccgagcaggcaguggcagacccucaagcagaacaccggcguggcccacuucgaguaucagauccgggugaccugcgacgacuauuacuacgguuucggcugcaacaaguuuuguaggccccgagacgacuucuucggccacuacgccugcgaucagaacgggaauaaaaccuguauggagggguggaugggccccgagugcaacagggccaucugcaggcagggaugcucccccaagcacggcagcugcaagcugccaggagacugcaggugucaguauggcuggcaggggcuguacugcgauaagugcauuccgcacccaggaugugugcacggaaucuguaacgagcccuggcagugccugugcgaaaccaacugggggggccaacucugcgacaaggaccugaacuacugcggcacccaccaacccugucugaacggcggcaccugcagcaacaccggccccgacaaauaccagugcagcugccccgagggcuacuccgggcccaacugcgagaucgccgaacacgcaugucugagcgacccuugccacaacaggggcagcugcaaggagaccucccucggcuuugagugcgaaugcagccccggcuggaccgggcccaccugcagcacgaacaucgacgacugcagccccaacaacugcucccacggcgggacgugccaggaucucgucaacggcuucaagugcgugugccccccccaguggaccggcaaaaccugccagcuggacgcaaacgagugcgaagccaagccgugcgucaacgcgaagagcugcaagaaccucaucgccagcuacuauugcgacugccugcccggcuggaugggccagaacugcgacauaaacaucaacgacugccugggccagugucagaacgaugccuccugcagggaccuggugaacggguaccgguguaucugcccccccggguacgcgggggaccacugcgagagagacaucgaugagugcgccuccaaucccugccugaacggcggccauugccagaacgagaucaaccgguuccagugccugugccccaccggcuucuccggcaaccugugccaacuagacaucgacuacugcgagcccaaucccugccagaacggcgcccaaugcuacaacagggccagcgacuacuucuguaagugccccgaggacuacgagggcaagaacugcucccaucugaaggaccacugccggaccacccccugcgaagugaucgacagcugcaccguggccauggccagcaaugacacccccgagggcgugagguauaucagcagcaacgugugcgggccccacgggaaaugcaagagccagagcggcggcaaguucacaugcgacuguaacaagggcuucacgggaaccuacugucacgagaacaucaacgacugcgagagcaaccccugccgcaacggcggcaccugcaucgacggcgugaacuccuauaagugcaucuguagcgauggcugggaaggggccuacugcgagaccaacauaaacgacugcagccagaaucccugccauaacgggggcaccugucgugaccuggucaacgacuucuacugcgacuguaagaacggauggaaggguaagaccugccacuccagggacucccagugugacgaagccaccugcaacaacggaggcaccugcuacgacgagggugacgccuuuaagugcaugugccccgguggcugggaggggaccacgugcaacaucgcccgcaacagcagcugccuuccgaacccaugccauaacggcggcaccugugucgugaacggcgagucguucaccugugugugcaaggaaggcugggaaggccccauaugcgcccagaacaccaacgacugcagcccccaucccugcuacaacuccggcaccugcguggacggggacaacugguacaggugugagugcgcccccggauucgccggucccgacugccggaucaacaucaaugagugucaauccagccccugcgccuucggcgccaccugcguggaugagaucaacggcuacaggugcgucuguccccccggccacuccggcgccaaaugccaggaggucagcggcaggcccugcaucaccaugggcuccguuauccccgacggcgccaagugggacgacgacugcaauaccugccagugucugaacgggaggaucgccugcuccaagguguggugcggccccaggcccugccugcugcacaagggccacagcgagugccccagcggccaguccugcaucccgauccuggacgaccagugcuuugugcaccccugcaccgggguaggcgagugccgguccagcagccugcagcccgugaaaaccaagugcaccagcgacagcuauuaccaggacaacugcgccaauaucaccuuuacguucaauaaagagaugaugagccccggccugaccaccgaacacaucugcagcgagcugcgcaaccugaacauucugaagaacgugagcgccgaguacagcaucuauauagccugcgagcccagccccucggcuaauaacgagauccacguggccauaagcgcggaggacauccgggacgacggcaaccccaucaaggagaucaccgacaagaucaucgaccuggugagcaagcgcgacgggaacucaucacugaucgccgccguggccgaggugagggugcagaggcggccccucaagaacaggaccgacuuccucgucccccugcugucgagcgugcucaccguggccuggaucugcugucucgugaccgcauucuacuggugccugaggaaacggcgcaagcccggcucgcacacccacagcgccagcgaagauaacaccaccaacaacgugagggagcagcucaaccagaucaagaaccccauagagaagcacggcgccaacacggugccaaucaaggacuaugagaacaagaacagcaagauguccaagauccgcacccacaacagcgaagucgaggaagacgacauggacaagcaccagcagaaagcgcguuucgccaagcagcccgccuacacccugguggacagggaggagaagccccccaacggaacccccacaaagcacccaaacuggacgaauaagcaggacaacagggaccuggagagcgcccagagucugaaccggauggaguacaucgug

SEQ ID NO: 104 - RNA, 3654 nt, Artificial Sequence
  Synthetic polynucleotide
augagaagucccaggacccgcgggcggagcgggcgcccccugagccuguuacuggcccuccugugugcccugcgcgcgaaggugugcggggccagcggccaguucgagcuggagauccugagcaugcagaacgugaacggggaacuacagaacggcaacugcugcggcggcgcccgcaauccgggagacaggaaguguaccagggaugagugcgacaccuacuuuaaagugugccugaaggaguaccagagcagggugaccgccggcggccccuguagcuucggcagcgggagcaccccggugaucggcggcaacaccuucaaccucaaggccuccaggggcaacgacaggaaccggaucgugcugcccuucagcuucgccuggccccgcagcuacacgcugcugguggaggccugggacagcucuaaugacacggugcagccugacucaauuauagagaaggccagccacagcggcaugaucaaccccucaagacaguggcagacccugaagcagaacaccgguguggcacacuucgaguaucagaucagggugacaugcgaugacuacuacuacggguuuggcuguaauaaguucugcaggccccgagacgauuucuucgggcacuaugccugcgaccaaaauggcaacaagaccugcauggagggguggaugggcccggaguguaaccgagccauauguaggcaaggcugcagcccgaagcacggcuccugcaagcugcccggugauugcaggugccaguacggcuggcaaggccucuacugcgacaagugcaucccgcaccccgguugcguccacggcaucugcaacgagcccuggcagugccugugcgagaccaacugggggggccagcugugcgacaaggaccucaauuacuguggcacccaccagcccugccucaacgguggcaccugcuccaacaccggccccgacaaguaccaguguagcugccccgagggguacagcggcccgaacugcgagaucgccgagcacgccugccuguccgaccccugccacaaucgcggcagcugcaaggagaccagccugggguucgaaugcgaguguuccccgggcuggaccggccccaccugcagcaccaauaucgaugacugcucccccaacaacugcagccacggcggcaccugucaggaccuggugaauggcuucaagugugugugcccaccgcaguggaccggcaaaaccugccagcucgacgccaacgagugcgaggccaagcccugugugaaugccaaguccugcaagaaccugaucgccagcuacuacugcgacugccugcccggguggauggggcaaaauugcgacauaaacauaaacgacugccugggccagugccagaacgacgccuccugucgggaccuggucaacggcuacaggugcaucugcccacccggcuacgccggcgaccacugcgagcgagauaucgacgaaugcgccagcaaccccugccugaacggggggcacugccagaaugagaucaacagguuucagugccugugccccaccggcuucagcggcaaccugugucaacuggacaucgacuauugugagcccaacccuugccaaaacggggcccagugcuacaaccgggccagcgauuacuucugcaagugccccgaggacuacgaaggcaagaacugcagccaccugaaggaccacugucggaccacccccugcgaagugaucgacagcugcaccguggccauggccagcaacgacacccccgagggcgugagguacaucagcagcaauguguguggcccgcacggcaagugcaagagccagagcggcggcaaguucacgugcgacugcaacaagggcuuuaccggcaccuacugccacgaaaacaucaaugacugcgagagcaacccgugucggaacggcggcaccugcaucgacggggugaacagcuacaagugcauaugcagcgacggcugggagggcgccuacugugaaaccaacaucaacgacugcagccagaaccccugccacaauggcgggaccugcagggaccuggugaaugacuucuacugcgacugcaagaacggcuggaagggcaaaaccugccacagcagggacagccagugcgacgaggccaccugcaacaacggcggcaccugcuaugacgagggcgacgccuucaagugcaugugccccggcggaugggagggcacgaccugcaauaucgcaaggaacagcuccugucugcccaaucccugccacaacggcgguaccugcguggugaacggggaaagcuucaccugcgugugcaaggaggggugggaggggcccaucugcgcccagaacaccaacgacugcagcccacaccccugcuacaauuccggcaccuguguggacggcgacaacugguauaggugcgagugcgcccccgguuucgccggcccggacugcaggaucaacaucaacgagugucaguccagccccugcgccuucggggccaccugcguggacgagaucaacggcuaucguugcgugugcccccccggccacuccggcgccaagugccaggaaguguccgggcgccccugcaucaccaugggcuccgugauccccgauggcgccaagugggaugacgacugcaacaccugucagugccugaacggcaggaucgccugcagcaagguguggugcggcccccgacccugccugcugcacaaggggcacagcgagugccccuccggccaguccugcauccccauacuggacgaucagugcuucgugcaccccugcaccggcgugggcgaguguaggagcuccagccugcagcccgugaaaaccaagugcaccucggacagcuacuaucaggauaacugcgccaacauuacguucaccuucaacaaggagaugaugucccccggccugaccacggagcacaucuguuccgagcugaggaaccucaacauccugaaaaaugugagcgccgaguauagcaucuauauagccugugagccgucccccuccgccaacaacgagauccacgucgccaucuccgcagaggacauucgcgacgacgggaaccccauaaaggaaauuacggacaaaaucaucgaccuggugagcaagagggacggcaacuccagccugaucgccgccguggccgaggugcgcgugcaacgcaggccgcugaaaaacaggacggacuuucuggugccgcugcuguccucggugcugaccgucgcuuggaucugcugccuggugaccgccuucuacuggugccugcgcaaaaggcgcaagcccgguagccauacccacuccgccuccgaagacaacaccaccaacaacgugagggagcagcugaaucagaucaagaacccuaucgagaagcacggcgccaacacggugcccaucaaggacuaugaaaacaagaacagcaagauguccaagaucaggacccacaacagcgagguggaggaagacgacauggacaagcaccagcagaaggcccgauucgccaagcagcccgcuuacacccugguggacagggaggaaaagcccccgaacggcacccccaccaaacaccccaacuggacuaauaaacaggacaaccgagaccuggagagcgcccagagccugaacaggauggaauauaucguc

SEQ ID NO: 105 - RNA, 3654 nt, Artificial Sequence
  Synthetic polynucleotide
augcguagccccaggaccagggguagguccgggaggccccugucacuccuccuggcccugcucugugcccuccgggccaaggugugcggcgccagcggacaguuugagcuggagauccuguccaugcagaacgugaacggugagcuccagaacgggaacugcugcggcggcgccaggaaccccggcgaucgcaaguguaccagggacgaaugugacaccuacuuuaaggugugccugaaagaguaccagagccgcgucaccgccggcgggcccuguuccuuuggcuccggcagcacucccgugaucggcggcaacaccuucaaccucaaggcgagcagggggaacgacaggaacaggaucgugcugcccuucagcuucgcguggccccgguccuacacccugcucguggaggcuugggacuccucaaacgacacgguccagccggauagcaucauugagaaggcgagccacuccggcaugaucaaccccagccggcaguggcagacccucaagcagaacaccggcguggcccacuucgaguaucagauccgcgugaccugcgaugauuacuacuacggcuuuggaugcaacaaguucugccggccccgcgacgacuucuucggacacuaugccugugaccagaacgggaacaagaccugcauggagggauggaugggucccgagugcaaccgggccaucugcaggcagggcuguagccccaagcacgggagcugcaagcugcccggcgacugcaggugccaguacggcuggcaggggcuguacugcgacaagugcaucccccacccgggaugcgugcacggcaucugcaacgagcccuggcagugccucugcgagaccaacuggggcggccagcugugcgacaaggaccugaacuacuguggcacgcaucagccaugccucaaugguggcaccugcagcaacacgggccccgauaaguaccaaugcucgugccccgaaggguacuccggcccaaauugcgagaucgccgagcacgccugccuguccgaccccugccacaacaggggcuccuguaaggagaccucccugggcuucgagugugagugcagccccggguggaccggccccaccuguuccaccaacaucgacgacugcagccccaacaacugcagccauggaggcaccugucaggaccuggugaaugguuucaagugugugugcccgccccaguggaccgggaagaccugccagcuggacgccaacgagugcgaggcuaagcccugcgucaacgccaagagcugcaagaaccucaucgccuccuacuacugcgacugccugccgggauggaugggccagaacugugacaucaacaucaacgacugucugggccagugccagaaugacgccagcugccgagaccuggucaacggcuacaggugcauaugcccccccggauaugccggggaucacugcgagcgggacaucgacgagugcgccagcaacccaugucugaacggcgggcacugccagaacgagaucaacagguuucaaugccugugccccaccggauuuagugggaaccucugucagcuggacauagacuacugcgagccgaaccccugccaaaacggcgcgcagugcuacaacagggccagcgauuacuucugcaagugcccggaggacuacgaggggaagaacugcucccaccugaaggaccacugcaggaccacccccugcgaggugaucgacucgugcaccgucgccauggccucaaacgacacccccgaggggguccgcuacaucucgagcaacgucuguggcccccacggcaagugcaagagccagagcggggggaaguucaccugcgacugcaacaaaggcuucaccggcacguacugucacgagaacaucaaugauugcgagagcaaccccugccggaacggcggcaccugcaucgacggcgugaacagcuacaagugcaucuguagcgacggcugggagggggccuacugcgagaccaacaucaacgacugcagccagaaccccugucacaacggcggcaccugcagggaccucgugaaugacuucuacugcgacugcaaaaacggguggaaagguaaaaccugccauagccgggacagccagugcgacgaggccaccuguaauaacggcggcaccugcuacgacgagggugacgccuuuaaguguaugugccccggcggcugggagggcaccaccugcaauaucgcccgcaacagcagcugucuccccaaccccugccacaacggggguaccugcguggucaacggcgaguccuuuaccugcgugugcaaggagggcugggaagggcccaucugcgcccagaacaccaacgacuguagcccccaucccugcuacaacuccgguaccugcguggacggcgacaauugguacaggugugaaugcgcaccaggcuucgcggggcccgacugcaggaucaacaucaacgaaugccagagcagccccugcgcguucggcgccaccugcguggacgagaucaacggguacaggugcgugugcccccccgggcacagcggggccaagugccaggaggucuccgggcggcccugcaucaccaugggcuccgugaucccggauggggcgaagugggacgacgauugcaacaccugccaaugccugaacgggaggaucgccuguagcaaggucuggugcggaccccggcccugccuccugcacaaaggccacuccgaaugccccagcggacaaagcugcauaccgauccuggacgaccaaugcuucgugcaucccugcacaggcgugggugaaugcaggagcuccagccugcagccagugaagacgaagugcaccagcgauagcuacuaccaggauaauugugccaacauaaccuucaccuucaacaaggagaugaugucccccggccugaccaccgagcacaucuguagcgagcuccgcaaccugaacauccucaagaacgugagcgccgaguacuccaucuacaucgccugcgagcccucgcccagcgccaauaacgagauccacguggccaucuccgccgaggacauccgcgacgacggcaaucccaucaaggagauuaccgacaagaucaucgaccuggugagcaagcgcgauggcaacagcagccugaucgccgcgguggccgaggugagggugcagaggcggccccucaagaaccgcacggacuuccuggugccacugcugagcuccgugcugaccguggccuggaucugcugucuggucaccgccuucuacuggugccugcggaaacggaggaagcccggaucccacacccacuccgccuccgaagacaacaccacgaacaacgucagggagcagcugaaccagaucaagaaccccaucgagaagcauggcgccaacaccgugccaaucaaagacuacgagaacaagaacagcaagaugagcaagauccggacccacaacagcgaaguagaagaggacgacauggauaagcaccagcagaaggccagguucgccaagcaacccgccuacacccucguggaccgcgaggagaaaccccccaacggcacccccaccaagcaccccaauuggaccaacaagcaagauaaccgcgaccuggagagcgcccagagccucaaccggauggaauacaucgug

SEQ ID NO: 106 - RNA, 3654 nt, Artificial Sequence
  Synthetic polynucleotide
augaggagcccaaggaccagggggaggagcggcaggccgcucagccugcugcucgcccugcugugcgcccugcgggcaaaggugugcggggccagcggccaguucgagcuggaaauccugagcaugcagaacgugaacggcgagcugcaaaaugguaauugcugcgggggcgccaggaacccgggcgacaggaagugcaccagggacgagugcgacaccuauuucaaggugugccugaaggaauaccagagccgcgucacggccgggggcccgugcuccuucggcaguggcuccacccccgugaucggcggcaacaccuuuaaccugaaggccucccgggguaacgacaggaacaggaucgugcugcccuucuccuucgccuggccgagguccuacacccuccugguagaggccugggacagcagcaaugauacggugcagcccgacuccaucauagaaaaggccagccacuccgggaugaucaauccgagcaggcaguggcaaacccucaagcagaacaccgguguggcccacuuugaguaccagaucagggucaccugcgacgacuacuacuacggcuucggcugcaacaaguuuugcaggccgagggacgacuucuucggccacuacgccugcgaccagaauggcaacaagaccugcauggaaggcuggaugggcccggaaugcaaucgcgccaucuguaggcaggggugcagcccaaagcaugggagcugcaagcugcccggggacugcaggugucaguacggauggcaggggcuguacugugacaaguguaucccacauccgggcugcgugcacggaauaugcaacgagcccuggcagugccugugugaaacgaacuggggcggucagcugugcgacaaggaccugaacuacugcggcacccaccagcccugccugaacggcgggacguguuccaacaccggccccgacaaguaucaguguagcugccccgagggcuauagcggcccgaacugcgagaucgccgaacaugccugucucagcgaccccugucacaacagggguagcuguaaggaaaccagccucggguuugagugugaaugcuccccgggcuggaccgggcccaccuguuccaccaacaucgacgacugcucccccaauaacugcagccauggcggcacgugucaggaccucgucaauggcuuuaagugugugugccccccgcaguggaccggcaagacgugccagcuggacgccaacgagugugaggccaagcccugcgucaacgcaaagagcugcaagaaccugaucgccuccuacuauugugacugccugcccggguggaugggacagaacugcgacaucaauaucaacgauugccuggggcagugccagaacgacgcgagcugcagggaccuggucaacggcuaccgaugcaucugccccccgggcuacgccggcgaccacugugaaagggacaucgacgagugcgccagcaaccccugccugaacgggggccacugccagaacgagaucaauagguuccagugccugugcccgaccgguuuuagcggcaaccugugccagcuggacauugacuauugcgagcccaaccccugccagaacggggcccagugcuacaacagggccucggacuacuucuguaagugccccgaggacuaugagggcaagaacugcagccaucugaaggaccacugcaggaccaccccgugcgaggucaucgacagcugcaccguggccauggccuccaaugauacccccgagggcgugagguacaucuccuccaacguguguggcccccacggcaagugcaaaagccagagcggcggcaaguucaccugugacuguaacaagggcuucaccggcaccuacugccaugaaaacaucaacgauugcgagucuaaucccugccggaacggcggcaccugcaucgauggcgugaacagcuauaaauguaucugcuccgaugggugggagggcgcauacugcgaaaccaacaucaacgacugcucccagaaccccugccauaacggcggcaccugccgcgaccucgucaacgauuucuacugcgacugcaagaacggcuggaagggcaagaccugccacagccgagacagccagugcgacgaggccacgugcaacaacggagggaccuguuaugacgagggcgacgccuucaagugcaugugccccgggggcugggagggcacgaccugcaacauugcccgcaauagcagcugcuugcccaaccccugucacaacggcggaaccugcgucgugaacggcgaguccuucaccugcguuugcaaagagggcugggagggcccaaucugugcccagaacaccaaugacugcagcccccaccccugcuacaauuccgguaccugcguggacggcgacaacugguauaggugcgagugcgccccgggauucgccggcccggacugcaggaucaacaucaacgagugccagagcagccccugcgccuucggggccaccuguguggacgagaucaauggcuacaggugugucugcccccccggacacucgggcgcgaaaugccaagagguguccggcaggcccugcaucaccauggguuccgugauacccgacggggcaaagugggacgacgauugcaauaccugccaaugccugaacggcaggaucgccuguagcaaggugugguguggcccgaggccuugccuccugcauaaaggccacagcgagugucccuccggccagagcuguauccccauccucgacgaucaaugcuuugugcacccuugcaccggggugggcgagugucgcagcagcagccugcagcccgugaagaccaaaugcaccagcgauagcuacuaccaggacaacugcgcgaauaucaccuuuacguucaacaaggagaugaugagcccgggccugaccacagagcacaucugcagcgagcugcgcaaccugaacauccugaagaacgugucugccgaguauagcaucuacaucgccugcgaacccagccccuccgcaaauaaugagauccacguggcgaucucggccgaggacaucagggacgacgggaaccccaucaaagagaucaccgacaagaucaucgaucuggugagcaagcgggacggcaacagcucccucaucgccgccguggcugagguccgagugcagcggcguccccuuaagaacaggaccgacuuccuggugccccuccugucguccgugcucaccguggccuggaucuguugccuggugaccgccuucuacuggugccugcguaagcgaaggaagcccggaucccacacccacagcgccagcgaagacaacaccaccaauaacguccgagagcagcugaaccagaucaagaaccccauagagaaacacggggccaacaccgugccuaucaaggacuacgagaacaaaaauagcaaaaugagcaagauuaggacccacaacuccgagguggaggaggacgacauggacaagcaucagcagaaggcccgcuucgccaagcaacccgccuacacccugguggaccgagaggaaaagccccccaacgggacccccacgaagcaccccaacuggaccaauaagcaggauaacagggaccucgagagcgcccagucccugaaucgcauggaguacaucgug

SEQ ID NO: 107 - RNA, 3654 nt, Artificial Sequence
  Synthetic polynucleotide
augaggagcccccgcaccagggggcguagcggccgcccccugagccugcugcuggcucugcugugugcccugcgagccaaagugugcggggccuccggccaguucgagcuggagauccugagcaugcagaacgugaacggcgagcuccagaacggcaacugcugcggcggcgcccgcaaccccggcgacaggaagugcacucgggacgagugcgacaccuauuucaaggucugccugaaggaguaccaaagccgugugaccgccggcgggccgugcagcuucggaagcggcuccaccccggucaucggggggaacaccuuuaaccugaaggccagccgggguaacgacaggaaccgaaucguacugcccuucagcuucgccuggccccggagcuacacccugcuggucgaggcaugggacuccagcaacgauaccgugcagcccgacagcaucaucgagaaagccagccacagcgggaugauuaaucccagcagacaguggcagacccugaagcagaacaccggcguggcccacuucgaguaccaaauccgggugaccugcgacgauuauuacuacggguuuggcuguaauaaauucugccggccccgggaugacuuuuucggccauuacgccugcgaucagaacgguaacaagaccugcauggagggcuggaugggaccggaguguaacagggcuaucugccgacaggguuguagccccaagcacggaagcugcaagcugcccggcgacugccggugucaguacggcuggcagggccuguacugcgauaagugcaucccccaccccggcugcguucacggcaucugcaacgagcccuggcagugccugugugaaaccaacugggguggacagcugugcgacaaggaucugaacuauugcggcacccaccagcccugccugaacggcggaaccugcagcaacaccggccccgauaaguaccagugcagcugccccgaaggcuacuccggccccaacugcgagaucgccgagcacgccugccugagcgacccgugccacaacagggggagcugcaaagagaccagccuggguuucgagugcgagugcagccccggcuggaccgggcccacuugcuccaccaacauugacgacuguagcccgaacaauugcagccacggcggcaccugccaggaccuggugaauggcuucaagugcgugugucccccccaguggaccgggaagaccugccagcuggacgccaacgagugcgaggccaagcccugugugaacgccaaguccugcaagaaccugaucgccuccuacuacugugacugucuccccggguggaugggccagaacugcgacaucaacaucaacgauugccucggccagugccagaacgacgccagcuguagggaccucgugaacggcuaccggugcaucugcccgcccggguacgccggagaccacugcgagagggacauugacgagugcgccucgaaccccugccugaacggcggccacugucagaacgagaucaauagguuccagugucugugucccaccggcuucuccggcaaccugugucagcuggacaucgacuacugugagcccaaucccugccagaauggcgcccagugcuauaaccgggccuccgacuacuuuugcaagugccccgaagauuacgagggcaagaacugcagccaucugaaggaccacugcaggacgacucccugcgaggugaucgacagcuguacugucgccauggccagcaacgacacccccgaggggguccgcuauaucagcagcaacgugugcgggccccaugggaaaugcaaaucccagucagggggcaaguuuaccugcgacuguaacaaaggcuucaccggcaccuacugccacgaaaacaucaacgacugcgaaucgaaccccugccggaacggcgggaccugcaucgauggagugaacagcuacaagugcaucugcagcgacgggugggagggcgcguacugcgaaaccaauaucaaugacugcagccagaaccccugccauaacggaggcaccugcagggaccuggugaacgacuucuacugcgauugcaagaacggcuggaaggggaagaccugccauagcagggacagccagugugacgaggccaccugcaacaacggcggcacauguuacgaugagggcgacgccuucaaaugcaugugccccggcggcugggagggcaccacaugcaacaucgcccggaacagcagcugccuccccaaccccugccauaauggcgguaccugcguggugaacggcgagaguuucaccugcgugugcaaggagggcugggagggccccaucugcgcgcagaacaccaaugacugcucgccccaccccugcuacaacagcggcaccugcguggacggugacaacugguaccguugcgagugcgccccaggcuucgccggcccggacugcaggaucaacaucaacgagugccaaagcuccccuugcgccuuuggcgcaaccuguguggacgagaucaauggguacaggugcgugugcccccccggccauuccggggccaagugccaagagguguccggccggcccugcauuaccaugggcagcguuauccccgacggcgccaagugggacgacgacugcaauaccugccagugccucaacggcaggaucgccugcagcaagguguggugcggacccaggccgugccugcugcauaagggccacagcgagugcccgagcggucaguccugcauccccauccucgacgaccaguguuucgugcaccccugcacgggcgugggugagugccgauccuccagccugcagcccgucaaaaccaagugcaccuccgacagcuacuaccaggacaacugcgccaacauaaccuucacguuuaacaaggagaugaugagccccggccugaccaccgagcacaucugcagcgagcugaggaaccugaacauccugaagaacguguccgccgaguacagcaucuacaucgccugugagcccagccccuccgccaacaacgagauccauguugccaucucggccgaagauauuagggacgacggcaaccccaucaaggagaucaccgacaagaucauagaccuggugagcaagcgggacggcaauuccagccugaucgccgccguggccgaggugagagugcagaggaggccccugaagaaccggaccgauuuccuggugccccugcugagcagcgugcugaccguggccuggaucugcugccuggugaccgcauuuuacuggugucugaggaagcggaggaaacccggcagccacacccacagcgcaagcgaggauaacaccacgaauaacgugcgcgagcagcugaaccaaaucaagaaccccaucgagaagcacggggccaacaccgugcccaucaaggacuacgagaauaagaacucgaagaugagcaagaucaggacgcacaacuccgagguggaggaggacgacauggauaagcaccagcagaaagcccgguucgccaagcagcccgccuacacccugguugaccgcgaggagaaaccccccaacggcacccccaccaagcaccccaacuggaccaacaagcaggacaaccgagaccuggagagcgcccagagccugaacaggauggaguauaucgug

SEQ ID NO: 108 - RNA, 3654 nt, Artificial Sequence
  Synthetic polynucleotide
augaggucccccaggaccaggggcaggagcgggaggccccugucccuucugcuggcgcugcugugcgcccugcgcgccaaggugugcggggcaagcggccaguucgagcucgaaauacucagcaugcaaaacgucaacggcgagcugcagaacggcaacuguugcgguggcgccaggaaccccggggaucgcaagugcaccagggacgagugugauaccuacuucaaagugugucugaaggaguaccagagccgggugaccgccgggggccccuguuccuucggcagcgggagcacccccgucaucggcgggaauacguuuaaccugaaggccuccaggggcaacgauaggaaccggaucgugcucccuuucagcuucgccuggcccagguccuacacccugcugguggaggccugggacuccagcaaugacacuguccagccugacaguaucauagagaaagccucccacuccggcaugaucaaccccagucgccaguggcagacccugaagcagaacaccggcguggcccacuucgaguaccagauccgggugaccugcgacgacuauuacuacggcuucggaugcaauaaguucuguaggccccgcgacgauuucuucggccauuaugccugcgaccagaacggcaacaagaccugcauggagggcuggauggggcccgagugcaacagggccaucugcaggcaggggugcucccccaaacacgggagcugcaaacugccgggggacugcaggugccaauacggcuggcagggccuguacugcgacaagugcaucccgcaccccgggugcgugcacggcauuugcaacgaacccuggcagugccucugcgaaaccaauuggggaggccagcugugcgacaaggaucugaacuacugcggcacgcaccagcccugccucaacggggggaccuguagcaacacgggccccgacaaguaccagugcuccugcccggagggauacucuggccccaacugcgagaucgccgagcacgccugccucuccgauccgugccacaauaggggcagcugcaaggaaacgucccugggcuucgaaugcgaaugcagucccggauggaccggccccaccugcagcaccaacaucgacgacugcagccccaacaacugcagccacggcggcaccugccaagaucucgugaacggcuucaagugcgugugccccccccaguggaccgggaaaaccugccaacucgacgccaaugagugugaggccaagcccugcgugaacgccaagucgugcaaaaaccugaucgccagcuacuacugcgacugccugcccggcuggauggggcagaacugcgacaucaacaucaacgacugccuggggcagugccagaaugacgcuagcugccgagaccuggucaauggauaccggugcauaugccccccgggcuacgccggcgaccauugcgagcgggacaucgacgagugcgccagcaacccaugccugaacggcgggcacugccagaacgaaauaaacagguuccagugucugugcccgacgggcuuuagcggcaaccucugccaguuggauaucgacuauugcgagccuaacccuugccagaacggcgcccagugcuauaaccgcgcaagcgauuauuucugcaaaugccccgaggacuacgagggcaagaauugcagccaucugaaagaccacugucggacgacccccugcgaggugaucgacagcugcaccguggccauggccuccaacgacacccccgaaggggugcgcuauaucuccagcaacgugugcggcccccacggcaagugcaagagccagucagggggcaaauucaccugcgacugcaacaagggcuucaccgggaccuacugccacgagaacaucaacgacugcgagagcaaccccugccggaacggcggcaccugcaucgauggggugaacuccuauaagugcaucuguagcgauggaugggagggggccuacugcgaaaccaacaucaacgacugcagccagaaccccugccacaacgggggcaccugcagggaccucgugaacgacuucuacugcgacugcaagaacggcuggaagggcaagacaugccacucccgggacucacaaugcgacgaagcgaccugcaacaauggcggcaccuguuacgaugagggggaugccuuuaagugcaugugccccgguggcugggagggcaccaccugcaauaucgccaggaauuccuccugccugcccaaccccugccauaauggcgggaccugcgucgugaacggcgagagcuucaccugcgugugcaaagaggggugggaaggacccaucugcgcccaaaauacgaacgacugcagcccccaccccuguuacaacagcggcacgugcguggauggggacaacugguaccgcugcgagugcgcccccggcuuugcaggcccggacugucggaucaacaucaacgagugccagagcagccccugcgccuucggagccacgugcguggacgagaucaauggcuacagaugcgugugccccccgggacacagcggcgccaagugccaggaaguguccggccgucccugcaucaccauggguagcgucauccccgacggcgccaagugggacgaugacugcaacacgugucagugucugaacggccgaaucgccugcuccaagguguggugcggcccccggcccugccugcugcacaagggccacagcgagugccccagcggccagucguguauccccauccucgacgaccaaugcuucgugcaccccugcaccggcgugggcgagugccgcagcucgagccugcagcccgugaagaccaagugcaccagcgauagcuacuaccaggacaauugcgccaacaucaccuucaccuuuaacaaggagaugaugagccccggccugacgaccgaacacaucugcuccgagcugaggaaccugaacauccugaagaaugucagcgcugaguacuccaucuacaucgccugugagcccagcccaagcgccaacaaugagauccacgucgcgaucuccgccgaggacauccgcgacgauggcaaccccaucaaggagaucaccgacaagaucaucgaccuggugagcaagagggacggcaacagcucccugaucgccgcgguggccgaggugaggguccaaaggaggccccugaagaacaggaccgacuuccuggugccccugcugucgagcgugcugaccguggccuggaucugcugccuggugaccgcguucuacuggugccugcguaagaggaggaagcccggcagccacacccauagcgcguccgaggauaacaccaccaauaacgugagggagcagcucaaccagaucaagaacccaaucgagaagcacggugccaacacugugcccaucaaggacuaugagaacaagaacagcaagaugaguaagaucaggacacacaacuccgagguggaagaagacgacauggacaagcaccagcagaaggcccgguucgccaagcagcccgccuacacccugguggacagggaagagaaaccccccaacgguacacccacgaaacaccccaacuggaccaauaagcaggacaacagggaccuggaguccgcccagagucugaacaggauggaguacaucgug

SEQ ID NO: 109 - RNA, 3654 nt, Artificial Sequence
  Synthetic polynucleotide
augcgguccccccggaccagggguaggagcggccgcccacugucccugcugcuggcccugcugugugcccugagggccaaggugugcggcgccuccggacaauucgagcuggagauucucucgaugcagaacgugaacggcgaacugcagaacggaaauugcuguggcggcgccaggaaucccggcgauagaaagugcaccagggacgagugugacacguacuucaaggugugccugaaggaguaccagagccgcgugaccgccggcgggcccugcuccuucgggucaggcagcacccccgugaucggcgggaacaccuucaaccucaaggccuccaggggcaacgacaggaauaggaucgugcuccccuucagcuucgccuggcccagguccuacacccugcugguagaggccugggacuccagcaacgacaccgugcagcccgauagcaucaucgagaaggcuagccacagcggaaugaucaaccccagccgccaguggcagacccugaaacagaacaccggcguagcccacuuugaguaccagaucagggugaccugcgacgacuauuacuauggcuucgguugcaacaaguucugccggccucgcgacgacuucuucggacacuacgccugugaucagaacgggaacaagaccuguauggaggguuggaugggccccgaaugcaacagggccaucugcaggcagggcugcucccccaagcacgggagcugcaagcugcccggcgacugccggugccaguacggcuggcagggucuguacugcgacaagugcaucccccauccuggcugcgugcacggcauaugcaacgagcccuggcagugccugugcgagaccaauuggggcggccagcugugcgacaaggaccugaauuacuguggcacccaccagcccugccucaacggcggcaccugcuccaacaccggccccgacaaguaccagugcagcugccccgaaggcuacagcggcccgaauugcgagaucgccgaacacgccugccucagcgaccccugccacaaccggggcagcuguaaggagaccucccugggcuuugaaugcgaauguagccccgguuggaccggacccaccuguuccaccaacaucgacgacugcagccccaauaacugcagccacgguggcacgugccaggaccucgucaacggcuuuaagugcgugugccccccccaguggaccgggaagaccugccagcuggacgccaacgagugcgaggccaagcccugcgugaacgccaagagcugcaagaaccucaucgccagcuacuauugugacugccugcccggguggaugggccagaacugugacauaaacaucaacgauugucugggccagugccagaacgaugccagcugucgggaccuggugaacggcuaccggugcaucuguccccccggcuacgccggagaucacugugagcgagacaucgacgagugcgccuccaaccccugccucaacggcgggcacugucagaaugagaucaacagguuccagugccugugcccgacgggauucuccgguaaccugugccagcucgacaucgacuacugugagcccaaccccugucaaaauggcgcccaaugcuacaaccgggccuccgacuacuucuguaagugccccgaggauuacgaggguaagaacuguagccaucugaaggaccacugcaggacuaccccgugcgaggugaucgacuccugcaccgucgccauggccuccaacgacacccccgagggcgugcgguacaucagcagcaacgugugugggccgcacggcaagugcaagagccagagcgggggcaaguucaccugugauugcaacaagggcuucaccgggacguauugccacgagaacaucaacgacugcgagagcaaccccugcaggaacggggggaccugcauagacggcgugaacagcuacaaaugcaucugcagcgaugggugggagggcgccuacugugagaccaacauuaacgacugcagccagaaccccugccacaacggggguaccugucgcgaccuggugaacgacuucuacugugacugcaagaacggcuggaagggcaagaccugucauucccgcgacagccagugcgacgaagccaccugcaacaacggcggcaccugcuacgacgagggcgaugccuucaagugcaugugcccgggcggcugggaggggaccaccuguaauaucgccaggaauuccagcugccuccccaauccgugccauaauggcggcaccugcguggucaacggcgaaagcuuuaccugcgucuguaaggaaggcugggaagguccgaucugugcccagaacaccaacgacuguagcccccaccccugcuacaauagcggaacgugcguggacggcgacaacugguaucggugcgagugcgcccccggcuuugcggggccggacugccggaucaauaucaacgagugccagagcagccccugcgccuucggcgccaccugcguggacgagaucaacggcuacaggugcguguguccccccggccacuccggcgccaagugccaggaggugagcgguaggcccugcaucaccaugggcagcgugauccccgacggggccaagugggacgaugacuguaacaccugccagugccugaacgggaggaucgccuguuccaaaguguggugcggcccgcgucccugccuacuccacaaggggcauuccgagugucccagcggacagagcuguauccccauccuggacgaccaaugcuucgugcaccccugcaccggcgugggugagugcagguccagcagccugcagcccgugaagacaaagugcaccagugauuccuacuaccaggauaacugcgccaacaucaccuucaccuucaauaaggagaugaugagcccgggccugaccacggagcacaucugcagcgagcugcgcaaccugaacauccugaagaacgucuccgccgaguacagcauauacaucgccugcgagcccagccccuccgccaauaacgagauccacguggccaucuccgcggaggacaucagggacgauggcaaccccaucaaggagaucaccgacaagauuaucgaccuggucagcaaaagggacggcaacuccagccucaucgccgccguggccgaggucaggguacagcgcaggccgcugaaaaaccggaccgacuuccuggugccccugcuuuccuccgugcucacgguggccuggauuugcugccugguaaccgcguuuuacuggugccugaggaagaggaggaagcccggcagccauacccacagcgccagcgaggacaacacaaccaacaacgugagggagcagcucaaccagauaaagaaccccaucgagaaacacggcgccaacacggugcccaucaaggacuaugagaacaagaacagcaagaugagcaagauccgcacccacaacagcgagguugaggaagacgacauggacaagcaccagcagaaggccagguucgccaagcagcccgccuacacccugguggaucgugaggagaaaccgcccaacgggacccccaccaagcaucccaauuggaccaacaaacaggacaacagggaccuggaguccgcccaaagccugaaccggauggaguacaucguc

SEQ ID NO: 110 - RNA, 3654 nt, Artificial Sequence
  Synthetic polynucleotide
augaggucccccagaacucgggggagguccggcaggccgcucagccuccugcucgcccugcugugcgcccugagggccaaggugugcggcgccuccggccaguucgagcuggagauucugagcaugcagaacgugaacggcgaacugcagaacggaaacugcugcgguggggccaggaaccccggcgaccggaagugcaccagggaugaaugcgacaccuacuucaaggucugccucaaggaguaccagagcagggugaccgccgggggcccguguagcuucggcuccggcagcacccccgugauaggcggcaacacguucaaccuuaaagccuccaggggcaacgaccgcaacaggaucgugcugcccuucuccuucgcguggccccgcagcuacacccugcugguggaggcgugggauagcagcaacgacaccguccagcccgauucaaucaucgaaaaggccagccacagcggcaugaucaaccccuccaggcaguggcagacccugaagcaaaacaccggcguggcccacuucgaguaccaaaucaggguuaccugcgacgacuacuacuauggguucggcugcaauaaguucugucggccgcgggacgacuuuuucgggcauuaugccugcgaccagaauggcaauaagaccugcauggagggcuggaugggacccgagugcaaccgcgccaucugcaggcagggcugcucccccaagcacggcagcugcaagcugcccggcgacugcaggugccaguacggguggcagggccucuacugcgacaagugcaucccccaccccggcugcgugcaugggauaugcaacgagccguggcagugccugugcgaaaccaacugggggggccagcugugcgauaaggaccucaacuacugcggcacccaccagcccugccucaacggcggcaccugcuccaauaccgggcccgauaaauaccagugcuccugcccugagggcuacagcgggcccaacugugagaucgccgagcaugccugccucucggaccccugccauaacaggggcagcuguaaggaaaccagccugggcuucgagugcgagugcagccccggguggaccgggccaaccugcuccaccaacaucgacgacuguagcccgaacaacugcucccacggcgggaccugccaggaccuggugaauggcuucaagugcguaugucccccacaguggaccggcaagaccugucaacucgacgccaacgagugcgaggccaaacccugcgugaacgccaaguccugcaagaaccugaucgccuccuacuacugcgacugucugcccggcuggaugggccagaacugcgauaucaacaucaacgauugccucggccagugucagaacgacgccuccugccgggaccuggugaacggcuaccggugcauuugccccccgggcuacgccggcgaucacugcgagcgcgacaucgacgagugcgcauccaaccccugucugaacggggggcacugucagaacgagaucaauagguuccagugccugugccccaccggcuucuccgggaaucugugccagcuggacaucgauuacugcgagcccaaccccugccagaacggcgcccaguguuacaacagggccagcgauuacuucugcaagugucccgaagacuaugagggcaagaauugcagccaucugaaagaccacugccgcaccacccccugugaggugaucgacucgugcaccguggcgauggccagcaaugacaccccggagggcgugcgguacaucagcagcaacgugugugggccccacggcaagugcaagucccagagcgggggcaaguucaccugcgacugcaacaaaggcuuuacagggacauauugccacgaaaacaucaaugacugcgagagcaaccccugccgcaauggcggcacuugcaucgacggcgugaacagcuacaaauguaucugcucagacgggugggaaggcgcguauugcgagaccaacaucaacgauuguagccagaaucccugccauaacggugguaccugccgggaucuggugaacgacuucuauugcgacugcaagaacggcuggaagggcaagaccugccauucgagggauagccagugcgacgaggccaccugcaacaacggcggcaccugcuacgacgagggcgaugccuucaagugcaugugcccuggcggcugggagggcaccaccugcaacaucgccaggaacagcuccugccugcccaaccccugccacaacggcgggaccugugucgugaacggggagagcuucacgugcgugugcaaggagggcugggaagggcccaucugcgcccaaaacaccaacgacugcagcccccaucccuguuacaacuccggcaccugcguggacggcgacaacugguaccgaugcgagugcgcccccggcuucgccggccccgacugccggaucaacaucaacgagugccagagcagccccugcgcguucggcgccaccugcguggaugaaaucaacggauauaggugcgugugcccccccggccacagcggggccaagugccaggaggucagcgggcgccccugcaucaccaugggcagcgugauacccgacggcgccaagugggacgacgacugcaacaccugccagugccugaacggcaggaucgccugcuccaagguguggugcgggccgcggccgugccugcugcacaagggccacagcgagugccccagcggccaguccuguaucccaauccuggacgaccagugcuucgugcaucccugcaccggcgugggcgagugcagguccuccucccugcagcccgugaagaccaaaugcaccagcgacucguacuaccaggauaacugcgccaacaucaccuucaccuucaacaaggaaaugaugagccccggccugaccaccgagcacaucugcagcgagcuccggaaccugaacauccugaagaacguguccgccgaguauagcaucuacaucgcgugcgaaccaaguccguccgccaacaacgagauccacguggcaaucuccgccgaggacauccgggacgacggcaaccccaucaaggagauaaccgacaaaaucaucgaccuggugagcaaaagggacggcaauucuagccugaucgccgcaguggccgaagugagggugcagcgcaggccccucaagaauaggaccgacuuccuggugccgcuccucagcagcgugcugaccguggccuggaucugcugccuggugaccgccuuuuacuggugccugaggaagcguaggaagcccggaagccacacacacuccgccagcgaggacaacaccaccaacaacgugcgggagcaacugaaccagaucaagaaccccaucgagaagcacggagccaacaccgucccuaucaaagacuacgagaacaagaacagcaagaugagcaagaucaggacccacaacagcgagguugaggaagacgacauggacaagcaccagcagaaagccagguucgcgaagcagcccgccuacacccugguggaccgggaggaaaagccccccaacggcacccccaccaagcacccgaacuggaccaacaagcaggacaacagggaccuggagagcgcccagagccugaaccggauggaguacaucguc

SEQ ID NO: 111 - RNA, 3654 nt, Artificial Sequence
  Synthetic polynucleotide
augcgcagcccccggaccaggggaagguccggcaggccccugucccugcugcuggcgcugcucugcgcccugcgagccaaaguguguggugccuccgggcaguuugagcuggagauccucagcaugcagaacgugaacggggagcugcagaaugggaacugcugcggcggcgccaggaaucccggggacaggaagugcacccgagaugagugcgacaccuauuucaaggugugccugaaggaguaccagagccgugugacggccggcggccccugcagcuuuggcagcggcagcacccccgugaucggcggaaacacauucaaccugaaggccagcaggggcaacgacaggaacaggaucgugcugcccuucagcuucgccuggcccagguccuacacccugcugguggaggccugggauagcagcaaugacaccgugcagcccgacuccaucaucgagaaggccagucacucuggaaugaucaacccgagcaggcaguggcagacccugaagcagaacaccggcguggcccacuucgaguaccagaucagggugaccugugacgauuacuacuacgguuuuggcugcaacaaguucuguaggccccgcgacgacuucuuuggucauuacgccugcgaucagaacggcaauaagaccugcauggaaggcuggaugggccccgaaugcaacagggccauuugcaggcaggggugcagcccgaagcacggcagcugcaagcugcccggcgacugcaggugucaguacggcuggcagggccuguacugcgacaaaugcaucccccacccugggugcgugcacggcaucuguaacgagcccuggcagugccugugugagaccaacuggggugggcaacugugcgauaaggaccugaacuacugcggaacccaccagcccugccugaacggcggcacaugcagcaacaccgggcccgacaaguaccagugcagcugccccgaaggguauagcgggcccaauugcgaaaucgccgagcacgccugccugagcgaucccugucauaaucgcggauccugcaaggagaccagccucggcuuugagugcgaaugcucccccggcuggaccggucccacgugcagcacgaacaucgacgacuguuccccgaacaacugcucccacggcggcaccugccaggaucuggugaauggauucaaaugcgugugccccccccaauggaccgggaagaccugccaacuggacgccaacgagugcgaagccaagcccugugugaacgccaagagcugcaaaaaccucaucgcuagcuacuacugcgacugccugcccggcuggaugggucagaacugugacaucaacaucaacgauugucugggccagugccagaacgacgccagcugcagggaccuggugaauggguaccgcugcaucugcccccccggcuacgccggagaucauugcgagcgggacaucgacgagugcgccagcaaccccugccugaacggcggucacugucagaaugagaucaaccgcuuccagugccugugccccaccggcuucagcggaaaucugugccagcuagacauugauuacugcgaaccgaacccuugccagaacggcgcccagugcuacaacagggccagcgacuacuuuugcaagugccccgaggacuacgaggggaagaauugcucccaccuaaaggaccacugccggaccacccccugcgaggugaucgacagcugcaccgucgcgauggccagcaacgacacccccgagggcgucagguacaucuccagcaacgugugcgguccccauggcaaaugcaagagccagagcggggggaaguuuaccugcgacugcaacaagggcuucaccgggaccuacugccaugagaacaucaaugacugcgagagcaaccccugcaggaacggcgggacaugcaucgacggggugaacuccuauaagugcaucugcuccgacgggugggaaggugccuauugcgagacaaacaucaacgacugcagccaaaaccccugccacaacgggggcaccugcagggaucuggugaacgacuucuacugugacugcaagaacggguggaagggaaagaccugucacagccgggacucccagugcgacgaggccacaugcaacaacggcggcacgugcuacgacgaaggagacgccuuuaagugcaugugccccggcggcugggagggcaccaccugcaauaucgcccgcaacuccuccugccugcccaacccgugccacaacgggggcaccugcguggugaacggcgaguccuucaccugcgucugcaaggagggcugggagggucccaucugugcccagaauaccaaugacugcagcccccauccuuguuacaauuccggcaccugcguggauggcgacaacugguaucggugugagugcgcccccggcuucgcgggccccgacuguaggaucaacaucaacgagugccagagcuccccaugcgcguuuggggcgaccugugucgacgagaucaauggguacaggugcgugugucccccggggcacuccggggccaaaugccaggagguaagcggccggccaugcauuaccaugggcucggugaucccagacggugccaagugggacgacgacugcaacaccugccagugccugaauggcaggaucgccugcagcaagguauggugcggacccaggccgugccugcugcacaaaggacacuccgaguguccgagcggccagagcugcauccccauccuggacgaccagugcuucgugcaucccugcacuggcgucggcgagugccgcagcuccagccugcagcccgugaagaccaaguguaccagcgacagcuacuaccaggacaauugugccaacaucaccuucaccuucaacaaggagaugaugagcccuggccugaccaccgagcauaucuguagcgagcugaggaacuugaacauccugaagaaugugagcgccgaguauuccauuuacauagccugugagcccagcccaagcgcuaacaaugagauccacguggccaucagcgccgaggacauccgggacgacggcaaccccaucaaagaaaucaccgacaagaucaucgaucugguaagcaagagggacgggaacagcagccucaucgccgccguggccgaggugcgcguccagcggaggccccucaaaaaccggaccgacuuucuggugccgcugcucagcuccgugcugaccguggccuggauaugcugccuggugaccgccuucuacuggugccugcggaagaggaggaagcccggcagccacacgcacagcgcgagcgaggacaacaccaccaacaacgugcgggagcaacugaaccagaucaagaaccccaucgagaagcacggcgccaacaccgugcccaucaaggacuacgagaacaagaauagcaagaugaguaagauuaggacccacaacagcgagguggaggaggacgacauggacaagcaccagcagaaggcccgcuucgccaagcagcccgccuauacccuggucgacagggaagagaagccgcccaaugggacccccaccaagcaucccaacuggaccaacaagcaggacaaccgggaucuggagagcgcccaaagccugaauaggauggaguacaucgug

SEQ ID NO: 112 - RNA, 142 nt, Artificial Sequence
  Synthetic polynucleotide
ugauaauaggcuggagccucgguggccuagcuucuugccccuugggccuccccccagccccuccuccccuuccugcacccguacccccuccauaaaguaggaaacacuacaguggucuuugaauaaagucugagugggcggc

SEQ ID NO: 113 - RNA, 141 nt, Artificial Sequence
  Synthetic polynucleotide
ugauaauaggcuggagccucgguggccuagcuucuugccccuugggccuccccccagccccuccuccccuuccugcacccguaccccccgcauuauuacucacgguacgaguggucuuugaauaaagucugagugggcggc

SEQ ID NO: 114 - RNA, 164 nt, Artificial Sequence
  Synthetic polynucleotide
ugauaauaguccauaaaguaggaaacacuacagcuggagccucgguggccuagcuucuugccccuugggccuccccccagccccuccuccccuuccugcacccguaccccccgcauuauuacucacgguacgaguggucuuugaauaaagucugagugggcggc

SEQ ID NO: 115 - RNA, 188 nt, Artificial Sequence
  Synthetic polynucleotide
ugauaauaguccauaaaguaggaaacacuacagcuggagccucgguggccuagcuucuugccccuugggccuccauaaaguaggaaacacuacauccccccagccccuccuccccuuccugcacccguacccccuccauaaaguaggaaacacuacaguggucuuugaauaaagucugagugggcggc

SEQ ID NO: 116 - RNA, 140 nt, Artificial Sequence
  Synthetic polynucleotide
ugauaauaggcuggagccucgguggccaugcuucuugccccuugggccuccccccagccccuccuccccuuccugcacccguacccccaguagugcuuucuacuuuaugguggucuuugaauaaagucugagugggcggc

SEQ ID NO: 117 - RNA, 181 nt, Artificial Sequence
  Synthetic polynucleotide
ugauaauagaguagugcuuucuacuuuauggcuggagccucgguggccaugcuucuugccccuugggccaguagugcuuucuacuuuauguccccccagccccucuccccuuccugcacccguacccccaguagugcuuucuacuuuaugguggucuuugaauaaagucugagugggcggc

SEQ ID NO: 118 - RNA, 184 nt, Artificial Sequence
  Synthetic polynucleotide
ugauaauagaguagugcuuucuacuuuauggcuggagccucgguggccaugcuucuugccccuugggccuccauaaaguaggaaacacuacauccccccagccccuccuccccuuccugcacccguacccccaguagugcuuucuacuuuaugguggucuuugaauaaagucugagugggcggc

SEQ ID NO: 119 - RNA, 142 nt, Artificial Sequence
  Synthetic polynucleotide
ugauaauaguccauaaaguaggaaacacuacagcuggagccucgguggccuagcuucuugccccuugggccuccccccagccccuccuccccuuccugcacccguacccccguggucuuugaauaaagucugagugggcggc

SEQ ID NO: 120 - RNA, 142 nt, Artificial Sequence
  Synthetic polynucleotide
ugauaauaggcuggagccucgguggcuccauaaaguaggaaacacuacacuagcuucuugccccuugggccuccccccagccccuccuccccuuccugcacccguacccccguggucuuugaauaaagucugagugggcggc

SEQ ID NO: 121 - RNA, 142 nt, Artificial Sequence
  Synthetic polynucleotide
ugauaauaggcuggagccucgguggccuagcuucuugccccuugggccuccauaaaguaggaaacacuacauccccccagccccuccuccccuuccugcacccguacccccguggucuuugaauaaagucugagugggcggc

SEQ ID NO: 122 - RNA, 142 nt, Artificial Sequence
  Synthetic polynucleotide
ugauaauaggcuggagccucgguggccuagcuucuugccccuugggccuccccccagccccuccuccccuuccugcacccguacccccaccccuaucacaauuagcauuaaguggucuuugaauaaagucugagugggcggc

SEQ ID NO: 123 - RNA, 188 nt, Artificial Sequence
  Synthetic polynucleotide
ugauaauagaccccuaucacaauuagcauuaagcuggagccucgguggccuagcuucuugccccuugggccaccccuaucacaauuagcauuaauccccccagccccuccuccccuuccugcacccguacccccaccccuaucacaauuagcauuaaguggucuuugaauaaagucugagugggcggc

SEQ ID NO: 124 - RNA, 188 nt, Artificial Sequence
  Synthetic polynucleotide
ugauaauagaccccuaucacaauuagcauuaagcuggagccucgguggccuagcuucuugccccuugggccuccauaaaguaggaaacacuacauccccccagccccuccuccccuuccugcacccguacccccaccccuaucacaauuagcauuaaguggucuuugaauaaagucugagugggcggc

SEQ ID NO: 125 - RNA, 3678 nt, Artificial Sequence
  Synthetic polynucleotide
augcguuccccacggacgcgcggccgguccgggcgcccccuaagccuccugcucgcccugcucugugcccugcgagccaagguguguggggccucgggucaguucgaguuggagauccuguccaugcagaacgugaacggggagcugcagaacgggaacugcugcggcggcgcccggaacccgggagaccgcaagugcacccgcgacgagugugacacauacuucaaagugugccucaaggaguaucagucccgcgucacggccggggggcccugcagcuucggcucaggguccacgccugucaucgggggcaacaccuucaaccucaaggccagccgcggcaacgaccgcaaccgcaucgugcugccuuucaguuucgccuggccgagguccuauacguugcuuguggaggcgugggauuccaguaaugacaccguucaaccugacaguauuauugaaaaggcuucucacucgggcaugaucaaccccagccggcaguggcagacgcugaagcagaacacgggcguugcccacuuugaguaucagauccgcgugaccugugaugacuacuacuauggcuuuggcugcaauaaguucugccgccccagagaugacuucuuuggacacuaugccugugaccagaauggcaacaaaacuugcauggaaggcuggaugggccccgaauguaacagagcuauuugccgacaaggcugcaguccuaagcaugggucuugcaaacucccaggugacugcaggugccaguacggcuggcaaggccuguacugugauaagugcaucccacacccgggaugcguccacggcaucuguaaugagcccuggcagugccucugugagaccaacuggggcggccagcucugugacaaagaucucaauuacugugggacucaucagccgugucucaacgggggaacuuguagcaacacaggcccugacaaauaucaguguuccugcccugagggguauucaggacccaacugugaaauugcugagcacgccugccucucugaucccugucacaacagaggcagcuguaaggagaccucccugggcuuugagugugaguguuccccaggcuggaccggccccacaugcucuacaaacauugaugacuguucuccuaauaacuguucccacgggggcaccugccaggaccugguuaacggauuuaagugugugugccccccacaguggacugggaaaacgugccaguuagaugcaaaugaaugugaggccaaaccuuguguaaacgccaaauccuguaagaaucucauugccagcuacuacugcgacugucuucccggcuggaugggucagaauugugacauaaauauuaaugacugccuuggccagugucagaaugacgccuccugucgggauuugguuaaugguuaucgcuguaucuguccaccuggcuaugcaggcgaucacugugagagagacaucgaugaaugugccagcaaccccuguuugaaugggggucacugucagaaugaaaucaacagauuccagugucugugucccacugguuucucuggaaaccucugucagcuggacaucgauuauugugagccuaaucccugccagaacggugcccagugcuacaaccgugccagugacuauuucugcaagugccccgaggacuaugagggcaagaacugcucacaccugaaagaccacugccgcacgacccccugugaagugauugacagcugcacaguggccauggcuuccaacgacacaccugaaggggugcgguauauuuccuccaacgucugugguccucacgggaagugcaagagucagucgggaggcaaauucaccugugacuguaacaaaggcuucacgggaacauacugccaugaaaauauuaaugacugugagagcaacccuuguagaaacgguggcacuugcaucgauggugucaacuccuacaagugcaucuguagugacggcugggagggggccuacugugaaaccaauauuaaugacugcagccagaaccccugccacaaugggggcacgugucgcgaccuggucaaugacuucuacugugacuguaaaaauggguggaaaggaaagaccugccacucacgugacagucagugugaugaggccacgugcaacaacgguggcaccugcuaugaugagggggaugcuuuuaagugcauguguccuggcggcugggaaggaacaaccuguaacauagcccgaaacaguagcugccugcccaaccccugccauaaugggggcacauguguggucaacggcgaguccuuuacgugcgucugcaaggaaggcugggaggggcccaucugugcucagaauaccaaugacugcagcccucaucccuguuacaacagcggcaccuguguggauggagacaacugguaccggugcgaaugugccccggguuuugcugggcccgacugcagaauaaacaucaaugaaugccagucuucaccuugugccuuuggagcgaccuguguggaugagaucaauggcuaccggugugucugcccuccagggcacaguggugccaagugccaggaaguuucagggagaccuugcaucaccauggggagugugauaccagauggggccaaaugggaugaugacuguaauaccugccagugccugaauggacggaucgccugcucaaaggucugguguggcccucgaccuugccugcuccacaaagggcacagcgagugccccagcgggcagagcugcauccccauccuggacgaccagugcuucguccaccccugcacuggugugggcgagugucggucuuccagucuccagccggugaagacaaagugcaccucugacuccuauuaccaggauaacugugcgaacaucacauuuaccuuuaacaaggagaugaugucaccaggucuuacuacggagcacauuugcagugaauugaggaauuugaauauuuugaagaauguuuccgcugaauauucaaucuacaucgcuugcgagccuuccccuucagcgaacaaugaaauacauguggccauuucugcugaagauauacgggaugaugggaacccgaucaaggaaaucacugacaaaauaaucgaucuuguuaguaaacgugauggaaacagcucgcugauugcugccguugcagaaguaagaguucagaggcggccucugaagaacagaacagauuuccuuguucccuugcugagcucugucuuaacuguggcuuggaucuguugcuuggugacggccuucuacuggugccugcggaagcggcggaagccgggcagccacacacacucagccucugaggacaacaccaccaacaacgugcgggagcagcugaaccagaucaaaaaccccauugagaaacauggggccaacacgguccccaucaaggauuaugagaacaagaacuccaaaaugucuaaaauaaggacacacaauucugaaguagaagaggacgacauggacaaacaccagcagaaagcccgguuugccaagcagccggcguacacgcugguagacagagaagagaagccccccaacggcacgccgacaaaacacccaaacuggacaaacaaacaggacaacagagacuuggaaagugcccagagcuuaaaccgaauggaguacaucguagacuacaaagacgaugacgacaag

SEQ ID NO: 126 - RNA, 3654 nt, Artificial Sequence
  Synthetic polynucleotide
augcgguccccacggacgcgcggccggcccgggcgcccccugagucuucugcucgcccugcucugugcccugcgagccaaggugugcggggccucgggucaguuugagcuggagauccuguccaugcagaacgugaauggagagcuacagaaugggaacuguugugguggaguccggaacccuggcgaccgcaagugcacccgcgacgagugugauacguacuucaaagugugccucaaggaguaucagucccgcgucacugccgggggacccugcagcuucggcucagggucuacgccugucaucggggguaacaccuucaaucucaaggccagccguggcaacgaccguaaucgcaucguacugccuuucaguuucgccuggccgagguccuacacuuugcugguggaggccugggauuccaguaaugacacuauucaaccugauagcauaauugaaaaggcuucucacucaggcaugauaaacccuagccggcaauggcagacacugaaacaaaacacagggauugcccacuucgaguaucagauccgagugaccugugaugaccacuacuauggcuuuggcugcaauaaguucugucgucccagagaugacuucuuuggacauuaugccugugaccagaacggcaacaaaacuugcauggaaggcuggauggguccugauugcaacaaagcuaucugccgacagggcugcagucccaagcaugggucuuguaaacuuccaggugacugcaggugccaguacgguuggcagggccuguacugcgacaagugcaucccgcacccaggauguguccacggcaccugcaaugaacccuggcagugccucugugagaccaacugggguggacagcucugugacaaagaucugaauuacugugggacucaucagcccugucucaaccggggaacauguagcaacacugggccugacaaauaccagugcuccugcccagagggcuacucgggccccaacugugaaauugcugagcaugcuugucucucugaccccugccauaaccgaggcagcugcaaggagaccuccucaggcuuugagugugaguguucuccaggcuggacuggccccacguguuccacaaacaucgaugacuguucuccaaauaacuguucccaugggggcaccugccaggaucuggugaauggauucaagugugugugcccgccccaguggacuggcaagacuugucaguuagaugcaaaugagugcgaggccaaaccuuguguaaaugccagauccuguaagaaucugauugccagcuacuacugugauugccuuccuggcuggaugggucagaacugugacauaaauaucaaugacugccuuggccagugucagaaugacgccuccugucgggauuugguuaaugguuaucgcuguaucuguccaccuggcuaugcaggcgaucacugugagagagacaucgaugagugugcuagcaaccccugcuugaaugggggucacugucagaaugaaaucaacagauuccagugucucugucccacugguuucucuggaaaccucugucagcuggacaucgauuacugcgagcccaacccuugccagaauggcgcccagugcuacaaucgugccagugacuauuucugcaagugccccgaggacuaugagggcaagaacugcucacaccugaaagaccacugccguaccaccaccugcgaagugauugacagcugcacuguggccauggccuccaacgacacgccugaaggggugcgguauaucucuucuaacgucugugguccccaugggaagugcaagagccagucgggaggcaaauucaccugugacuguaacaaaggcuucaccggcaccuacugccaugaaaauaucaacgacugcgagagcaaccccuguaaaaacgguggcaccugcaucgauggcguuaacuccuacaaguguaucuguagugacggcugggagggagcgcacugugagaacaacauaaaugacuguagccagaacccuugucacuacggggguacaugucgagaccuggucaaugacuuuuacugugacugcaaaaauggcuggaaaggaaagacuugccauucccgugacagccagugugacgaagccacguguaauaauggugguaccugcuaugaugaaguggacacguuuaagugcaugugucccgguggcugggaaggaacaaccuguaauauagcuagaaacaguagcugccugccgaaccccugucauaauggagguaccugcguggucaauggagacuccuucaccugugucugcaaagaaggcugggaggggccuauuuguacucaaaauaccaacgacugcaguccccauccuuguuacaauagcgggaccuguguggacggagacaacugguaucggugcgaaugugccccggguuuugcugggccagacugcaggauaaacaucaaugagugccagucuuccccuugugccuuuggggccaccuguguggaugagaucaauggcuaccaguguaucugcccuccaggacauaguggugccaagugccaugaaguuucagggcgaucuugcaucaccauggggagagugauacuugauggggccaagugggaugaugacuguaacaccugccagugccugaauggacggguggccugcuccaaggucugguguggcccgagaccuugcaggcuccacaaaagccacaaugagugccccagugggcagagcugcaucccgguccuggaugaccaguguuucgugcgccccugcacugguguuggcgagugucgguccuccagccuccagccagugaagaccaagugcacaucugacuccuauuaccaggauaacugugcaaacaucacuuucaccuuuaacaaagagaugaugucuccaggucuuaccaccgaacacauuugcagcgaauugaggaauuugaauauccugaagaauguuucugcugaauauucgaucuacauagccugugagccuucccugucagcaaacaaugaaauacacguggccaucucugcagaagacauccgggaugaugggaacccugucaaggaaauuaccgauaaaauaauagaucucguuaguaaacgggauggaaacagcucacuuauugcugcgguugcagaagucagaguucagaggcguccucugaaaaacagaacagauuuccugguuccucugcugagcucugucuuaacaguggcuugggucuguugcuuggugacagccuucuacugguguguaaggaagcggcggaagcccagcagccacacucacuccgcccccgaggacaacaccaccaacaaugugcgggagcagcugaaccaaaucaaaaaccccaucgagaaacacggagccaacacgguccccauuaaggauuacgagaacaaaaacucgaaaaugucaaaaaucaggacacacaacucggaaguggaggaggaugacauggauaaacaccagcagaaaguccgcuuugccaaacagccaguguauacgcugguagacagagaggagaaggcccccagcggcacgccgacaaaacacccgaacuggacaaauaaacaggacaacagagacuuggaaagugcccagagcuugaaccggauggaauacaucgua

SEQ ID NO: 127 - RNA, 3162 nt, Artificial Sequence
  Synthetic polynucleotide
augcgguccccacggacgcgcggccggcccgggcgcccccugagucuucugcucgcccugcucugugcccugcgagccaaggugugcggggccucgggucaguuugagcuggagauccuguccaugcagaacgugaauggagagcuacagaaugggaacuguugugguggaguccggaacccuggcgaccgcaagugcacccgcgacgagugugauacguacuucaaagugugccucaaggaguaucagucccgcgucacugccgggggacccugcagcuucggcucagggucuacgccugucaucggggguaacaccuucaaucucaaggccagccguggcaacgaccguaaucgcaucguacugccuuucaguuucgccuggccgagguccuacacuuugcugguggaggccugggauuccaguaaugacacuauucaaccugauagcauaauugaaaaggcuucucacucaggcaugauaaacccuagccggcaauggcagacacugaaacaaaacacagggauugcccacuucgaguaucagauccgagugaccugugaugaccacuacuauggcuuuggcugcaauaaguucugucgucccagagaugacuucuuuggacauuaugccugugaccagaacggcaacaaaacuugcauggaaggcuggauggguccugauugcaacaaagcuaucugccgacagggcugcagucccaagcaugggucuuguaaacuuccaggugacugcaggugccaguacgguuggcagggccuguacugcgacaagugcaucccgcacccaggauguguccacggcaccugcaaugaacccuggcagugccucugugagaccaacugggguggacagcucugugacaaagaucugaauuacugugggacucaucagcccugucucaaccggggaacauguagcaacacugggccugacaaauaccagugcuccugcccagagggcuacucgggccccaacugugaaauugcugagcaugcuugucucucugaccccugccauaaccgaggcagcugcaaggagaccuccucaggcuuugagugugaguguucuccaggcuggacuggccccacguguuccacaaacaucgaugacuguucuccaaauaacuguucccaugggggcaccugccaggaucuggugaauggauucaagugugugugcccgccccaguggacuggcaagacuugucaguuagaugcaaaugagugcgaggccaaaccuuguguaaaugccagauccuguaagaaucugauugccagcuacuacugugauugccuuccuggcuggaugggucagaacugugacauaaauaucaaugacugccuuggccagugucagaaugacgccuccugucgggauuugguuaaugguuaucgcuguaucuguccaccuggcuaugcaggcgaucacugugagagagacaucgaugagugugcuagcaaccccugcuugaaugggggucacugucagaaugaaaucaacagauuccagugucucugucccacugguuucucuggaaaccucugucagcuggacaucgauuacugcgagcccaacccuugccagaauggcgcccagugcuacaaucgugccagugacuauuucugcaagugccccgaggacuaugagggcaagaacugcucacaccugaaagaccacugccguaccaccaccugcgaagugauugacagcugcacuguggccauggccuccaacgacacgccugaaggggugcgguauaucucuucuaacgucugugguccccaugggaagugcaagagccagucgggaggcaaauucaccugugacuguaacaaaggcuucaccggcaccuacugccaugaaaauaucaacgacugcgagagcaaccccuguaaaaacgguggcaccugcaucgauggcguuaacuccuacaaguguaucuguagugacggcugggagggagcgcacugugagaacaacauaaaugacuguagccagaacccuugucacuacggggguacaugucgagaccuggucaaugacuuuuacugugacugcaaaaauggcuggaaaggaaagacuugccauucccgugacagccagugugacgaagccacguguaauaauggugguaccugcuaugaugaaguggacacguuuaagugcaugugucccgguggcugggaaggaacaaccuguaauauagcuagaaacaguagcugccugccgaaccccugucauaauggagguaccugcguggucaauggagacuccuucaccugugucugcaaagaaggcugggaggggccuauuuguacucaaaauaccaacgacugcaguccccauccuuguuacaauagcgggaccuguguggacggagacaacugguaucggugcgaaugugccccggguuuugcugggccagacugcaggauaaacaucaaugagugccagucuuccccuugugccuuuggggccaccuguguggaugagaucaauggcuaccaguguaucugcccuccaggacauaguggugccaagugccaugaaguuucagggcgaucuugcaucaccauggggagagugauacuugauggggccaagugggaugaugacuguaacaccugccagugccugaauggacggguggccugcuccaaggucugguguggcccgagaccuugcaggcuccacaaaagccacaaugagugccccagugggcagagcugcaucccgguccuggaugaccaguguuucgugcgccccugcacugguguuggcgagugucgguccuccagccuccagccagugaagaccaagugcacaucugacuccuauuaccaggauaacugugcaaacaucacuuucaccuuuaacaaagagaugaugucuccaggucuuaccaccgaacacauuugcagcgaauugaggaauuugaauauccugaagaauguuucugcugaauauucgaucuacauagccugugagccuucccugucagcaaacaaugaaauacacguggccaucucugcagaagacauccgggaugaugggaacccugucaaggaaauuaccgauaaaauaauagaucucguuaguaaacgggauggaaacagcucacuuauugcugcgguugcagaa

SEQ ID NO: 128 - RNA, 3138 nt, Artificial Sequence
  Synthetic polynucleotide
augcgguccccacggacgcgcggccggcccgggcgcccccugagucuucugcucgcccugcucugugcccugcgagccaaggugugcggggccucgggucaguuugagcuggagauccuguccaugcagaacgugaauggagagcuacagaaugggaacuguugugguggaguccggaacccuggcgaccgcaagugcacccgcgacgagugugauacguacuucaaagugugccucaaggaguaucagucccgcgucacugccgggggacccugcagcuucggcucagggucuacgccugucaucggggguaacaccuucaaucucaaggccagccguggcaacgaccguaaucgcaucguacugccuuucaguuucgccuggccgagguccuacacuuugcugguggaggccugggauuccaguaaugacacuauucaaccugauagcauaauugaaaaggcuucucacucaggcaugauaaacccuagccggcaauggcagacacugaaacaaaacacagggauugcccacuucgaguaucagauccgagugaccugugaugaccacuacuauggcuuuggcugcaauaaguucugucgucccagagaugacuucuuuggacauuaugccugugaccagaacggcaacaaaacuugcauggaaggcuggauggguccugauugcaacaaagcuaucugccgacagggcugcagucccaagcaugggucuuguaaacuuccaggugacugcaggugccaguacgguuggcagggccuguacugcgacaagugcaucccgcacccaggauguguccacggcaccugcaaugaacccuggcagugccucugugagaccaacugggguggacagcucugugacaaagaucugaauuacugugggacucaucagcccugucucaaccggggaacauguagcaacacugggccugacaaauaccagugcuccugcccagagggcuacucgggccccaacugugaaauugcugagcaugcuugucucucugaccccugccauaaccgaggcagcugcaaggagaccuccucaggcuuugagugugaguguucuccaggcuggacuggccccacguguuccacaaacaucgaugacuguucuccaaauaacuguucccaugggggcaccugccaggaucuggugaauggauucaagugugugugcccgccccaguggacuggcaagacuugucaguuagaugcaaaugagugcgaggccaaaccuuguguaaaugccagauccuguaagaaucugauugccagcuacuacugugauugccuuccuggcuggaugggucagaacugugacauaaauaucaaugacugccuuggccagugucagaaugacgccuccugucgggauuugguuaaugguuaucgcuguaucuguccaccuggcuaugcaggcgaucacugugagagagacaucgaugagugugcuagcaaccccugcuugaaugggggucacugucagaaugaaaucaacagauuccagugucucugucccacugguuucucuggaaaccucugucagcuggacaucgauuacugcgagcccaacccuugccagaauggcgcccagugcuacaaucgugccagugacuauuucugcaagugccccgaggacuaugagggcaagaacugcucacaccugaaagaccacugccguaccaccaccugcgaagugauugacagcugcacuguggccauggccuccaacgacacgccugaaggggugcgguauaucucuucuaacgucugugguccccaugggaagugcaagagccagucgggaggcaaauucaccugugacuguaacaaaggcuucaccggcaccuacugccaugaaaauaucaacgacugcgagagcaaccccuguaaaaacgguggcaccugcaucgauggcguuaacuccuacaaguguaucuguagugacggcugggagggagcgcacugugagaacaacauaaaugacuguagccagaacccuugucacuacggggguacaugucgagaccuggucaaugacuuuuacugugacugcaaaaauggcuggaaaggaaagacuugccauucccgugacagccagugugacgaagccacguguaauaauggugguaccugcuaugaugaaguggacacguuuaagugcaugugucccgguggcugggaaggaacaaccuguaauauagcuagaaacaguagcugccugccgaaccccugucauaauggagguaccugcguggucaauggagacuccuucaccugugucugcaaagaaggcugggaggggccuauuuguacucaaaauaccaacgacugcaguccccauccuuguuacaauagcgggaccuguguggacggagacaacugguaucggugcgaaugugccccggguuuugcugggccagacugcaggauaaacaucaaugagugccagucuuccccuugugccuuuggggccaccuguguggaugagaucaauggcuaccaguguaucugcccuccaggacauaguggugccaagugccaugaaguuucagggcgaucuugcaucaccauggggagagugauacuugauggggccaagugggaugaugacuguaacaccugccagugccugaauggacggguggccugcuccaaggucugguguggcccgagaccuugcaggcuccacaaaagccacaaugagugccccagugggcagagcugcaucccgguccuggaugaccaguguuucgugcgccccugcacugguguuggcgagugucgguccuccagccuccagccagugaagaccaagugcacaucugacuccuauuaccaggauaacugugcaaacaucacuuucaccuuuaacaaagagaugaugucuccaggucuuaccaccgaacacauuugcagcgaauugaggaauuugaauauccugaagaauguuucugcugaauauucgaucuacauagccugugagccuucccugucagcaaacaaugaaauacacguggccaucucugcagaagacauccgggaugaugggaacccugucaaggaaauuaccgauaaaauaauagaucucguuaguaaacgggauggaaacagc

SEQ ID NO: 129 - RNA, 783 nt, Artificial Sequence
  Synthetic polynucleotide
augggagucaaaguucuguuugcccugaucugcaucgcuguggccgaggccugugaugacuacuacuauggcuuuggcugcaauaaguucugccgccccagagacaagacccacaccugcccccccugccccgcccccgaggccgccggcggccccagcguguuccuguucccccccaagcccaaggacacccuguacaucaccagggagcccgaggugaccugcguggugguggacgugagccacgaggaccccgaggugaaguucaacugguacguggacggcguggaggugcacaacgccaagaccaagcccagggaggagcaguacaacagcaccuacaggguggugagcgugcugaccgugcugcaccaggacuggcugaacggcaaggaguacaagugcaaggugagcaacaaggcccugcccgcccccaucgagaagaccaucagcaaggccaagggccagcccagggagccccagguguacacccugccccccagcagggacgagcugaccaagaaccaggugagccugaccugccuggugaagggcuucuaccccagcgacaucgccguggagugggagagcaacggccagcccgagaacaacuacaagaccaccccccccgugcuggacagcgacggcagcuucuuccuguacagcaagcugaccguggacaagagcagguggcagcagggcaacguguucagcugcagcgugaugcacgaggcccugaaguuccacuacacccagaagagccugagccugagccccggcaag

SEQ ID NO: 130 - RNA, 828 nt, Artificial Sequence
  Synthetic polynucleotide
augggagucaaaguucuguuugcccugaucugcaucgcuguggccgaggccgacaagacccacaccugcccccccugccccgcccccgaggccgccggcggccccagcguguuccuguucccccccaagcccaaggacacccuguacaucaccagggagcccgaggugaccugcguggugguggacgugagccacgaggaccccgaggugaaguucaacugguacguggacggcguggaggugcacaacgccaagaccaagcccagggaggagcaguacaacagcaccuacaggguggugagcgugcugaccgugcugcaccaggacuggcugaacggcaaggaguacaagugcaaggugagcaacaaggcccugcccgcccccaucgagaagaccaucagcaaggccaagggccagcccagggagccccagguguacacccugccccccagcagggacgagcugaccaagaaccaggugagccugaccugccuggugaagggcuucuaccccagcgacaucgccguggagugggagagcaacggccagcccgagaacaacuacaagaccaccccccccgugcuggacagcgacggcagcuucuuccuguacagcaagcugaccguggacaagagcagguggcagcagggcaacguguucagcugcagcgugaugcacgaggcccugaaguuccacuacacccagaagagccugagccugagccccggcaaggguggcgguggcucgggcgguggugggucggguggcggcggaucuugugaugacuacuacuauggcuuuggcugcaauaaguucugccgccccaga

SEQ ID NO: 131 - protein, 1218 aa, Artificial Sequence
  Synthetic polypeptide
MRSPRTRGRPGRPLSLLLALLCALRAKVCGASGQFELEILSMQNVNGELQNGNCCGGVRNPGDRKCTRDECDTYFKVCLKEYQSRVTAGGPCSFGSGSTPVIGGNTFNLKASRGNDRNRIVLPFSFAWPRSYTLLVEAWDSSNDTIQPDSIIEKASHSGMINPSRQWQTLKQNTGIAHFEYQIRVTCDDHYYGFGCNKFCRPRDDFFGHYACDQNGNKTCMEGWMGPDCNKAICRQGCSPKHGSCKLPGDCRCQYGWQGLYCDKCIPHPGCVHGTCNEPWQCLCETNWGGQLCDKDLNYCGTHQPCLNRGTCSNTGPDKYQCSCPEGYSGPNCEIAEHACLSDPCHNRGSCKETSSGFECECSPGWTGPTCSTNIDDCSPNNCSHGGTCQDLVNGFKCVCPPQWTGKTCQLDANECEAKPCVNARSCKNLIASYYCDCLPGWMGQNCDININDCLGQCQNDASCRDLVNGYRCICPPGYAGDHCERDIDECASNPCLNGGHCQNEINRFQCLCPTGFSGNLCQLDIDYCEPNPCQNGAQCYNRASDYFCKCPEDYEGKNCSHLKDHCRTTTCEVIDSCTVAMASNDTPEGVRYISSNVCGPHGKCKSQSGGKFTCDCNKGFTGTYCHENINDCESNPCKNGGTCIDGVNSYKCICSDGWEGAHCENNINDCSQNPCHYGGTCRDLVNDFYCDCKNGWKGKTCHSRDSQCDEATCNNGGTCYDEVDTFKCMCPGGWEGTTCNIARNSSCLPNPCHNGGTCVVNGDSFTCVCKEGWEGPICTQNTNDCSPHPCYNSGTCVDGDNWYRCECAPGFAGPDCRININECQSSPCAFGATCVDEINGYQCICPPGHSGAKCHEVSGRSCITMGRVILDGAKWDDDCNTCQCLNGRVACSKVWCGPRPCRLHKSHNECPSGQSCIPVLDDQCFVRPCTGVGECRSSSLQPVKTKCTSDSYYQDNCANITFTFNKEMMSPGLTTEHICSELRNLNILKNVSAEYSIYIACEPSLSANNEIHVAISAEDIRDDGNPVKEITDKIIDLVSKRDGNSSLIAAVAEVRVQRRPLKNRTDFLVPLLSSVLTVAWVCCLVTAFYWCVRKRRKPSSHTHSAPEDNTTNNVREQLNQIKNPIEKHGANTVPIKDYENKNSKMSKIRTHNSEVEEDDMDKHQQKVRFAKQPVYTLVDREEKAPSGTPTKHPNWTNKQDNRDLESAQSLNRMEYIV

SEQ ID NO: 132 - protein, 1054 aa, Artificial Sequence
  Synthetic polypeptide
MRSPRTRGRPGRPLSLLLALLCALRAKVCGASGQFELEILSMQNVNGELQNGNCCGGVRNPGDRKCTRDECDTYFKVCLKEYQSRVTAGGPCSFGSGSTPVIGGNTFNLKASRGNDRNRIVLPFSFAWPRSYTLLVEAWDSSNDTIQPDSIIEKASHSGMINPSRQWQTLKQNTGIAHFEYQIRVTCDDHYYGFGCNKFCRPRDDFFGHYACDQNGNKTCMEGWMGPDCNKAICRQGCSPKHGSCKLPGDCRCQYGWQGLYCDKCIPHPGCVHGTCNEPWQCLCETNWGGQLCDKDLNYCGTHQPCLNRGTCSNTGPDKYQCSCPEGYSGPNCEIAEHACLSDPCHNRGSCKETSSGFECECSPGWTGPTCSTNIDDCSPNNCSHGGTCQDLVNGFKCVCPPQWTGKTCQLDANECEAKPCVNARSCKNLIASYYCDCLPGWMGQNCDININDCLGQCQNDASCRDLVNGYRCICPPGYAGDHCERDIDECASNPCLNGGHCQNEINRFQCLCPTGFSGNLCQLDIDYCEPNPCQNGAQCYNRASDYFCKCPEDYEGKNCSHLKDHCRTTTCEVIDSCTVAMASNDTPEGVRYISSNVCGPHGKCKSQSGGKFTCDCNKGFTGTYCHENINDCESNPCKNGGTCIDGVNSYKCICSDGWEGAHCENNINDCSQNPCHYGGTCRDLVNDFYCDCKNGWKGKTCHSRDSQCDEATCNNGGTCYDEVDTFKCMCPGGWEGTTCNIARNSSCLPNPCHNGGTCVVNGDSFTCVCKEGWEGPICTQNTNDCSPHPCYNSGTCVDGDNWYRCECAPGFAGPDCRININECQSSPCAFGATCVDEINGYQCICPPGHSGAKCHEVSGRSCITMGRVILDGAKWDDDCNTCQCLNGRVACSKVWCGPRPCRLHKSHNECPSGQSCIPVLDDQCFVRPCTGVGECRSSSLQPVKTKCTSDSYYQDNCANITFTFNKEMMSPGLTTEHICSELRNLNILKNVSAEYSIYIACEPSLSANNEIHVAISAEDIRDDGNPVKEITDKIIDLVSKRDGNSSLIAAVAE

SEQ ID NO: 133 - protein, 1046 aa, Artificial Sequence
  Synthetic polypeptide
MRSPRTRGRPGRPLSLLLALLCALRAKVCGASGQFELEILSMQNVNGELQNGNCCGGVRNPGDRKCTRDECDTYFKVCLKEYQSRVTAGGPCSFGSGSTPVIGGNTFNLKASRGNDRNRIVLPFSFAWPRSYTLLVEAWDSSNDTIQPDSIIEKASHSGMINPSRQWQTLKQNTGIAHFEYQIRVTCDDHYYGFGCNKFCRPRDDFFGHYACDQNGNKTCMEGWMGPDCNKAICRQGCSPKHGSCKLPGDCRCQYGWQGLYCDKCIPHPGCVHGTCNEPWQCLCETNWGGQLCDKDLNYCGTHQPCLNRGTCSNTGPDKYQCSCPEGYSGPNCEIAEHACLSDPCHNRGSCKETSSGFECECSPGWTGPTCSTNIDDCSPNNCSHGGTCQDLVNGFKCVCPPQWTGKTCQLDANECEAKPCVNARSCKNLIASYYCDCLPGWMGQNCDININDCLGQCQNDASCRDLVNGYRCICPPGYAGDHCERDIDECASNPCLNGGHCQNEINRFQCLCPTGFSGNLCQLDIDYCEPNPCQNGAQCYNRASDYFCKCPEDYEGKNCSHLKDHCRTTTCEVIDSCTVAMASNDTPEGVRYISSNVCGPHGKCKSQSGGKFTCDCNKGFTGTYCHENINDCESNPCKNGGTCIDGVNSYKCICSDGWEGAHCENNINDCSQNPCHYGGTCRDLVNDFYCDCKNGWKGKTCHSRDSQCDEATCNNGGTCYDEVDTFKCMCPGGWEGTTCNIARNSSCLPNPCHNGGTCVVNGDSFTCVCKEGWEGPICTQNTNDCSPHPCYNSGTCVDGDNWYRCECAPGFAGPDCRININECQSSPCAFGATCVDEINGYQCICPPGHSGAKCHEVSGRSCITMGRVILDGAKWDDDCNTCQCLNGRVACSKVWCGPRPCRLHKSHNECPSGQSCIPVLDDQCFVRPCTGVGECRSSSLQPVKTKCTSDSYYQDNCANITFTFNKEMMSPGLTTEHICSELRNLNILKNVSAEYSIYIACEPSLSANNEIHVAISAEDIRDDGNPVKEITDKIIDLVSKRDGNS